European Patent Application EP 4 692 338 A1, published February 11, 2026. Title: CAS12 PROTEINS AND USES THEREOF. Applicant: GUANGZHOU REFORGENE MEDICINE CO., LTD. Application EP PCT/CN2024/119862, filed September 19, 2024. The sequence listing filed with the application follows.

SEQUENCE LISTING (974 sequences)

SEQ ID NO: 1 - protein, 888 aa, synthetic construct
MKTKDIINTVRSSNIKFKSYDKELETFYNHLQDDYKKFFHLFLDWLCLGYTYINEDNQSVIVEPEEQLKQLKKYTKGNQKLEANIKAFVNLLTSGQTPASSCYNSFYANYSAAETSRCNKKLVEKLLESNKKQIEEYIESSKNALLKNISVDKWLEHKKELSKFKSISDKKKREKAQAEYWKEHIGQATLNTDRHCGAYLRKELKIKCRHPENASYCKTLCEMIRRQLTAVLEHNKQHAEELNKTKEQIEKFSQDESFKLICKIAETYPDDFHHYNFKNALNHIFYNKKMDSKNKDKIQLIVDALLPSKGLGYKTLFKAFDNWEIFERYQYRIKNRKYPLKPRLSDVNVPFDNFRFSDGSKFQGKLLNFNFECCYSHYFHDLQFEKIKEGYNLSFFHRLKNGNTKNVILTSNKISGTVKEVSVLKKNNELHLSVPYNIYHSNQNENLKYYFSFAAPSSEKLDLLPDSFKAIGVDLNIQDPVVVTLGAITKKDSYKIKVRDFGSAKLLETQTLVPDTNLSNEIKKLNSEIMTIKGILYEIKKISKDDSLEFDIESLGYLGLEIDRSKDHIGARGVVQNKIKLLKSKIKQYRHKCRNTGNKSVSELIRLIEIVDNFNSMISVYQRLHLKSGEQLLATKRNDNTRKNLKKDLLKKLANKIVKYCLDNQVSLVFLEDLDSEQSSRNSRERNSLIRLFSAKSILDSIETALGKYGISCLSNIDKKGTSKTDPFTGNIAYRDEKDKRNLYVNVKKKNKLVCYNADHTASLNVFLRGIDHSIIPYSFLWANSKDKDKEKGKRISRFLKDKFGTTKVYFYDLGEDHLTVSTKSLKNKSKYFGKIYYRNNKFITEKQHFEMEEKLKKEIMDGLAVGTQVEKIDITSKNINTCVNFQE

SEQ ID NO: 2 - protein, 997 aa, synthetic construct
MSETTKSKFPINKQVTNTVSADILADEKTTSKLTDILNVNSIVKNDLLKLMLTFRGGKCQLDDVEFDSDKEFDKLYAALGTSLPKEVIKALAKEFYYGLTGGLTSRAVKNIIYSPKEIKTSVSYKMDVPDQPNKKESKDKDQKKGKTSKKAKKPKKSVVTSEFDILRKSGIFPLKTPQECSGGMLYSVVKTVQNDLISLEEKTKAYEADKQCWLSKLATALCKFPHIGRYGDFLASVEGLSGIKSWNANGYIRFIKLWHDNSSRKGIRSFLLEKHTQYGNKSVAFTAEDTCGFGYQPDFFDSLYKNFKDLWLIEDVIGNEDYISFICGRDNTEDDKKNKGGAYHWRKEFINISSPERYGKKAVLMLSNGVDNDKGNFVPFTLDFSNENWIMTIDNPLTGEKLSFKLSKGTYYNNFSVLPNKPVKVKKDKNVKKDKNVKVEKAKGGYKIRYSTRKDDKYMYISYLKQPCLRYDPKKGCFKIDFINSDKQVEGLDVNVKNLRGMQKYFSTSSNFDKRAKDVLPGFENKEFIAIGADRGTFPTAAFAVARVNKSKDGTFTIKEWLDEEFLSRNENADEMTRKIKNVTDKITAVKRLTNETVKFKKGEIAEIPPTFTRTFKGKDGTVTATIKWQTLLEIDAEDYTGQVKKLPYDKDSKFTLLQQWIPSSVEWDVKRVMHDIKIEKNAIKNAFQNSENKTEYLQQNNKVDSSTYRKLEMIKGWISLQKKFCGSGPDVCKKDYDWLNGLRKHIDNQLSSNIVAVARKYREKYGLEVVVFLEKLDAFLSGFDDKHHNSTKALWGIGSLNKKLSEKGEKFGILFVPVDPYQTSIMDSETNLLGYRNWAEDKSDLYVKRNGEIQVVNADINAAKNIIIRGIFRHKNIVEFSSDEISDDLYRVMPVGKQRKGALFGHTGSDAILLSDKDGDGELFVASKSLNEAQQQATPINKDKKKVYVVFQDGKWIFRHKLDEQLKQYPSLLKAKPQVSKGNKKSVISRDLQLAH

SEQ ID NO: 3 - protein, 903 aa, synthetic construct
MSCVCNNSIPIDEEIYMALIQRAGVLKTKSDFPKVIKDWHDSLLADYRKFFPIIFSWCPEYGYTTIQDNKPVFVSPEERIESIRKEAKEHLNEVLAFGKMIGSKGVGGSSSYAIFYKHHKNNENGAYTPSRAKFMKEGIHNRRVELVDALMLNAIPDKEWIRIAQEVVGYSEDRLKLYWNKFIAKKVVSHDRKLGKIVREKYLEPKGLVCAQPENSTYCRVLTEIIKRQLHSQIEKSKFHEEELKSIEKTVSEFDSPLLDVICQYAEELNQINSGLSKYVIKNAVKEVISPPEKQSEIYVQSQVLSQEKYKPLVNATIKEILSGYEQWKVKSRYENRLKNRKYVLYPKLSANYKIPIGQNSLGRFKINVSENGEIVIRLNNMADVVCMPSKYFFNLKSSPVVDKKKQLVGYQISFNHNSRRKEPTEKPDFNGIVKEIGLQLKDDGRFYITLPYCMEYSNDNFDLIRPLLTSSPTEDQIKKMPSEFNVVGFDLNLSMPLPITRAIVGKSVKGEINVEYLGQAKVIESTHLIYDNNRCKVLIAYKRQCDLIKRAIREWKICKGKNIDISEKTYEWLESHTKRWNPSRQPESMQDRFSVSKMRIQILVNKAKSRIAKYNDNSWKTGHGNESELIRLIDADDAYNSLVSTYNRIHLKSNQFIYALPSKNNSRSNKKEYCLRRIAAKIARYCHLHNVNICIGENLSFQQDSDNISKDNSLVRLFSSKSIASYMKLAMEKFGIAFIDSADPSGTSKTDPVTGNIGYRNKFDKRKLHVLRNGNWGWVDSDIAASLNILIRGINRSIVPYKFFVGKKKQESKRLNHFLNKIFGTTKVFFYEDQFGFANPSLSKKEGENLIANQYLYYREGKFVTQKIHRQIEDDFKKIDFSNTPEVNLIPSGVKLKNFQFE

SEQ ID NO: 4 - protein, 907 aa, synthetic construct
MATLDAMPAIHGFDSTSRCYMALIQRAGVLKTKSDFPKVIKDWHDSLLADYRKFFPIIFSWCPEYGYTTIQDNKPVFVSPEERIESIRKEAKEHLNEVLAFGKMIGSKGVGGSSSYAIFYKHHKNNENGAYTPSRAKFMKEGIHNRRVELVDALMLNAIPDKEWIRIAQEVVGYSEDRLKLYWNKFIAKKVVSHDRKLGKIVREKYLEPKGLVCAQPENSTYCRVLTEIIKRQLHSQIEKSKFHEEELKSIEKTVSEFDSPLLDVICQYAEELNQINSGLSKYVIKNAVKEVISPPEKQSEIYVQSQVLSQEKYKPLVNATIKEILSGYEQWKVKSRYENRLKNRKYVLYPKLSANYKIPIGQNSLGRFKINVSENGEIVIRLNNMADVVCMPSKYFFNLKSSPVVDKKKQLVGYQISFNHNSRRKEPTEKPDFNGIVKEIGLQLKDDGRFYITLPYCMEYSNDNFDLIRPLLTSSPTEDQIKKMPSEFNVVGFDLNLSMPLPITRAIVGKSVKGEINVEYLGQAKVIESTHLIYDNNRCKVLIAYKRQCDLIKRAIREWKICKGKNIDISEKTYEWLESHTKRWNPSRQPKSMQDRFSVSKMRIQILVNKAKSRIAKYNDNSWKTGHGNESELIRLIDADDAYNSLVSTYNRIHLKSNQFIYALPSKNNSRSNKKEYCLRRIAAKIARYCHLHNVNICIGENLSFQQDSDNISKDNSLVRLFSSKSIASYMKLAMEKFGIAFIDSADPSGTSKTDPVTGNIGYRNKFDKRKLHVLRNGNWGWVDSDIAASLNILIRGINRSIVPYKFFVGKKKQESKRLNHFLNKIFGTTKVFFYEDQFGFANPSLSKKEGENLIANQYLYYREGKFVTQKIHRQIEDDFKKIDFSNTSEVNLIPSGVKLKNFQFE

SEQ ID NO: 5 - protein, 831 aa, synthetic construct
VVTPESQSDAKKAFADALFAGQEAAYGSFYAKYTPLPFPRKDSALGRLTAELGTIGDEKYAKALKLNGLDPDEWAGYRNRAIAGEPPDALWEEIKVKVGVTNKATLASRGVGNLPTLRPDSKSYATALAYMLSSSLSSWEECAKLHRARREEIAAKAAVPDSMTEEYALVCQLAQALEEAGSGLTAKMLNGAIREMAKTDSVYMVAITELADPKYKPLLALDKEDRARLMDTWQAERKLSTSLAAPKRPLFDKDYQIPFGMTGRGESFALRTDDSGRLWVKIGDHEEFSCAASDYFGNLKVEALPSDKGYKITYRKMVKNRRRQRAGYKSSVGGPLIEGEVKQILLQRRMNRRGKESFYVYLPHSIAVKDDRRHLSWFFKRADWKDGKGLEELPDQLIVSGIDLNIDQPVTVTKAIVSKNYTEGEINCPYGGGHLTGKPRSVCPDTPISQEAKLTHRKMRLLIEVIRESKACHKAGTPLSSEGSERLKILYADISKPPCRNNRESIQVVYSSLKKTYRRLKYELMQQGANDVSGCIRMLQLDDTHRALTACFDAFSGKPALAGRNFGVARKKTSKGTARLNFREHVSHLYANAVLRACHGSDVVFIEDLSTSFDGNAHNSLKRLFAPGQLIDAITSLLESHGIAVVTVDPSGTSRRHPITGDIWYRDSMKKRELVGLIDGELVSVNDDLAASINVLTKGLNHSVVPHKFKVDPSGRVNVKEDGGKRLKVFLREKGLSGRLPVGSADAAKSKKAKALTVYPSSSGLLSDRQVFEVLEQIKHLLAAGCKPRPVELMAGPGETYAAFSLKEVLEWSKSKSSEDLRHTGLGDETG

SEQ ID NO: 6 - protein, 882 aa, synthetic construct
MEKFPRCSHLKVKQHCGPFVEWYEDLQSDRQKYVSLFFPWIGIGYGERKDEGDDIDFISPEQTLERRKAELGKLEELVVRFVTVMLKGGSSASSCYSLFYEDYKGKDTAKKSTSKVNFIKALPLLSKKEIEDRVLGDNQLSLINLDEWMELGQSGLSADDIWDKVSQRLVTGERSLGVDVRHTLKIRCQRPRDRGYCVVLMEMVARQLRSCYECYKNHLNELQELREKTTKQITESRDDLFSLVCDLATVLTEQDSGLSERTLFSGRKQALKPQGKPSKIQAIVDELRQPQYSPLLEADDKELRQAYKAWNSQRRLRDRETRRPYPCRPNWRNDYQVSLGLTGRGGFWMWMDGSDVVVDLQDCGRLTCSPSHYFGDLAIEGQLHQYDIRYRNKLKRRGKKLRKPPAYGEWIEATIKEIGIQRKGGDYYVYLLPVISHDSTNFQAAKKFFAAAAPKQEIIDALPDEMKVLALDLNISNPVCSVKARIGRALDGPLSVLDYGQGEIVDGPKILVTDGPRCVALIELHSDVFFVKDAIREYKRTHGVAFNGAGMDDEMLERLSSIPSPSPSVRCQIQAWVAAIGKRLHLLHYGMRREGYKNLGEAIRLLAAMDAYDSMLQSYQRIHLKKGQSLPRQAKNDHSRAGLRETITRRIAYAIAQEARDCNVVFVEDLKADFDADNDNNALLRLFAVKTLIRYIQEALEKIGVGLVLVAKDGTSKTNPMNGDLGWRDRNNKEHLYFELNGEAVRCHADLVASLNVLLRGLDHSVCPYSFVTKDTNKKPGRADQKDKGYGKRLKRFFKDRFGSSNLRFVAKPDGEVTATTRRPKDALIGERVYYHGGKLVTSEVHYRMENEIKHLLTLKSPAKELSLTEDGIRSYENFTHV

SEQ ID NO: 7 - protein, 882 aa, synthetic construct
MEKFPRCSHLKVKQHCGPFVEWYEDLQSDRQKYVSLFFPWIGIGYGERKDEGDDIDFISPEQTLERRKAELGKLEELVVRFVTVMLKGGSSASSCYSLFYEDYKGKDTAKKSTSKVNFIKALPLLSKKEIEDRVLGDNQLSLINLDEWMELGQSGLSADDIWDKVSQRLVTGERSLGVDVRHTLKIRCQRPRDRGYCVVLMEMVARQLRSCYECYKNHLNELQELREKTTKQITESRDDLFSLVCDLATVLTEQDSGLSERTLFSGRKQALKPQGKPSKIQAIVDELRQPQYSPLLEADDKELRQAYKAWNSQRRLRDRETRRPYPCRPNWRNDYQVSLGLTGRGGFWMWMDGSDVVVDLQDCGRLTCSPSHYFGDLAIEGQLHQYDIRYRNKLKRRGKKLRKPPAYGEWIEATIKEIGIQRKGGDYYVYLLPVISHDSTNFQAAKKFFAAAAPKQEIIDALPDEMKVLALDLNISNPVCSVKARIGRALDGPLSVLDYGQGEIVDGPKILVTDGPRCVALIELHSDVFFVKDAIREYKRTHGVAFNGAGMDDEMLERLSSIPSPSPSVRCQIQAWVAAIGKRLHLLHYGMRREGYKNLGEAIRLLAAMDAYDSMFQSYQRIHLKKGQSLPRQAKNDHSRAGLRETITRRIAYAIAQEARDCNVVFVEDLKADFDADNDNNALLRLFAVKTLIRYIQEALEKIGVGLVLVAKDGTSKTNPMNGDLGWRDRNNKEHLYFELNGEAVRCHADLVASLNVLLRGLDHSVCPYSFVTKDTNKKPGRADQKDKGYGKRLKRFFKDRFGSSNLRFVAKPDGEVTATTRRPKDALIGERVYYHGGKLVTSEVHYRMENEIKHLLTLKSPAKELSLTEDGIRSYENFTHV

SEQ ID NO: 8 - protein, 994 aa, synthetic construct
MSETTKSEFPINKQVTNTVSADILADEKTTSKLTDILNVNSIVKNDLLKLMLTFRGGKCQLDDVEFDSDKEFDKLYAALGTSLPKEVIKALAKEFYYGLTGGLTSRAVKNIIYSPKEIKTSVSYKMDVPDQPNKKESKDKDQKKGKTSKKAKKPKKSVVTSEFDILRKSGIFPLKTPQECSGGMLYSVVKTVQNDLISLEEKTKAYEADKQYWLSKLATCKYPHIGRYGDFLASVEGLSGIKSWNANGYIRFIKLWHDNSSRKGIRSFLLEKHTQYGNKSVAFTAEDTCGFGYQPDFFDSLYKNFKDLWLIEDVIGNEDYISFICGRDNTEDDKKNKGAYHWRKEFINISSPERYGKKAVLMLSNGVDNDKGNFVPFTLDFSNENWIMTIDNPLTGEKLSFKLSKGTYYNNFSVLPNKPVKVKKDKNVKKDKNVKVEKAKGGYKIRYSTRKDDKYMYISYLKQPCLRYDPKKGCFKIDFINSDKQVEGLDVNVKNLRGMQKYFSTSSNFDKRAKDVLPGFENKEFIAIGADRGTFPTAAFAVARVNKSKDGTFTIKEWLDEEFLSRNENADEMTRKIKNVTDKITAVKRLTNETVKFKKGEIAEIPPTFTRTFKGKDGTVTATIKWQTLLEIDAEDYTGQVKKLPYDKDSKFTLLQQWIPSSVEWDVKRVMHDIKIEKNAIKNAFQNSENKTEYLQQNNKVDSSTYRKLEMIKGWISLQKKFCGSGPDVCKKDYDWLNGLRKHIDNQLSSNIVAVARKYREKYGLEVVVFLEKLDAFLSGFDDKHHNSTKALWGIGSLNKKLSEKGEKFGILFVPVDPYQTSIMDSETNLLGYRNWAEDKSDLYVKRNGEIQVVNADINAAKNIIIRGIFRHKNIVEFSSDEISDDLYRVMPVGKQRKGALFGHTGSDAILLSDKDGDGELFVASKSLNEAQQQATPINKDKKKVYVVFQDGKWIFRHKLDEQLKQYPSLLKAKPQVSKGNKKSVISRDLQLAH

SEQ ID NO: 9 - protein, 887 aa, synthetic construct
MALIQRAGVLKTKSDFPKVIKDWHDSLLADYRKFFPIIFSWCPEYGYTTIQDNKPVFVSPEERIESIRKEAKEHLNEVLAFGKMIGSKGVGGSSSYAIFYKHHKNNENGAYTPSRAKFMKEGIHNRRVELVDALMLNAIPDKEWIRIAQEVVGYSEDRLKLYWNKFIAKKVVSHDRKLGKIVREKYLEPKGLVCAQPENSTYCRVLTEIIKRQLHSQIEKSKFHEEELKSIEKTVSEFDSPLLDVICQYAEELNQINSGLSKYVIKNAVKEVISPPEKQSEIYVQSQVLSQEKYKPLVNATIKEILSGYEQWKVKSRYENRLKNRKYVLYPKLSANYKIPIGQNSLGRFKINVSENGEIVIRLNNMADVVCMPSKYFFNLKSSPVVDKKKQLVGYQISFNHNSRRKEPTEKPDFNGIVKEIGLQLKDDGRFYITLPYCMEYSNDNFDLIRPLLTSSPTEDQIKKMPSEFNVVGFDLNLSMPLPITRAIVGKSVKGEINVEYLGQAKVIESTHLIYDNNRCKVLIAYKRQCDLIKRAIREWKICKGKNIDISEKTYEWLESHTKRWNPSRQPESMQDRFSVSKMRIQILVNKAKSRIAKYNDNSWKTGHGNESELIRLIDADDAYNSLVSTYNRIHLKSNQFIYALPSKNNSRSNKKEYCLRRIAAKIARYCHLHNVNICIGENLSFQQDSDNISKDNSLVRLFSSKSIANYMKLAMEKFGIAFIDSADPSGTSKTDPVTGNIGYRNKFDKRKLHVLRNGNWGWVDSDIAASLNILIRGINRSIVPYKFFVGKKKQESKRLNHFLNKIFGTTKVFFYEDQFGFANPSLSKKEGENLIANQYLYYREGKFVTQKIHRQIEDDFKKIDFSNTPEVNLIPSGVKLKNFQFE

SEQ ID NO: 10 - protein, 824 aa, synthetic construct
MESIRKEAKEHLNEVLAFGKMIGSKGVGGSSSYAIFYKHHKNNENGAYTPSRAKFMKEGIHNRRVELVDALMLNAIPDKEWIRIAQEVVGYSEDRLKLYWNKFIAKKVVSHDRKLGKIVREKYLEPKGLVCAQPENSTYCRVLTEIIKRQLHSQIEKSKFHEEELKSIEKTVSEFDSPLLDVICQYAEELNQINSGLSKYVIKNAVKEVISPPEKQSEIYVQSQVLSQEKYKPLVNATIKEILSGYEQWKVKSRYENRLKNRKYVLYPKLSANYKIPIGQNSLGRFKINVSENGEIVIRLNNMADVVCMPSKYFFNLKSSPVVDKKKQLVGYQISFNHNSRRKEPTEKPDFNGIVKEIGLQLKDDGRFYITLPYCMEYSNDNFDLIRPLLTSSPTEDQIKKMPSEFNVVGFDLNLSMPLPITRAIVGKSVKGEINVEYLGQAKVIESTHLIYDNNRCKVLIAYKRQCDLIKRAIREWKICKGKNIDISEKTYEWLESHTKRWNPSRQPESMQDRFSVSKMRIQILVNKAKSRIAKYNDNSWKTGHGNESELIRLIDADDAYNSLVSTYNRIHLKSNQFIYALPSKNNSRSNKKEYCLRRIAAKIARYCHLHNVNICIGENLSFQQDSDNISKDNSLVRLFSSKSIANYMKLAMEKFGIAFIDSADPSGTSKTDPVTGNIGYRNKFDKRKLHVLRNGNWGWVDSDIAASLNILIRGINRSIVPYKFFVGKKKQESKRLNHFLNKIFGTTKVFFYEDQFGFANPSLSKKEGENLIANQYLYYREGKFVTQKIHRQIEDDFKKIDFSNTPEVNLIPSGVKLKNFQFE

SEQ ID NO: 11 - protein, 903 aa, synthetic construct
MNHFTQNLAVTKIDSSVQTLYDDFQEDFRKWYSILCSWAKVPYRVEDDNGNITHVHAKQRAAELSSLYSAQEQLLIERFMRVFLGASKEASSSYSLFYDKYAPNGAKKTAALKEFLGEIPTLDDSQVEKKANTNKNCKRITVKEWRDFAAQFNKLGIDAIWGKLKEKITSPDRGVGLQVRGFVSERCKHPENAGYCRQLCQKLTEQVKSTVRICELYIQETADLQSEIGNKTKQPEVKKCFDLLCQLSDELRDVNSGLSGRVLFQSIKDIQGGKDSDRKNKVCRTVMSDDKYLCLIDSDKKIVQRAFQAWKLSITLKKRQEKLYPKQRSHQNDVPMPFGLTGLASFDVSPDGSKFTFSEGSVETKPSLYFDGLRFQKNKHSFDMEYRVAYASRRTKKGRRPKRVGRLRKATLKQVELFNKGGKFVIKLPHGIELPEHRAKLATFLMCADPKEKGYSKGGLVDEFRALAIDVNLSNPLAACVADVSKHGDGPIQALDYGRAKLCVDPFFLVANTPVCGQLIKLCKECKAVVQAIKEFKECQAAGSDFSFETDLFLPAGHSPRHRIQSKVQELSRVLRDWKFKLQNTNQVAEMIRLLELMDAYQSMISSYQRIHLKAGQTLPPQKKNSTKRANYRKDISRRLAFVVADYAQSLNVDVVFGEDLKADFDRDKNTNSLSRLFAGGMFLQHLENALAIRGIAFVKCAKNGTSITDPVSGVFGWRDKFNKERLWIERDGELGWVNSDHAACLNVLLVGLMHSVVPYRVYVKAGRKTTDDVEVFEEDHPIGPRKKRFFELCFGENKPKFEVVENRVILDNAGTYQGFIYAHCLDAMQSEKQHWAEYDRIKELALAETNPKQFGLTPKKGEGYRNFCQPDIHEQVEVVGNKRVAATKQILESLADEKIEAT

SEQ ID NO: 12 - protein, 872 aa, synthetic construct
MAYPPFVRTQNFKIKNITTNDELLQWYEDLQFDQRKFYNEFFSWTGLGYYVLAENDEIIYTSPEEAAIQRKEKLGDNESCVARYVDLILQGGKSASSCYNVFYENYKSTGKAKFSEMKCEFLKNLPFQTKKQIQEKISKNKQLSCLTLNEWWGIRDKIKTINKLESNEEKEIETKKVWNTISSQIADTDQTIGVEVRELLNIKCRRPNDCQYCKILSDMVGRQLRSFSEVTKNHLKGTDELKQKLNDSKNDLYNIICEYSDALDALESGLSKYVLFQAIKEAEKPNPESKIQLAVNEIKKGKYESLRQASRKELMKAWKALKLKKRLQIRKKYPRFVVGGNDYPINVGLTGKGNFRLSTHNNKILIEINNFGTFECYPSCYFGNFQATPIMRNKCICGYNIKFRNINKSKNSVTYGPWVIGVVKEVGIKRKNGNYYVSMPYTMRPEDTNFKIATYFAKAKPTLDEFEALPNEIICAGYDLNISNPVVQTTGRVVKNGHGPLKALDYGAGHITKIPTILTPNGLRCHRLIQLKADVYKTKDAIKEYSGNLKQHQDVSNETKEWLKSSDHNNTRYLIQKKIGSITKRFKTLAFEMRAEGYQNLAECIRLLDAMDARNSLLNSYKRGVQKLPPKRQFDSKRADFRNYINRRIGYLIAKSASEENCNIVFLEDLESDFDRDNNNNSLMRLFTPNTLIKCIEEALEKKGIGLVTVAKDGTSKTDPITGSPAHRDRYNKEKLYVERNGQIGWVHADESASLNVLLQGLNHSVCPYKFYVKESTKDYGIRMQRFLKERYGTTNVSFVEDNGQVEAVPKKRPANRLQNTYVYAHHDGIMVTKDKHLQIERKIEDSVMQQIDLPKFSLTDCDERGYRNFSV

SEQ ID NO: 13 - protein, 464 aa, synthetic construct
MPRNSKKKKQSEVRTLRLDVLPVRFGLHNAERVKYPAETTDEAKARVGEACNTVRTYIRKYRLAIRKACAPLLFAQAATEEWSDEKGRAVIGKADAVTEEMSKLTGDKVCIQRNLDRFVKALIPTLKCECFQQVANRIYTAITAKDPDIPISRHLLILDGVRKLPWFMNEPIHLKYCPTYRSDVIFNGHRVFLRWDKELGYVEFKLIGKKLKQNAKGNSKRGLDASQWYIIKQLQSGAWAPGGAKLQLMKDGDFRLICGYQGFELDRPELRAKAGRERIELIPVDKDRIDELSFTEDRERFMVLQLSSGHRASAGIPVDEVTKHEWSALGMLAHVDRLSKQQDRSKKRTSSCGAFHKAREAEQARRDRITRARENAVANWAHEWSLQVANRCMAMRCGQLRVFDIPKEVLFFRPFPWSKFRFDLEYKCRERGIEVSYHESPKDSKGSSDPNAEDSATASVDGQE

SEQ ID NO: 14 - protein, 617 aa, synthetic construct
MSETKEVFEAKKKLEEQEPTAEAVVALGKLLLAAEEEIGLNAASELLPKYLRKRMQLLLSAATGGKAEIEAALEPFVLDWHKKAINSAWKELREVKLERQLIQLARTLQEIDGRIGRQKLVSITPKRLLQQRKLDTLLTVASGLESAEEALEKVVSEPRPLRLQVRPIRVGLERPEHPKKIKNETAEEAKARVGAACEKLRAYLRKYRFSLRQAMNVMYWAQARTEKWNEEKGVPRVGSVEEVKAELRKMTGDPVSIVRNIDRYVRTMLPRINANCLQMASARMYVAWTSKMPETGIPRNLAVMDAAARMPWFANEPLHFKCFKSLNSDVKFDGHRIFVRFDHDLKWVELKIINTKHKRTYNEKPPPKGKRNGGKKSLDYMYWYVLKNLQKGEYSPAGARLQMKDGKFSFSCCYNSERGRPELNDGKKRPFRKVSYDRVADASFTEERTSFIKLSLREGHEPSAGIPVDQVREYPISAEAAIAAIDRLDAQQRKAENRIAATGSSNKRRKAEQKRRKRITEHRENVINQYCHDWSRQLADWCSVMGCGRMMVFDVPDLLFGRSFQWAKLRFHLQSKCRERGIEASFHESPKDSTGDTSRSGDPQAEVSAPCSVGLDE

SEQ ID NO: 15 - protein, 517 aa, synthetic construct
MEVKVLTKVKQPRKEGRGGGSILAARNDLVLKSDSLNVLFDGDLSHFRGVLSKWRCMIQEMENLVEIVEKAVADFSMKKKVVSEIDDPKHPGEKKKVSTWVPTDYVIVRMKLDDAKQAATSILGKDVNLCETKYQEWYRKWQELDVSMGGPHFDRRMFEQAIKIMGAIRNKKVPDRGNIPRNHLVVAGAAKQPWFGNVPLECIYASQSNVFRAKFVKEGNIRKVVLMLNDKDEDAKLTFVVRGAIVDKNGKPHTIGTKKSDRVFDNYFEGRWIPTNPRANIDKRGYCHLYVSNYRPRRAFTGLLDANTLEVTFHKINGEDIRKPWRPEKEQDRLTGRVFTIHTRIMRGNKRSWPANIAINDAIAAMRGYSKRMDEKRECWNTRRFGPKRLRRPFQEIIDNISKAKERTQRQINHRWTNEVIFQATRKGRCRTIRLYGFPDGVKAGLLLDGTVQWPWSEWLRMLIYKAEEAGCFIELVTTQEDINAMGVALHEELTRVKHKEEEEEDDDEAEYGPEAA

SEQ ID NO: 16 - protein, 844 aa, synthetic construct
MEFTNVVSKIREGIFHISMSTSPEITNKHRPLAMARSGSLTFSGNTVTFKGETHTVETPLTDERMPVHVTLTNYNGKVYEFPRSPNVDGLFAVKQKNGDFFLRGSNRNRGDKTEKEQGNYLTVKGRVYHHHRGVETSAELPAWAEAIRTRWKQGWNVLALTLRWVLWKTEDCGETEQDWEALIKNKVDHLLNSREGYVQPDALSPESTAIVDRIRRVIVDSSMAHYATRGREAKLSIPIVLRDNSKVPPAFSDLRNFAYQLGRYEKEEGVKVQMVDEGGEIDILSEWLGIELKALKRNKAPLKAFKALLKAKGEVWTDGFMGTLFGRIRAHLGMDALEAEALSTRFTAVLKQRESKSMPFDRGWPRPIRTGEDAWQLVYNLKGKTTLGELMNNKCSDIQFTQPVSSEISGSPNNKVVTKLKDGTFDVTNEYKPLTPGSVASQRELRGLSFTKGKKGMEPYKLAVLMHRNDVDLNAKVKRVVLSIKTEIEPYVIYKGQPTPSLGAASAFTSPAGRKVTFYQLNICLEGVKTNEKYDRRGTGASHLKLGWKVNGDQLTVVTETRPTGVIVPYSLPLGEVWKTEGILDAGCHSDKPGNAWSRRNNYKMAFYALNGWPVSPLVIEAQKQELVSRFIEGRLTLDWLKTTSLSLPKQIDTLLNVAKAEGFKLMTGGQRAIVTREGWHMVHQKGLVRRIKELRMAENGEAYPASNSNPSRSKEPSKPLGKNKELLTLWLRWLEYNDRLRAVERMVRGHLLGRRKAYYYALAHHLCDHTAAIQYTKLNLKDQAEKKTRKKKDKGEKAVVDNSQKYRMWASLGEFTTILKQVGIKRGVEVKEIEIALTKVAAA

SEQ ID NO: 17 - protein, 629 aa, synthetic construct
MKTKTKTATKTATKTHIDLVLRARLAERGSAGSAVRREARIVIFGADQQTPHPDSEKIVEDDLRGTHEYYNRLVRAVSPKYKKARGLVVGPEARKQELREKQISALYQERHDCAKSEEARINEEILKLKQERRESWALVDKERTALRKKNAEKIQDLIGPSTITPLIKAERNRVSVYGKTRQSSDPTIGWGNYTLAEKDFGLATRKAFNLKSIPHFRGEDRDGTAPEDFRAYKFWQKDGTLRSDFTQKNHHAHRTPEAIFGGKGKLMTIRPFEESDLAAFNLPAAFWDQIARHRSEGKPDRWYVILIVRNGTKVPDADWYGVVANFPAGSKQTPSLLDRLRSVDHVTEARIVRKKQGLRLETHVNLHVKIAVAAKVARETVEVSWGSFTNKGVGKLLVTYPDGRVDEFSEANVPALLRCRQHEETSRKLHESLSKHEKDARKAFKTLNLDPSIIWDREEFPRSPGSIRHVYRRLFRDEMVEALGGEAAREKRDEIMRLCLKLYRQPGPDGEKNPYGGDPDQAREIVAMRMAEIFPISEDKAAAMAVVFVFMERFNHLADWAHRSGFRYHTSRREFYRTFAAELCQKYNVTYLRPPKAGRKVSGDRSVVAPFVLETILKTAALKMGRAWE

SEQ ID NO: 18 - protein, 437 aa, synthetic construct
MSISDIFKANQFKTEIEELKRECNRLQSLLTPEMQDAAQLKREIDKLNFDKYNINNQINDLDKTLDAKYDAIKKLDIVINNKKSQIIWMDDEILVQEFGLYQPKFEFANSQQYKEKLNNNRKLQKESIKNCTAVTGSTNWTVDGNKSKGNKMVKDMQKLLLRAFNGECDELIGKVKYNNYDTSLKRITASKDAISKLGTIMGISITDTYFRLKKEELNLALEYQLKKQQEKEALAQARAEMREAVKLQKELDEQRKKIEKEQNHYQNALHSILKQLENAKDNEKEALETKRLELSKELENIKTSLKDLDYREANQKAGYVYIISNIGAFGENIYKIGMTRRLDPQERIDELGDASVPFKFDVHAIIFSDNAPALEAKLHKAFDSKKVNMVNQRREFFNVSLDEIKEVIRKNYDKTVEFIDVPEAEQFRISQKMKEQL

SEQ ID NO: 19 - protein, 425 aa, synthetic construct
MLEDNEFSKFAFTTHMKKYYKWCRSNISSMVAQAISENVWRAFEKYFYSNGKRLHFKKIGSVTTVAGKGGASGPREIRFKDGYVLWNGLRLKVKLDESNVYEQQMLEHRIRFCRILKKPDRRKNHYYVQFVLEGRPEIKIRPDTGEALHPVGVGRVGIDIGPQTIAYAAECGAGLRELAEGVGNIEREKRLLQRKLDRSRRATNPNNYNADGTIRRGVKLTKNKSNRYLAVQRELAYVYQRQAAMRKQKHIALANELLALGDTFFVEDMPWKGLAKKAKKTEISPKTGKYKRKKRFGKSLGNKAPATLIMILDNKLKSLGLDGVQKIPTTARASQYNHITQTYTQKTLSQRWNTMEDGTKIQRDLYSAFLLQHINEDNKTFNQQTLEEDYPAFQRYHDRVIVQLQNNPHNVASMGIRSATHKRAE

SEQ ID NO: 20 - protein, 416 aa, synthetic construct
MGIIKAAIQSATSTLADQWLDIIEPDTMDNTTLMCKGVLMSKNKKRGSNTKGSVDYISDGSIIRVYPNMMMLLVDGGQIIDYTAEEGYYKVDNSAAPSLFNGDFEGALNESFERFRFGGVTPSKQEVFFINLQEIRGIRFGTQQPINYFDNFYNAELFVRAHGSYSIAITDPILFFKNVVPKGVTRLTIDEINEQFLMEFVSGLQSSINQLSAQGERISYLASKTAELSKVMNQNLDEQWKSLRGIEIVSIALASISYTDDSQQLINMRNKGAMFNDPNLRESFMQTSIAQGIADAGNNPNGAANAFFGMNMGANLTGDYLSQASRQNQAQTQQAAQKQQTANTSSAQESSWQCPNCNQENTGKFCSNCGTPKPTPTANTGMKVRCSKCKSVIEITNAMPKFCPECGQPFLAESLD

SEQ ID NO: 21 - protein, 416 aa, synthetic construct
MGIIKAAIQSATSTLADQWLDIIEPDTMDNTTLMCKGVLMSKNKKRGSNTKGSVDYISDGSMIRVYPNMMMLLVDGGQIIDYTAEEGYYKVDNSAAPSLFNGDFEGALNESFERFRFGGVTPSKQEVFFINLQEIRGIRFGTQQPINYFDNFYNAELFVRAHGSYSIAITDPILFFKNVVPKGVTRLTIDEINEQFLMEFVSGLQSSINQLSAQGERISYLASKTAELSKVMNQNLDEQWKALRGIEIVSIALASISYTDDSQQLINMRNKGAMFNDPNLRESFMQTSIAQGIADAGNNPNGAANAFFGMNMGANLTGDYLSQASRQNQAQAQQAAQKQQTANTSAAQESSWQCPNCNQENTGKFCSNCGTPKPTPTTNAGMKVRCSKCKSVIEITNAMPKFCPECGQPFLAESLD

SEQ ID NO: 22 - protein, 1125 aa, synthetic construct
MAKRSVTPLTEDRQLWEPLPPDDVRLAFVKYLDRRPGSIRRTIQLQLHNPGWRKTQNLLWARKHFNNYIFTILETLREDPHQFRDDGAFECIHEMMVRREETRRQGKPPGKYTRVLGEVIAERFRRPARSGPNNQDTNDETVADNASDRRNHPSRRRPPLRILEARDYPIIHMLRPGAQRRCALILLNFYIQSQKIPQAHEQAPDSQSDEASQNTASNRELEHAHDASHSTAAADFSDEEAAEREETLEAEMEALETDSIPTIEMMHQMWAQRWMRYEAAASTRIPYGQHRGKPFGEALAARRMRTGRERGRLVRKPGKRRVRWLKERTYALEQVHTCLRAVQILLHRDTYGNDSAEVLEAEQVRHLWKYESRTLRRPRARRVEHYRSRQSQPLATLGSLSQEELHTFRDELYEQLDHAHQYAQIAEAVDIFLEHAPPSYPTIDIGLFNDSPERREHHSALNWFPRPVTRGSIRDSDDDIERRPGPSVDELLHRAEYDAVTRLLQAESELGERALQPLTYTRTMRPPAPLPCWALLYKRSCPSHEEREQCARRLPKRMRQRYKDTALNSTDGYVYTFVLAMVVHHTTHAFTGEQPADYFSPSLSEDEYFYVNFPLTPFHPPQGVSLMMFPLECGEEYQEGLLHDLIERLRAEQHAQYAHQFTDPDVDPADRVPVEACLPTQAALGEAKIVTRQNGDDWYEFFLHCAVPIDILVREPPERILGLHHHQHGYSWALIDAVGTLINAGDLQIPWHVRLRPGSSAYSDNYAFEVANQIVALAQEQNALICIENTWTNKKATTSAHQNQRAFAHPSRKIYDQVVSKAIEAGLPRPRAVYGISRSRCGACGNRINNQRGKETLSACPACGSLSRSAHIQFPLASLAPTADGSTAAWVLLAQEQEHGERAAALTDFFYWTLRQAAADVVPAPDRRQAFIAGLEQVQWQGRQVFRPKSGRNTYTRNNQQAGTNSAPSYTFRPRRLEADVVIAGPEAYAPRVQQWIAAYELVAPDVLIEYVSMLREHALDILYGGREDAVADVILLDTPASERELAAGLAQQRSWFCQDCGQHWQVDELRFRCTYEPCRHHDLARYNTAAVVAQIAVHKLLEGSQQERQHATPGTTGGEHETLA

SEQ ID NO: 23 - protein, 465 aa, synthetic construct
MEKYNVSISKSELMSKQDFFKLWMRAYDGAEEVEENHWMTRFDNIINNSAKRIPRYKEKIAQIVFKVLEESYPFFIWGIPNEEQGDFIKTCEKDIKNATKKTISIIIAPCTSLSDFCAKYVRLQLMGGQEWLDMFASNISHYIPTYYAANYLQMPKSEEETLSSFFKGSAITVDNESVSFASLFERELQTACFVYLAKKIMDDEDITEENFIRRLPLLGTPDAGILFHDILSSLLPRLFFDVYQLFAQRSAVEAASSGKTLKKMEEEKKALKAQVSDLNKKLKEKERIIAEKETKIQTLSKKLVTANETSKNIEEVVEKRTEAIAYENKSLMRQNKKLQAYYSDLRSKYDRLKIEMGSSGADVEEDEREEMREVDVNARYLFLLYDDIGCRQNIKQEFPNAEFTSKVVPLSSHKYDMVVSLTECIDHSNYLAMKKQCKIHGVPFAHSPYSNIDMIKTVIWNVLNG

SEQ ID NO: 24 - protein, 1235 aa, synthetic construct
MTAKKKQQPRVWEPPARDALLHAFEQAYAARPDTVTLTIILKLLTQRDTEALLHTAQMRVTNMLHDVTVRFFDDLEQIDAGTTAEHLIDAIIELVSDPIQVDAHHAQAVSQLRASLAVVRTQTIGAMDTTFVSALIAAAASADTADPSHRGWSVLRAFLEQWYIDHPGDKMISTINHAAQATSKRKVKDEHGNLKKDAQGKPMTDVVQTYTPEQVYHIKLALTLRLALVARHEAQVITTRAMALVVLALRQCSNTQAFAWVSTTLTQRFTNTRIHAALALLLVVQQRVHDEACHRIFVTINQRCAGNQMFAVIEVIVELVSRHIPEADNKPAVADTVRHYLYQLTRSRKQRRKPHHVTHANAQVPADETAHADAALFVDEKPHPVRPVLLRIVDALVGSNENTGILPLRMCLEHWYSSFAEQEREERFSAGDRRLIAIARDPTRQDEAGDRHTGMSLLLFHWLQYHCVLSTDVLLLVSLSEKAIRRIGDGDTVLSGILSNCYGEVCSRYQYPLSGELREGVFFNRGGAILGWCQLVADYVAERDKRRPGTTLPPWKTGKPKNVSRVDFFKGNRVVRIGLAYALWKREDTAYKAAVATEAPVGPDEGKTLGNPYAYTELRRQVAGNRRRRVTILGRGSIGKRGARRMKKWMLPAAERRATLRHLDVLLYPELVWNDEERVAAAQASHPYWMKRTKRGITAVRPTQFRLYPSTYPKSLKDLSREKQIQLREELREQERYAPQFAPFRHALDRFLEAAPPAPPFIAPMVLTDADMAQLTPEAQLEWTATFETYKAEFDQNLNWYRDFRPSRGTPTEEYSDEKLYDVETLHNRELEWSAATLAQRHPQPIYFKRGMNAELKPRSFALLYHIPQRKGCARYRFTFVCDLVGETATEREALLTKRRARGEHTVENFLVNHPDQRVTHPNETTLHYFATQMGSDHQERILLEYMDWRRREPERKKPLISTARIVSHKRTRQRTDWYAHLPVPLPAPTHTATLDTVIGFHEHEGTFFYAVVDLDGRLLALGDVDLPNCVRPKRTDGMTNDNFAFETAVRMVWRSMTQQYFHKFRDNPKRYTAFIGIENTGWKQDRVGTKAADNRQNISLPRQRIIEIVTYKAIRHGLPTPLSVKRISPGRDCGHCDARIEHGSGIEKRPVTHCFHCQTLGIEHELEWHKEADNKWSARCITCGRSWRKEEPQFKCQHCRTQQYARYNTALATVHCTVDILVGRKRNTPDSEQE

SEQ ID NO: 25 - protein, 404 aa, synthetic construct
VAKKKPEWLMRTVSVPVRFWPSDVGGDGRLVLDDKGEPVPTHTRQQMWAACGEAWKLSTELANWAGRELLRADVSPPHPGKLPAMPKVYLYGLLTPLLKERWAGQLASANCVLRAVERAYRAKRFEVQARCSAAPAAFRYPYPFRVHNQIWSVHVPADAEMNAGEHPVCTLTLPGIGRVHLPLSRASGHRRALALLRRIAAGDPTVKKGELTVTRQRDGDRNGGHGTDGGPDRAKRAWTIMLRFSVGTRPAENDGTQTMNLVTDPEALLVCWLVGRKDWVVNDDHVRRRIAAHAARRQRLSQDRKAERRLRRGVGIQARLDLECEKHERFMDTYLHQTAAAVAGYAVRNRVGCVFADLSPSGYVDSFPWFKLRERIGNRLAREGVELVDDKWAGSNETSTPEED

SEQ ID NO: 26 - protein, 517 aa, synthetic construct
LEDTSKNVFQSPLLLSKTAETYTPIGYEEAVAITFYYAEDNRRKPGFLRRTGERITLVAPLNYALYIIDIDGRNSVIIDPNKGSELEITYYKPLISLIEEKIEKLRTAETKEFIDILTELKQVLQGMASDKAGVEKYSIRISNILKNRPLIEELKILVRNASENIYEALRIEEKKIDLQGTKNNIREALILLSETRKKLVNLLGEINPIHEKWLEEIRTSYAEKIHEIEQKLEEVKKDVDEKINELKKKQAEEIKNIREKYIGQIETLERRMNEINTKLGQLKTQYEKAKEYGEDTRMIKKRINDLTKKLSDLNKEKKELKEKMNSEMEAVRSKYLEYINAERMRIDKLKKEIEKLNDELESIEKQAGDRLDEIRSLINQLIDKASRAESKLLSIMINTPPHGEGAHYLPVMIITYKSKNKSRRDSFTPAYISVGKLSRTPKISFFEEVRKYLSDIPSILSDARYADQVEKYNLLKTVNPSRIISLLDRLADNGIINRKKVQKIAEKIVEQIKMAQA

SEQ ID NO: 27 - protein, 731 aa, synthetic construct
MAENTNKLPVIGTAYFKDIEGYAAFWKAKDHDWVKTQRKELPPLIYPVDKTHNGVVVKALYRWLYEYWSMSQLTEEELHRRVQDQANEQMKQLREAVYFSETYQQPFQVRALFDFGAYITLGNADFFVFEHEKYLSEITYPKDYSQYTLGELRAIASGVSAGSTVPATLSNEISISQAKDSIQAAKNRLEEMKKEAENLQWERHEELAELKRQAEEAMAKLRQRKSELLDMLEQKREELEDKIEAMNDQVFFLESQIYCIECYLGETVNFAKVRSGRNAPDDEPIVLYQKQRFLDEEMGRLASVYELDFSELNLFEEFLAASPAALEVFAPNERCVTLVRLSKTSLEYGLHPKWANMLKAYDKFHGKMVGIIIRNGENIYIGWTDDDKVIVTDDLFLDFTPAEEVPSDIPVDETERQMKARMRKERAQMRVFAKEAVSRVFIFNILQGIVDNSPILPLPKGEKITKESKYVRFSMADRWLADNRFGSFTDIVSRCNAQFSEGDMLLTTQYLRPENGKHTKNDRGRGYADRTHDVSVQNCAIYPLNLIEYDRPKQVTEYQFKMPACGNTPERWVTSTTDGDGSRLDPKDTRIIRTYTKRDAHYFVSLEKKWSYSGARANFEVFPDEVLNLHYMNSVWLMYAITNRNLGGWRVGGESVDYAFAIRYLKTALDFIRKREADEKMVLDEVAPGFTDRNPEWPVALSEWKLEKKARSFTPVLAKRFVNWAKEREKG

SEQ ID NO: 28 - protein, 491 aa, synthetic construct
MLRRSVAVELEVTKDLNKLFYSVETAYLSIVREVVEYAVANNVTGANKLQRLFYNKYRLEYPSLNSQLIIQAIRQASEIARSFLRRKRKGLVDKPYPEVRRVSIRFSEMAWSYEEFVKSVAPVRLGLSLPNGRMEVWLRPHKRFWQYWWRVLIGEAELASTLMIKRRLNRWYAVFIFELKPRVEKPQSIIAFDINENTVVVGRIDIETTVGKVVDWNRQYVTPQLYMIRTDFGRLARRYEAIRNKIIEKLKPEFALPSGNYVNVANTREFRKRVKRLREGDRKIGRVRQVANELTKTPSIIITEELGENPQESMIEDVGKDELRHRIKQTPFKALVRAVEDKALERGSKLFHVSSYRNSRVCPIHFTRLGETNDWHTLQCPKGHYMHRDYASVTNMAWKLTPESWIKAFWWNMKKDMNWREHEGKSNPLIPHPIVHHLHATLREFMASLEKSPAVLARGNPMNPAGRADEDWARETTRPPGREGGRCRVCG

SEQ ID NO: 29 - protein, 517 aa, synthetic construct
LEETSKKAFQSPLLLSRTAETYTPIGYEEAIAITFYYAEDNRRKPGFLRRTGERITLVAPINYALYIVDIDGRNSIIIDPNKGSELVITYYKPITSLIEEKIYKLRAAESKEFIDILTELKQVLQGMTNDKSGVEKYSIRISNIVKDRTLIEELKILVRNASENIYEALRIEEKKIDLLETKKNIREALILLSDTRKKLVKLLGEINPIHEKWLEEIRTSYAEKIHEIEQKLEEVKKEVDERINELKKKQAEEIKSIREKYIGQIETLERRINEINAKLEQLKAQYEKAKEYGEDTKMIKKRINDLSKKLSDLIKEKKELEEKMNSEIEAVRSKYLEYINAERMRIDKLKKEIEKLNNELDSIEKQAGDRIDEIRALINQLIDKASKAENGIVSIMINTPPHGEGLHYLPVMIITYRSKNKSRRDSFTPAYISTGKLSRTPKISFFEEVRKYLSDIPGILSDARYADQVEKYNLLKTVNPTRIISLLDRLADNGIINRKKVQKIAEKIVEQIKMVQA

SEQ ID NO: 30 - protein, 664 aa, synthetic construct
MIDMVKEGIKEDLVKLYDNISSSSVVEDFYFPIIASNPKFYSTSGLQHYLGTAFLAFRISQHLSLDDYSSATAFLSGLLHDANKWGIPQDEIVKRFENTKLFSIFSEFFGEEKTKKIIKDSMEIAKTLERGGSSRNLQKISEAVRISDYISGDERSWKISRVIDILRNSSLINIGYEHIYPIYLGRQRLVTVYLSHLVKDELIERGMIPLITSSEGMIFLRRSSVSITYDDVIKRMIPLLSSGFRRSKTKSPDASKLVRALEDCKMNLSRSYESLSGYDYDDLLEGLEEAKISRIDHINYLLTLIYVLQRPEGKEHREKREKIFRKISEILNTNLSSSKLCETLITIRDVLMKSDDDFIRRFEEKILEMIREEMREKEVKPDLLRRKISRYISLPREEDVSEDNITRRCPVCGEEILEARPLSAFLKELKKIVGKINTVEIFLPGIQGSPDRPGSIEKLGHKTDVCETCFFEIKELMPRLGLADGLWSAVLTYYPNISIDLADVISNSIKTIVGLDKSSESYKIVPDYMSGRILVGISVRGKGLDKKALSNALKVWLIFGGNMFITTNPLTSPPLIDAPIRLEVGDMIFLECSSKYLEILKKASAYSSYLSFTSQMRYWLFTSLLRYVSSLETTSSGSDAMFRRSFGYTTGFCTLDVLSSESIR

SEQ ID NO: 31 - protein, 1276 aa, synthetic construct
MIYNSLLLNSGGGIIPQFQKSAQSKEAAVLAIGIGGTGVRALSRLKQKVYQQLKSDNEEDDSAVKLYKHIQFLAIDSDETDFKQIRGEAKINADTEFISIQDPALNTIISHNDKKPILDDPRLNWMDIDHITALLAPHGAGGVRQLGRYMIIKKAQRLSTLISGKINLAMENMPNDNVHVYIFAGISGGTGSGCFLDTCYIVRKALKDLGIGGNGKIMGFFFLPDVVTSKREVAANRELVLYNESNGYAAIKELDYLMNLRSAKERFKQVYDEGFVVDTDEPPVDMCHLISAKKADGTVITDGFKYCIHVAADYVMSYLAVVDGNNLEADDTGLTMSGHLANVTAGVGLLPKDAGVNLNYHILGAANAEIPMTQIATYLTTGFIRRFHELVGVKTVTVTKDTVNSFAENIGLSVDDLIEYIHRSNNYPNVQIPDADYQTIYEIGSDNPGVYPRVWVQPRDKAIDSLRGVITYLKNALTSVPDDLDVEKLTANGGESLQVKIFLELCKISAEEEKGPYFASAILGQGGYNLINYIEGQIRQVGEYIQTANKDLYFAQDQAYKAQAEIFKNNGIFANKKKLAKNYKDCVQDWFNYEVEIEELKGAERILETLRISLRNQLKDGFFSKLINMLDNIKDTFKENGDYLNSLRSTQTDAYTIRLVQLTEVRDTLDEAIKKMQPNQLVTDFINRLLKSPKKWLSNDDTQIGQFISTYMQEIFNVEMNKSIQTYLQEKYPDVAGTTELTELVKSTIISELNDKAQPMFWKNPIFNMGASFSTGRMSVPAASNVICNAASSFVENKADKNYTVRKTGINDRVFVLRFHSGLPFYAYQGVTKMYESYRSVANAMPGVGAHLYAKTGRGSGIDDSGMHDWRNELPTPMPYSKVPEFTPNGEELEKLYVKAEEEKVIMPVDINAQPVNYKICYSEKIVKKEFKKEDYLLASGEFNLQKWDEDKKWLENELNRRITRPEKVIDDFADGAADSPVVQRRIHIDYFIHYKYYQKIVLDELESREYLKKAMKRLDDIKKELELYINEVNRYNDIILFGFINCLNATGKFDINRYRIKSINYKYEDKFGVAREEIFAKINDDSEFSSEPLYRGFLHYCKMNPDEEPRRSIDNMLNERKSSTLKAGRDTFIAYQFETNWNKDILADMEIEIKGKLTNEQQEDVKRYYRFMITKVQELKKQFLLNEWQLNPEDENRVEPKKETIRFNENTNTTQEFSNTWECPECGFRKNIGNFCSGCGKAKPKAEVSATWECPECGFRKNIGNFCSGCGRKRD

SEQ ID NO: 32 - protein, 548 aa, synthetic construct
MSDINDIKFKTGWLKDPKDNQKFAPKTTTNQVLTGDGERLTDTLATFITNAADDLKNYYLKSETYTQDEVNELISLIPKFKLEVVASLDDLSATDINEATVYLVSNKSTSGSNVYTEYVYKNNRWEILGEQKLDLSGYVTEEYINNNFEDKNVIKQKLDVVTELVNNNLEAANDYTDEVKEQLSNYETKEAASNKLTEAKQFATNEASKIKNDLLNGAGAAYDTLKELGDLIDESVDAVEALKIIATNKADKEHTHEFTAKYDITTLTELQNASTAGKNIKVVRNFERPIPGAYDENDTMLYSWQELLDMDVEYEEFDGFDETGANVWVTKIDKCLTVEDGALKSIVTYSPSTHSYTNWSIDALTGVTKLVINEGVTAIGPSGLAAFNVAEIIMPSTLTTIEDDALSHIFEYWDWGDYSVTVHIPKAVNNISFNAFSYSKVFIKYEGTETEFNTIASVADFNLNSYEFNYSCNYNLVPAPIYGYIKNKLEDRFIFTAHEDDGEIEYVCNSSGWSTRNIQMMKLGDAVFKYDYDNARIILSFPMEGAVG

SEQ ID NO: 33 - protein, 1138 aa, synthetic construct
MTYRVVGCSECQSLWLLEDTDDESATCPTCGTRHQRHRLRTLAQADDKDGANQQRSALLAERADAGDADLDPYWEQATRASEPIVDDRAYLDGLGIDPNLVEDLTSEDDDTSASEQTTRTPGIGPDVPAPVADRPQLRGPVDDARSPGVSLIEAGGQLGIAGQTYHEVSPRTFEWLADVVSDLVPSTARLVQDLARERYNFDYRDPDAGAGAVATFIHEELVGRVAQLDTADAPTAAVEEARSYLDAIGRYALLWADDVYRVRRGFDGAEQFEHITRTLETTGTSQGQFNAGVDALRHSLVALHAERAVPRTLTFVLDGEQWTGADRETIKRALTAVDALAAGFDVRLWMSPGVRQRVRRLTSTALDDDDAPTWAERFAFLTDAGQTSRRSPEATASSTSADEAEEAWAFVEDNRTQTGLLTLLAQLDADSERSVRALKRDTQIDYADASIDRYVADLEAAGLVAIDRSHASNRLSLTALGIAAQNYVTPTGDVVHRYQSRLVGASYGHPSASHKYSVAPQGTGGDHHPPAERWLADTGDPAEDGYVQFLGDSTGPREIEPPVFHRRMLAGERVSGVNFADADLIDWTNERQAPTGDGRVTYASIFDDHALLITQWGGPAQTMARLCAGLLGNRMLSKALSVDAVGTQFEQTHGGVKAFENDLHDVLVRAQQIGWLSEDELEHYDNWRDRIGAVRSNILSKIGELDELDSGLRRELFRDLQGLLTSATHLYYAAGIDVTINLRLPRTTELLANDEALQHFLDFMRFTVTKQAGYEDENGFHSWYRMCIEDRKEKLKARAAYDVDEADSTADLTASWIISGPGATALKDHVQEAIGEESSRLRERVDEGVEDAATLDIPMVEANSHGHIRGLVREIADRKGFYETNRRDLDRLTRCLEAALATNDRGPDPFLVADALAALESRDTARDRLDTLSVQNALATLPSEAVFPTLPPAARRMLSALFASDEPLDRQALIEVTSESSYDRHWKTLRAFFLVEETDDGFVAQLEPWWASTNEERKPFHEDHPNPVTQPPGGHIKQHAPPTRPYGVIFEIANETDFFEIPPDRYYEFGQRWDEIEWILDELDLERLRPILKAYCADWPDYTAQSYSDPSGVQIAPQQPDSPSTQATLATAATINRQ

SEQ ID NO: 34 - protein, 408 aa, synthetic construct
MELTLLLIIAALLVALLVLTLTRNNRAQSEEMQRALRQQMQENREELNRSIRELRMEMTQTLNQGLQQLQDAMHKNMMTTGELQRQKFDAMARQQETLIQSTEKRLDDMRVMVEEKLQKTLNERIGQSFEIVRSQLENVQKGLGEMKSLAQDVGGLKKVLSNVKMRGTFGEVQLGALLEQMMSPEQYEANVKTKKSGTEFVEFAIKLPGNDDANSTVYLPIDAKFPKDVYEQYYDAFEAGDAALMESCGRQLETTIKKMAKDIHDKYVDPPFTTDFAILFLPFESIYAEVIRRTSLVETLQKDYKIVVTGPTTLGAILNSLQMGFRTLAIQKRTGEVWTVLGAVKTEFGKFGGLLEKVQKNLQSAGDQLEEVMGKRTRAIERKLRQVEELPHEESRRILPIDDGGEDD

SEQ ID NO: 35 - protein, 408 aa, synthetic construct
MELTLLLIIAALLVALLALTLTRNNRAQSEEMQRALRQQMQENREELNRSIRELRMEMTQTLNQGLQQLQDAMHKNMMTTGELQRQKFDAMARQQETLIQSTEKRLDDMRVMVEEKLQKTLNERIGQSFEIVRSQLENVQKGLGEMKSLAQDVGGLKKVLSNVKMRGTFGEVQLGALLEQMMSPEQYEANVKTKKSGTEFVEFAIKLPGKDDANSTVYLPIDAKFPKDVYEQYYDAFEAGDAALMESCGRQLETTIKKMAKDIHDKYVDPPFTTDFAILFLPFESIYAEVIRRTSLVETLQKDYKIVVTGPTTLGAILNSLQMGFRTLAIQKRTGEVWTVLGAVKTEFGKFGGLLEKVQKNLQSAGDQLEEVMGKRTRAIERKLRQVEELPHEESRRILPIDDGGEDD

SEQ ID NO: 36 - protein, 408 aa, synthetic construct
MELTLLLIIAALLVALLVLTLTRNNRAQSEEMQRALRQQMQENREELNRSIRELRMEMTQTLNQGLQQLQDAMHKNMMTTGELQRQKFDAMARQQETLLQSTEKRLDDMRVMVEEKLQKTLNERIGQSFEIVRSQLENVQKGLGEMKSLAQDVGGLKKVLSNVKMRGTFGEVQLGALLEQMMSPEQYEANVKTKKSGTEFVEFAIKLPGKDDANSTVYLPIDAKFPKDVYEQYYDAFEAGDAALMESCGRQLETTIKKMAKDIHDKYVDPPFTTDFAILFLPFESIYAEVIRRTSLVETLQKDYKIVVTGPTTLGAILNSLQMGFRTLAIQKRTGEVWTVLGAVKTEFGKFGGLLEKVQKNLQSAGDQLEEVMGKRTRAIERKLRQVEELPHEESRRILPIDDGGEDD

SEQ ID NO: 37 - protein, 408 aa, synthetic construct
MELTLLLIIAALLVALLVLTLTRNNRAQSEEMQRALRQQMQENREELNRSIRELRMEMTQTLNQGLQQLQDAMHKNMMTTGELQRQKFDAMARQQETLIQSTEKRLDDMRVMVEEKLQKTLNERIGQSFEIVRSQLENVQKGLGEMKSLAQDVGGLKKVLSNVKMRGTFGEVQLGALLEQMMSPEQYEANVKTKKSGTEFVEFAIKLPGNDDANSTVYLPIDAKFPKDVYEQYYDAFEAGDAALMESCGRQLETTIKKMAKDIHDKYVDPPFTTDFAILFLPFESIYAEVIRRTSLVETLQKDYKIVVTGPTTLGAILNSLQMGFRTLAIQKRTGEVWTVLGAVKTEFGNFGGLLEKVQKNLQSAGDQLEEVMGKRTRAIERKLRQVEELPHEESRRILPIDDGGEDD

SEQ ID NO: 38 - protein, 681 aa, synthetic construct
MGSECIYIFRAYRDGRLSDILRDLDRCDSASTVLFTISEYRMVRLRYASEQGYMAGRLLTAYISLKGYAPVTRNILYEWVSRMLAVSSREKAEHNIELLWRDRQIVNLQKNAVEEVIRELSKEGLENLAINPPKPIQKVLETLIKCPRCGSQPSYGEKYCKQCGARIPTKAWETTEETHKPITVEIEQKAGTPTIECPHCGKALRQGAKYCTKCGSSIVSPAHKGMKIREIFRKIQQDVSRKTTPEEPAPELGREVSPESAEKPTLTTFKEPVKSEEKPSQVEEHVKPTAEKPAAEREPRTPTDVGEKPQPQQPAPPTRGVTAPEPVPAGVDWEPDEDMVEAFDDMGVPLEAFRREAIRLALLDVDERVFEREVMRSASKLATSVEGLNRDFRDQLTLSISQYLRDAVFIIRKEIKRPETPRPTVPEHIISEKPAQPALEPPKHVIQQPKPPEQLEKRAPTVESAKQQPPKMDGIELWTLVREGPKPGHVYLLDLPRSALPTSIISKMFEGVVNVEEVDYVGPDTPVALTRTTYRANYISLIKPSPTNPYANKLYRIVEMRCGSCIITTLETYFMNRYVFDSRGLKPFKIILDIEASRKALEKVMHPQYAARLAKLGALLPWLAEELASNGLDGVRNRLHGLLSPEDGEEVYQAIKGVLENDMRYVNKALAISLGIIDEEE

SEQ ID NO: 39 - protein, 444 aa, synthetic construct
MATRIKAIKCPHCGSSNHRQTGEKRFVCNNCGTEFFLDDDDINININHYNHNSDAPLLSMDSDNAKKLKAALLIFFPVLILFFFISSLFHTSPISDKAGKDSIRVREEYLLVQTFAKEDTYIVFCISDRNYYADYNNKSKKQPTNGIYYMFRNVRTGEIVKEGLLISDEQKGDRAFYTFGDNVKLRRFANTRRWYLIIGNRLVYEVNPKRMTLVDAAPQLMSAQKALSSGFAAIGFINKNEAEGFAIQNNLGKIYYYCPATNHLYTKVAFDYATALPANEMPGQCRDSTYYLLQNASSEESENITRIWRVTYKHFNGDPEDRIDRIDDWYLDRLSRYRISEIKPVSSWFISFHPTIIYQDRQHILLQYEATMAPNSPVTLQLRGTDGRVKWTRTLNRELNRTSAEKSSVGYIITTWPYSFIEISNNGKQLTEYTLPEEYQIKAK

SEQ ID NO: 40 - protein, 507 aa, synthetic construct
MSNFCSICGKEFKSSRVGQKACSECLKSEFSVASKMEEEEVEMYRAKQAAAARRQHARMAKLLDSYKNGTMFNMSGKIMFCVGLFILLFCHLIFFLDGRELIYWGVEGMDESGKKAISMLLSFACVLLLVFSTRRFKIVMMLGSVVILLLGWYATAIWKSSSDAMTGGGIVEKKQLPEPGNEAVIPITEEELGVFYELKKNYPRATHYAVFLDNQEPIVRDLVREALTRLLEAEYTRAYTRSNGVLYVVANAAGVPRNVSPIVDRLGEIVNADVAKGLYLVRFDAEKTNLVCKYSSEVLSSPLNSSFVIANINELRCLDAMRIRVAARSLRNANVQMLRREVRDALVRVLGDSWTQDQDTYSALIDSLVTYASAKDREVINICSDYFMKRYGAKKDVLPGVVDYLIKEVPDQMVQPIIDYWLLNPMSWTVQMRNLSWRVQPKLLERMEQEVSIKDLSLILRYLQNNGNEDAIPAVKKLLTHSDAIIRFSAQETLRELESKASEKIEE

SEQ ID NO: 41 - protein, 507 aa, synthetic construct
MSNFCSICGKEFKSSRVGQKACSECLKSEFSAASKMEEEEVEMYRAKQAAAARRQHARMAKLLDSYKNGTMFNMSGKIMFCVGLFILLFCHLIFFLDGRELIYWGVEGMDESGKKAISMLLSFACVLLLVFSTRRFKIVMMLGSVVILLLGWYATAIWKSSSDAMAGGGIVEKKQLPEPGNEAVIPITEEELGVFYELKKNYPRATHYAVFLDNQEPIVRDLVREALTRLLEAEYTRAYTRSNGVLYVVANAAGVPRNVSPIVDRLGEIVNADVAKGLYLVRFDAEKTNLVCKYSSEVLSSPLNSSFVIANINELRCLDAMRIRVAARSLRNANVQMLRREVRDALVRVLGDSWTQDQDTYSALIDSLVTYASAKDREVINICSDYFMKRYGAKKDVLPGVVDYLIKEVPDQMVQPIIDYWLLNPMSWTVQMRNLSWRVQPKLLERMEQEVSIKDLSLILRYLQNNGNEDAIPAVKKLLTHSDAIIRFSAQETLRELESKASEKIEE

SEQ ID NO: 42 - protein, 765 aa, synthetic construct
MALTIIGKARFYNFAGFATWHEALTREQAQKLWQSSICSRQNELGKAYDNVYTNFNAFGFDSGNQERRKRLQKFQDYLELTDQPWDVRYVDHVAKFMVISYGQCDDNTKGKENQFLIENWPEYIEYTPFTDFSAVPMSQLRQITMLGCEGITGGTSLIPQNAGINLSVADVRRGISAQEQALADLQAKVKAVEEGKTEELSPLKKQIDELMAQMNALQEKKKAELSAMKAELEAKKKEMEKQIFILEAEIYSIRCFLGETIQFVKLRSGSNAPLEQPVILYQKLRFMVEDLQKFAIMWPEEKIGKSIEAALKASDSLMDAFAPSTKCITLIRYSETGKVFRAHEEELNILDEYELMHGNQLAILIRNGENLYIGWADEDKITLKDNFFLKPTEAKMEAMPEQRPNESDEYYQARLERMQKDMEEANKKAAREGLSRHFLFSILNGVSASDNSILPLPKFSNKAERNQHIIFSMADGALVDRRFGSFGNIVKRCNSVVKKGDMILTTMSLRAEGPYWSKPGQYTTWYNDRGRGERNRTHDVHASDCTIYPVNLVEFDKPERKVRYRSTYTIPEEVNGEYRQVKRTSIHVTDADAKLSEDVEILEYFDYIQQHTFISLQKEGGWWKCDVGPSYANFEVNTDEFINLTYMNSVWLNYVLSCRDLSGWRVGGTTVNYEYALRYLKKALSHIREREKTEEENIRLAGGAAILADPDWPVALSEWKMDKGVRNMTEYQAKRFVKAMLAGEIDITPKPVAEGDVEMYDAVIV

SEQ ID NO: 43 - protein, 516 aa, synthetic construct
MVDAAARSPGRLLVFVHIPKTAGTTLRTVLGMNEPGARSRALGNVFKGGGGISKSLIDRLRKDKGPDLSGVGLIRGHFPLGIREHLPRYLPRGREVACFTFLREPADRTLSHYFAIREHGRGYQLPPLPAEATVEDALERGYIHDNVQTRMLSGLAEPFGEVDQEMLERAKDNLREELVFFGLTERFDESLVLAKRRLGFRSILYKTSGRVNVNRARGDEVPAELREAAQACNRYDIELYRYAEQLFETAPERQELEFDAELAALRAAKANGDGESTSISVPASYGGDEQAWTMLVEARAELLRLEFERRRHRVPHVAATVQDEVRESELKAARTRTKKLEQEVERLKTAQAKTKRLEQQVERLKAASSRVEELEREVERLNAVASRAEELEQRLEQQVEHLNAASAKTEKFEQQVERLKAARSRNRKLQQEVERLKTAVARTEELEEEVQRLETAAAKAEGLEEEVERLKTAASRAEELEHELEQQLKLLDAARSRKTKLEQKVERLRDAAAVRE

SEQ ID NO: 44 - protein, 1123 aa, synthetic construct
MDKTALEPTRTYHATVDLGENTEAFLAHHVATNNAAGELAGALKHMIATLVPAQWVELWENHAGTPAGVRIASWIAGSWVGTERSDSAPPRTVTHAQAIDAVRRRAVELRPGIDAEQFLKDAAILHGTVRDDAVWVDYLDGDPVPAIGWEGLDVRLLGSASEPVKSNDEITKPGKGDMVQSCSRLWGRAVGTGRKADGLLLVERSAALRDAAADPTNRTVADVAQALTGQPLDGAGLAAWANHTNPKSPTKVTAALVGNDASADLSTEVAGKTLRDRIVTGASEVHANWVARTGEARRAADGEILAGTWLHGILLRHMAANLTGGARTNVLSAAASTVATHRDRLHKQAVELAALQQSLANALEQVDPDDLADLDAWARAHLYENEDSPGYLLPRIPRREGTAKLATVTNKWRNKPKMGVEERVAAAKGAGAGWTVWWDYLARNEHLWNPNTDRLLRVVGGGDGFAGVQPLRRKIAGVQMPTFARPHPQAAPAPSYYGGGRLTGRLGADGTLVLQVATPDGLARISARWMSTRLREALKVGAQVVDGQPTITRDDPTSRLAAGVDQDTPVNVAADPTSSTFTVGYDRENQRWLLAVAIKHHTPRRYLPGDPLRLMGVQIGMNRHDVTYAVWETVDGVSAPQDVEVADVHAVNARGQATVRRARRVAATGNLFEFARPVREGSIDLPAGDRESQVGESAQIAELLDDLPVHDAYIQGELRRVARDAAVDLGAGTPRSQLLQAAMRVLNRALDAQGCLARLAGQARGLGEAGPDDLEELESIWPATGGDLGALWSQRAATIARYARIVRDDLLTRAHSRRVSVERVVELDEFARLLRRLETCPTPSRPFEHRTLPFGFAPTIRTMRNRAREAWTDKIASDTVKTALRLGVSVIAVYKDEDSTPSQVRPAHINRRLATEARRAIADQIALVAPLHGIEVKVVSKGVGHRARVVDGREMFAVTPITLGEFADLARRDTKGAKGAIASWDNRVVAAANLLAGKEKKRKGRDGRVYEESAQRKAANLAVAALTVQAGQFLDRELEPVLGLNDRAFRTWRSSAAASQTLHLPGLFPDGQVLVPADAQYEPGTLRFRSVSSRDIAIAHAVAHRGCTWVLNPKKQKKDDESE

SEQ ID NO: 45 - protein, 1073 aa, synthetic construct
VRPAVRNYNVAAGAHKQERDERTYIKGAFGSFSREEDNRASTQFLRPAGSQHYSAILASFTDENRDDTFTLAVLLYLNSEGGADKVYCFANGERSIAADCSRIETVEKLRQQMEWRGFHATTTYTEYYGWFRRKTGVQFKAMDVFNQTVAVKDIKSLNQFVREHMLEAKPWSEKVDSLLNHFTQLHEAHQSLLRVQRQFQLLEPVGEAGEVYRVHAEKLESVRRLIDATDSFFRQKTVDILGPSAKEWKDLRHAVGRQRERLDQDIREVLEECRRLQNEIEQAGGDRLRQIPLLIKQHESNAATKRTANGHYHGALAAASIRETVADAEGFARIQAQIPQLVRDLDQQIEETDKRKEDLVIERATLNQSIRNDETELESLKQRQGNLPHALVTVRQTICTDLQLPERELPFVAELVAVKPEEQAWEASAELALRTFALSLLVPHRHYPLVAGFVDRTRITDAAGAGQRLVYLRVGDRAKVAAQAALHPQSLIRKLTFRDGHPLLPWVKGELEDRFDYRCCETLEEFQEAHGLAMTRHRHLKIRGVRHEKDDRDRVADPRFYVLGWNNSDKKRRLVERIREHQESRTQLNKRIEGIDAKLAALRTRHEALRKAGEVADFGEIDYRVHEWELEALRLEKKQLEENNDAIRLLQGRLADAESRHTGLRASRDDALLKEAKLTDEISQAEKLVANAETVLHERQVSGALQHHASSFPDLDACFIEQTLTAATLLAEERRFIDARRAECDRLGREIEPKKLDLTRAMSRYLREFQDDRADLEAQAEYLDSFLDLRDHIRKEDLPRHEKRFKAHLNEKVIQEIGILNGTFQSERSEIITRINQLNASLRQLEYRPGTHMVLEPRAVRDGDIVDFQNALRECLAGTFEGSPEADEARFIRIEKPITRLREEQTWREKVTDVRRWFDFAARELENVTNKERSYHEDSAGQSGGEKAKLAFTILVAAIAYQYDIDPDHPTSSRFHFVVVDEMFSKVDDQYSEYALELFKKFGLQLLIVAPLDAKALVTEPYVGCYLHAVKDPRTNRSEVFTMSAREFADTLSAAGQGQKNAMGPAPVKVRSR

SEQ ID NO: 46 - protein, 1118 aa, synthetic construct
MKTDDEKKDTAIKSYTSWLLPNDRKEKDMVRSFLALDQGSRFFFDLMQAWYGGLTPDIIKSVTKERDLVDLWCAIYWFRPMKKELASHPIDRVDLAKTFQRYYGGPASDVVQEYLSASIGEDCCWNDCRQKYQEFCKNLGVDFTPDLKTLVREKLIAVALNDGSQAAISNLFGNGGKEDRNVKVNICKKILIALEKAGKSVKYVRDVQSIILKCANAKDREDFNRIYADKNGRPGTLLLLLDRKGENTYDAEVLKRYLRKTIKSKNAPLVWNYNQKLFEYIERGIRNLLRRTINYDAWAWGEMWRVGHTPLQTKATRNYHFAQEQLKRHSDIAAASQSSHAIAVALNEFFESPFFDGENPFTICPHHLGKNLEKLFKAWADEKNQTDEEDAGETAITDYCAEFKDGFDREPIRNLLRYVYASLRSKYSAKELIQAAKYNQQFERYQRQKAHPVTPDNQGYTWPEAVIKPSKAERKNRENSLDTRIWVSVKLLQKDGTWEKHHIPFYNLRFFEEVYAAASIAEDMPSPTFRNSRFGFKLPKLLNTHAKINKKKKDGKKDKKAVNAAKREARIYLAAKEGRLPAPSVPLDKLSAVIARVNGKFQVTVPVKFKVNKQPKYPLPQLGQIILGYDQNLTANHAWALFEVVTEDTPGAHFCRNQYLRVLKTGQVRSITKTKDGQEIDQLSYDGLEYKEYGEWRKQAKKFASQWYITTKVRKGKETTLLSQPALERFESIEKYKPALYRFNKEYARLLLAVIRRKTLNELEEIRPEIFRLVEQGFGICRFGSLSLSSFEAIRAAKAVIYGYFSTALKHDHNTPITDDERQAFDPELFGLLNKLETLRQNKGEEKINRAANALIRIALENKADFIRGEGDLPTTNKSVKKGQNSRSMDWLARGLFNKICQLAVMHNIIPTAANPHSTSHQDPFEHNKDFDDPQPAMKCRYAEFKIEDIGDSVLERLGTSLRNAKAGQTGAYYYKGAQDFLAHYGLQDIEEELKKCRRGRKANMPCWELQKRLIQKLGSKDAVVYIPMRGGRIYLATHSVTTGAKPIIFNGEEVWVSNADEIAAVNIGLTIIPTSKKDEEHPDRENDDKAIRKSVRRPRKSGERRSGDKMPATARKT

SEQ ID NO: 47 - protein, 640 aa, synthetic construct
MDTGIEEYSSIHKDEYDRDPIVDLYRHIYPHREVISAKNFIDAAVLNKLLRLNASRHVHPTVFGKTVISFSPKSSAYGRITPPSEIVRGRPAGSHGMIWLTMELFDDGKWIEHHLPFHNSRYYEEVYCYQEGLPVKDEPRSPMFGYRVGNAIADTSKIDNRRRKASKQFLRAQQNITHNVSFDENTAFSVVRNGEDFSITISSRIKASNAKSLMTIGDRIMGIDQNQTAANTYSIWEVVGDGDAGSIQHGNLSLKRIEDGHITSIIRGRGGNFDQLNYGGLSYAKFSEWRSARLGFISSLNAELASKMNWDWCCLYEWNARYASALRKIIYSHKGIDIERVFRREIEDFVEGVLRIGSLSSDALQCLTNAKSLISSYFFLNGKKEPEEQRKFDQGLFDLSAKIDKKRVNKRQQKTKRIMSSIMQIARDRGVSFIVVEGKLSTATKDNKSKANQKAIDWCARAVVENLEHSCSLVGIKLVAIDPMNTSHLDPFVYVLKTSLGKEARFASVVPAKINARHMKNFKSWSSLLAGNGKIKKTTDAIYVGAFQDFCREYGFVAEDISKMSQSEIQDKLSSHQFVLVPQRGGRVYMSTHPVSSEAKKIVYAGRERWYNNADVVAAVNITLRGCERLSASRKTASTR

SEQ ID NO: 48 - protein, 1018 aa, synthetic construct
IFPTQRRNTMSGNVVRSYKSVLRPNIRKRELLDATFNWFDRAYKKFFDVFVCLYGGVEHDTVHSALLKETTDPDLVCATMWFRVVPKSSCDGISAQEMIRRFGVYAGHEPSAVAMSYLTGNFDDKKNHWIDCREKFVALARDMVVKPESLSIDIKSMIEHKILPICSQDNWQAWNAISQLFGEGKKENKAEKAQIFVDVVSMLSNNSVQTWEDYKEVISKATGCRTAGEINSKFGGRPGILSVDFSKDDTGSLPKDFIERRIKDLSQKAKEKSAAYELPNRMRLRELIASVIGPYRLETWSSVAQRACGDIRSKNSNNLLYASERFNRTKEIEEILSAKGDVARAQGQFRSGEFNEFAVEKRHLGNLESLYNIWSKSDMDTGIEEYSSIHKDEYDRDPIVDLYRHIYPHREVISAKNFIDAAVLNKLLRLNASRHVHPTVFGKTVISFSPKSSAYGRITPPSEIVRGRPAGSHGMIWLTMELFDDGKWIEHHLPFHNSRYYEEVYCYQEGLPVKDEPRSPMFGYRVGNAIADTSKIDNRRRKASKQFLRAQQNITHNVSFDENTAFSVVRNGEDFSITISSRIKASNAKSLMTIGDRIMGIDQNQTAANTYSIWEVVGDGDAGSIQHGNLSLKRIEDGHITSIIRGRGGNFDQLNYGGLSYAKFSEWRSARLGFISSLNAELASKMNWDWCCLYEWNARYASALRKIIYSHKGIDIERVFRREIEDFVEGVLRIGSLSSDALQCLTNAKSLISSYFFLNGKKEPEEQRKFDQGLFDLSAKIDKKRVNKRQQKTKRIMSSIMQIARDRGVSFIVVEGKLSTATKDNKSKANQKAIDWCARAVVENLEHSCSLVGIKLVAIDPMNTSHLDPFVYVLKTSLGKEARFASVVPAKINARHMKNFKSWSSLLAGNGKIKKTTDAIYVGAFQDFCREYGFVAEDISKMSQSEIQDKLSSHQFVLVPQRGGRVYMSTHPVSSEAKKIVYAGRERWYNNADVVAAVNITLRGCERLSASRKTASTR

SEQ ID NO: 49 - protein, 1035 aa, synthetic construct
IFPTQRRNTMSGNVVRSYKSVLRPNIRKRELLDATFNWFDRAYKKFFDVFVCLYGGVEHDTVHSALLKETTDPDLVCATMWFRVVPKSSCDGISAQEMIRRFGVYAGHEPSAVAMSYLTGNFDDKKNHWIDCREKFVALARDMVVKPESLSIDIKSMIEHKILPICSQDNWQAWNAISQLFGEGKKENKAEKAQIFVDVVSMLSNNSVQTWEDYKEVISKATGCRTAGEINSKFGGRPGILSVDFSKDDTGSLPKDFIERRIKDLSQKAKEKSAAYELPNRMRLRELIASVIGPYRLETWSSVAQRACGDIRSKNSNNLLYASERFNRTKEIEEILSAKGDVARAQTNEKAKDILNKINDNLIGQFRSGEFNEFAVEKRHLGNLESLYNIWSKSDMDTGIEEYSSIHKDEYDRDPIVDLYRHIYPHREVISAKNFIDAAVLNKLLRLNASRHVHPTVFGKTVISFSPKSSAYGRITPPSEIVRGRPAGSHGMIWLTMELFDDGKWIEHHLPFHNSRYYEEVYCYQEGLPVKDEPRSPMFGYRVGNAIADTSKIDNRRRKASKQFLRAQQNITHNVSFDENTAFSVVRNGEDFSITISSRIKASNAKSLMTIGDRIMGIDQNQTAANTYSIWEVVGDGDAGSIQHGNLSLKRIEDGHITSIIRGRGGNFDQLNYGGLSYAKFSEWRSARLGFISSLNAELASKMNWDWCCLYEWNARYASALRKIIYSHKGIDIERVFRREIEDFVEGVLRIGSLSSDALQCLTNAKSLISSYFFLNGKKEPEEQRKFDQGLFDLSAKIDKKRVNKRQQKTKRIMSSIMQIARDRGVSFIVVEGKLSTATKDNKSKANQKAIDWCARAVVENLEHSCSLVGIKLVAIDPMNTSHLDPFVYVLKTSLGKEARFASVVPAKINARHMKNFKSWSSLLAGNGKIKKTTDAIYVGAFQDFCREYGFVAEDISKMSQSEIQDKLSSHQFVLVPQRGGRVYMSTHPVSSEAKKIVYAGRERWYNNADVVAAVNITLRGCERLSASRKTASTR

SEQ ID NO: 50 - protein, 1037 aa, synthetic construct
IFPTQRRNTMSGNVVRSYKSVLRPNIRKRELLDATFNWFDRAYKKFFDVFVCLYGGVEHDTVHSALLKETTDPDLVCATMWFRVVPKSSCDGISAQEMIRRFGVYAGHEPSAVAMSYLTGNFDDKKNHWIDCREKFVALARDMVVKPESLSIDIKSMIEHKILPICSQDNWQAWNAISQLFGEGKKENKAEKAQIFVDVVSMLSNNSVQTWEDYKEVISKATGCRTAGEINSKFGGRPGILSVDFSKDDTGSLPKDFIERRIKDLSQKAKEKSAAYELPNRMRLRELIASVIGPYRLETWSSVAQRACGDIRSKNSNNLLYASERFNRTKEIEEILSAKGDVARAQKEDILSAANILNDFRRGEFGQFRSGEFNEFAVEKRHLGNLESLYNIWSKSDMDTGIEEYSSIHKDEYDRDPIVDLYRHIYPHREVISAKNFIDAAVLNKLLRLNASRHVHPTVFGKTVISFSPKSSAYGRITPPSEIVRGRPAGSHGMIWLTMELFDDGKWIEHHLPFHNSRYYEEVYCYQEGLPVKDEPRSPMFGYRVGNAIADTSKIDNRRRKASKQFLRAQQNITHNVSFDENTAFSVVRNGEDFSITISSRIKASNAKSLMTIGDRIMGIDQNQTAANTYSIWEVVGDGDAGSIQHGNLSLKRIEDGHITSIIRGRGGNFDQLNYGGLSYAKFSEWRSARLGFISSLNAELASKMNWDWCCLYEWNARYASALRKIIYSHKGIDIERVFRREIEDFVEGVLRIGSLSSDALQCLTNAKSLISSYFFLNGKKEPEEQRKFDQGLFDLSAKIDKKRVNKRQQKTKRIMSSIMQIARDRGVSFIVVEGKLSTATKDNKSKANQKAIDWCARAVVENLEHSCSLVGIKLVAIDPMNTSHLDPFVYVLKTSLGKEARFASVVPAKINARHMKNFKSWSSLLAGNGKIKKTTDAIYVGAFQDFCREYGFVAEDISKMSQSEIQDKLSSHQFVLVPQRGGRVYMSTHPVSSEAKKIVYAGRERWYNNADVVAAVNITLRGCERLSASRKTASTR

SEQ ID NO: 51 - protein, 1041 aa, synthetic construct
IFPTQRRNTMSGNVVRSYKSVLRPNIRKRELLDATFNWFDRAYKKFFDVFVCLYGGVEHDTVHSALLKETTDPDLVCATMWFRVVPKSSCDGISAQEMIRRFGVYAGHEPSAVAMSYLTGNFDDKKNHWIDCREKFVALARDMVVKPESLSIDIKSMIEHKILPICSQDNWQAWNAISQLFGEGKKENKAEKAQIFVDVVSMLSNNSVQTWEDYKEVISKATGCRTAGEINSKFGGRPGILSVDFSKDDTGSLPKDFIERRIKDLSQKAKEKSAAYELPNRMRLRELIASVIGPYRLETWSSVAQRACGDIRSKNSNNLLYASERFNRTKEIEEILSAKGDVARAQKDILLAASILGDFRRGEFNRSVVGQFRSGEFNEFAVEKRHLGNLESLYNIWSKSDMDTGIEEYSSIHKDEYDRDPIVDLYRHIYPHREVISAKNFIDAAVLNKLLRLNASRHVHPTVFGKTVISFSPKSSAYGRITPPSEIVRGRPAGSHGMIWLTMELFDDGKWIEHHLPFHNSRYYEEVYCYQEGLPVKDEPRSPMFGYRVGNAIADTSKIDNRRRKASKQFLRAQQNITHNVSFDENTAFSVVRNGEDFSITISSRIKASNAKSLMTIGDRIMGIDQNQTAANTYSIWEVVGDGDAGSIQHGNLSLKRIEDGHITSIIRGRGGNFDQLNYGGLSYAKFSEWRSARLGFISSLNAELASKMNWDWCCLYEWNARYASALRKIIYSHKGIDIERVFRREIEDFVEGVLRIGSLSSDALQCLTNAKSLISSYFFLNGKKEPEEQRKFDQGLFDLSAKIDKKRVNKRQQKTKRIMSSIMQIARDRGVSFIVVEGKLSTATKDNKSKANQKAIDWCARAVVENLEHSCSLVGIKLVAIDPMNTSHLDPFVYVLKTSLGKEARFASVVPAKINARHMKNFKSWSSLLAGNGKIKKTTDAIYVGAFQDFCREYGFVAEDISKMSQSEIQDKLSSHQFVLVPQRGGRVYMSTHPVSSEAKKIVYAGRERWYNNADVVAAVNITLRGCERLSASRKTASTR

SEQ ID NO: 52 - protein, 1021 aa, synthetic construct
IFPTQRRNTMSGNVVRSYKSVLRPNIRKRELLDATFNWFDRAYKKFFDVFVCLYGGVEHDTVHSALLKETTDPDLVCATMWFRVVPKSSCDGISAQEMIRRFGVYAGHEPSAVAMSYLTGNFDDKKNHWIDCREKFVALARDMVVKPESLSIDIKSMIEHKILPICSQDNWQAWNAISQLFGEGKKENKAEKAQIFVDVVSMLSNNSVQTWEDYKEVISKATGCRTAGEINSKFGGRPGILSVDFSKDDTGSLPKDFIERRIKDLSQKAKEKSAAYELPNRMRLRELIASVIGPYRLETWSSVAQRACGDIRSKNSNNLLYASERFNRTKEIEEILSAKGDVARAQNILGQFRSGEFNEFAVEKRHLGNLESLYNIWSKSDMDTGIEEYSSIHKDEYDRDPIVDLYRHIYPHREVISAKNFIDAAVLNKLLRLNASRHVHPTVFGKTVISFSPKSSAYGRITPPSEIVRGRPAGSHGMIWLTMELFDDGKWIEHHLPFHNSRYYEEVYCYQEGLPVKDEPRSPMFGYRVGNAIADTSKIDNRRRKASKQFLRAQQNITHNVSFDENTAFSVVRNGEDFSITISSRIKASNAKSLMTIGDRIMGIDQNQTAANTYSIWEVVGDGDAGSIQHGNLSLKRIEDGHITSIIRGRGGNFDQLNYGGLSYAKFSEWRSARLGFISSLNAELASKMNWDWCCLYEWNARYASALRKIIYSHKGIDIERVFRREIEDFVEGVLRIGSLSSDALQCLTNAKSLISSYFFLNGKKEPEEQRKFDQGLFDLSAKIDKKRVNKRQQKTKRIMSSIMQIARDRGVSFIVVEGKLSTATKDNKSKANQKAIDWCARAVVENLEHSCSLVGIKLVAIDPMNTSHLDPFVYVLKTSLGKEARFASVVPAKINARHMKNFKSWSSLLAGNGKIKKTTDAIYVGAFQDFCREYGFVAEDISKMSQSEIQDKLSSHQFVLVPQRGGRVYMSTHPVSSEAKKIVYAGRERWYNNADVVAAVNITLRGCERLSASRKTASTR

SEQ ID NO: 53 - protein, 933 aa, synthetic construct
MSIVAEPESVADAAEAAPKKKKSDYFTTTRSASLKSTVNPAFEMYEAFQRDFRKNIEILFPWLGIGYGVPDADAKGGIRYVGPEEAVAARNASLPSAKAVAIVERFVTCLSKNAKTLSSCYSLYYKHYKPTGAKRGESVKKIEKLLESDSFSDLAKSHPGIDWQAAKLVPKDKLWGHLKPQLTDKNREIGREVRQFVTLPCSYPEACDYCKLLWSAVLAFLQSRLEIYQYHMDGTAALKTAFDKGNTPLYAAFVQYTDAVAAMLGNSLSPREILHVIECAKGRKIAERPHLQLAIDELKKPAYALLLAAETATVKRCFATRTVAAKLKKRKAYPTKSALDKDQTMNVGSPMFSIPDTSPVSPTKHITVTVTVNGEQVEFPCKHTEYLANLTLEKVSPKKGEAYYKMGFNTNHKARTLGELKTVSIQKRGGNFYVTLPYTITHPVANFNLAWRFFQAASPKMENLVLPDQVVCASYDLGINNPVTGCLFKIGRDLQGPIKARGYGEGYILKLPTYLTSSGSQKNGSAYCQAVVALRNKLGLFHDAMKGLKIHRNTGFPMLEDEVEFLRSAPNMSEKSRQHVAKKNDLRLCVSYWMGFLNAERKRLNYELRATGYKDQVGELIRNIELDDIYYKVRSRYDSLDVSRETPRRYDTSRANRKVNANRLIASAIARDCLANGVWIVFVENLASKYAKGSANLLAKLFNASTLLDTIKAALDKIGVALVRVEKNGTSQHDPVTGALGYRDDTNHENLIVSRDGELCSIPCDKSASLCVGLVGVNHSVVPHKFYVPKPDAEAEAEEEEEEDGGSKRLTAFLADAGKTLKDLKNLTAGPGGVVRFTSDPTAKRIAGQSVYPCHATGKLYTAAAKDAIQDGIRNRCKAGEVPRPAEVIPDGAKTYKAFSTGLVLELAQPSGDQELENIVLPKKRSRSRRVRD

SEQ ID NO: 54 - RNA, 36 nt, synthetic construct
  source 1..36: mol_type = other RNA
gtgcttttactcatttctagcgaactgaataagcac

SEQ ID NO: 55 - RNA, 36 nt, synthetic construct
  source 1..36: mol_type = other RNA
gtgcttattcagttcgctagaaatgagtaaaagcac

SEQ ID NO: 56 - RNA, 36 nt, synthetic construct
  source 1..36: mol_type = other RNA
gtgcttttactcatttctaacgaattgaataagcac

SEQ ID NO: 57 - RNA, 36 nt, synthetic construct
  source 1..36: mol_type = other RNA
gtgcttattcaattcgttagaaatgagtaaaagcac

SEQ ID NO: 58 - RNA, 36 nt, synthetic construct
  source 1..36: mol_type = other RNA
gtgcttttactcatttctagcgaattgaataagcac

SEQ ID NO: 59 - RNA, 36 nt, synthetic construct
  source 1..36: mol_type = other RNA
gtgcttattcaattcgctagaaatgagtaaaagcac

SEQ ID NO: 60 - RNA, 36 nt, synthetic construct
  source 1..36: mol_type = other RNA
gtgcttttacccgtttctagcgaattggataagcac

SEQ ID NO: 61 - RNA, 36 nt, synthetic construct
  source 1..36: mol_type = other RNA
gtgcttatccaattcgctagaaacgggtaaaagcac

SEQ ID NO: 62 - RNA, 36 nt, synthetic construct
  source 1..36: mol_type = other RNA
gtgcttttacttatttctaacgaattaaataagcac

SEQ ID NO: 63 - RNA, 36 nt, synthetic construct
  source 1..36: mol_type = other RNA
gtgcttatttaattcgttagaaataagtaaaagcac

SEQ ID NO: 64 - RNA, 36 nt, synthetic construct
  source 1..36: mol_type = other RNA
gtgtttttacccatttctagcgaattggataagcac

SEQ ID NO: 65 - RNA, 36 nt, synthetic construct
  source 1..36: mol_type = other RNA
gtgcttatccaattcgctagaaatgggtaaaaacac

SEQ ID NO: 66 - RNA, 36 nt, synthetic construct
  source 1..36: mol_type = other RNA
gtgcttttactcatttctaacgaattgaacaagcac

SEQ ID NO: 67 - RNA, 36 nt, synthetic construct
  source 1..36: mol_type = other RNA
gtgcttgttcaattcgttagaaatgagtaaaagcac

SEQ ID NO: 68 - RNA, 36 nt, synthetic construct
  source 1..36: mol_type = other RNA
gtgcttttactcatttctaacgaactgaataagcac

SEQ ID NO: 69 - RNA, 36 nt, synthetic construct
  source 1..36: mol_type = other RNA
gtgcttattcagttcgttagaaatgagtaaaagcac

SEQ ID NO: 70 - RNA, 36 nt, synthetic construct
  source 1..36: mol_type = other RNA
gtgtttttattcatttctagcgaactgaataagcac

SEQ ID NO: 71 - RNA, 36 nt, synthetic construct
  source 1..36: mol_type = other RNA
gtgcttattcagttcgctagaaatgaataaaaacac

SEQ ID NO: 72 - RNA, 36 nt, synthetic construct
  source 1..36: mol_type = other RNA
gtgcttttactcacttctaacgaattaaataagcac

SEQ ID NO: 73 - RNA, 36 nt, synthetic construct
  source 1..36: mol_type = other RNA
gtgcttatttaattcgttagaagtgagtaaaagcac

SEQ ID NO: 74 - RNA, 36 nt, synthetic construct
  source 1..36: mol_type = other RNA
gtgcttttactcatttctaacgaatcgaataagcac

SEQ ID NO: 75 - RNA, 36 nt, synthetic construct
  source 1..36: mol_type = other RNA
gtgcttattcgattcgttagaaatgagtaaaagcac

SEQ ID NO: 76 - RNA, 36 nt, synthetic construct
  source 1..36: mol_type = other RNA
gtgcttttatccatttctaacgaattgaataagcac

SEQ ID NO: 77 - RNA, 36 nt, synthetic construct
  source 1..36: mol_type = other RNA
gtgcttattcaattcgttagaaatggataaaagcac

SEQ ID NO: 78 - RNA, 36 nt, synthetic construct
  source 1..36: mol_type = other RNA
gttacaatacctagaggttttaccactagattgtac

SEQ ID NO: 79 - RNA, 36 nt, synthetic construct
  source 1..36: mol_type = other RNA
gtacaatctagtggtaaaacctctaggtattgtaac

SEQ ID NO: 80 - RNA, 36 nt, synthetic construct
  source 1..36: mol_type = other RNA
gttacaatacctagaggtctttccaataggttgtac

SEQ ID NO: 81 - RNA, 36 nt, synthetic construct
  source 1..36: mol_type = other RNA
gtacaacctattggaaagacctctaggtattgtaac

SEQ ID NO: 82 - RNA, 31 nt, synthetic construct
  source 1..31: mol_type = other RNA
gttgcgaacacatggcatctagcgttgccat

SEQ ID NO: 83 - RNA, 31 nt, synthetic construct
  source 1..31: mol_type = other RNA
atggcaacgctagatgccatgtgttcgcaac

SEQ ID NO: 84 - RNA, 31 nt, synthetic construct
  source 1..31: mol_type = other RNA
gttgcgaacacatggcatctagcgttgccac

SEQ ID NO: 85 - RNA, 31 nt, synthetic construct
  source 1..31: mol_type = other RNA
gtggcaacgctagatgccatgtgttcgcaac

SEQ ID NO: 86 - RNA, 31 nt, synthetic construct
  source 1..31: mol_type = other RNA
gttgcgaacagatggcatctagcgttgccat

SEQ ID NO: 87 - RNA, 31 nt, synthetic construct
  source 1..31: mol_type = other RNA
atggcaacgctagatgccatctgttcgcaac

SEQ ID NO: 88 - RNA, 40 nt, synthetic construct
  source 1..40: mol_type = other RNA
tgttgcgaacacatggcatctagcgttgccatgcagcaca

SEQ ID NO: 89 - RNA, 40 nt, synthetic construct
  source 1..40: mol_type = other RNA
tgtgctgcatggcaacgctagatgccatgtgttcgcaaca

SEQ ID NO: 90 - RNA, 36 nt, synthetic construct
  source 1..36: mol_type = other RNA
gtgctggcgacctgctacggcggatcgccaaggcac

SEQ ID NO: 91 - RNA, 36 nt, synthetic construct
  source 1..36: mol_type = other RNA
gtgccttggcgatccgccgtagcaggtcgccagcac

SEQ ID NO: 92 - RNA, 36 nt, synthetic construct
  source 1..36: mol_type = other RNA
gtgctggcgacctgctacggtggatcgccaaggcac

SEQ ID NO: 93 - RNA, 36 nt, synthetic construct
  source 1..36: mol_type = other RNA
gtgccttggcgatccaccgtagcaggtcgccagcac

SEQ ID NO: 94 - RNA, 37 nt, synthetic construct
  source 1..37: mol_type = other RNA
agtgctggttctcgtcgctaggggagagtcaaagcac

SEQ ID NO: 95 - RNA, 37 nt, synthetic construct
  source 1..37: mol_type = other RNA
gtgctttgactctcccctagcgacgagaaccagcact

SEQ ID NO: 96 - RNA, 37 nt, synthetic construct
  source 1..37: mol_type = other RNA
ggtacaatctagtggtaaaacctctaggtattgtaac

SEQ ID NO: 97 - RNA, 37 nt, synthetic construct
  source 1..37: mol_type = other RNA
gttacaatacctagaggttttaccactagattgtacc

SEQ ID NO: 98 - RNA, 37 nt, synthetic construct
  source 1..37: mol_type = other RNA
agtacaacctattggaaagacctctaggtattgtaac

SEQ ID NO: 99 - RNA, 37 nt, synthetic construct
  source 1..37: mol_type = other RNA
gttacaatacctagaggtctttccaataggttgtact

SEQ ID NO: 100 - RNA, 37 nt, synthetic construct
  source 1..37: mol_type = other RNA
tgtacaatctagtggtaaaacctctaggtattgtaac

SEQ ID NO: 101 - RNA, 37 nt, synthetic construct
  source 1..37: mol_type = other RNA
gttacaatacctagaggttttaccactagattgtaca

SEQ ID NO: 102 - RNA, 36 nt, synthetic construct
  source 1..36: mol_type = other RNA
gctgcatggcaacgctagatgccatgtgttcgcaac

SEQ ID NO: 103 - RNA, 36 nt, synthetic construct
  source 1..36: mol_type = other RNA
gttgcgaacacatggcatctagcgttgccatgcagc

SEQ ID NO: 104 - RNA, 36 nt, synthetic construct
  source 1..36: mol_type = other RNA
gctgcgtggcaacgctagatgccatgtgttcgcaac

SEQ ID NO: 105 - RNA, 36 nt, synthetic construct
  source 1..36: mol_type = other RNA
gttgcgaacacatggcatctagcgttgccacgcagc

SEQ ID NO: 106 - RNA, 36 nt, synthetic construct
  source 1..36: mol_type = other RNA
gctgtatggcaacgctagatgccatctgttcgcaac

SEQ ID NO: 107 - RNA, 36 nt, synthetic construct
  source 1..36: mol_type = other RNA
gttgcgaacagatggcatctagcgttgccatacagc

SEQ ID NO: 108 - RNA, 30 nt, synthetic construct
  source 1..30: mol_type = other RNA
tggcaacgctagatgccatgtgttcgcaac

SEQ ID NO: 109 - RNA, 30 nt, synthetic construct
  source 1..30: mol_type = other RNA
gttgcgaacacatggcatctagcgttgcca

SEQ ID NO: 110 - RNA, 30 nt, synthetic construct
  source 1..30: mol_type = other RNA
tggcaacgctagatgccatctgttcgcaac

SEQ ID NO: 111 - RNA, 30 nt, synthetic construct
  source 1..30: mol_type = other RNA
gttgcgaacagatggcatctagcgttgcca

SEQ ID NO: 112 - RNA, 36 nt, synthetic construct
  source 1..36: mol_type = other RNA
gtgctgttccttcccgtcagagaaggaagagggcac

SEQ ID NO: 113 - RNA, 36 nt, synthetic construct
  source 1..36: mol_type = other RNA
gtgccctcttccttctctgacgggaaggaacagcac

SEQ ID NO: 114 - RNA, 33 nt, synthetic construct
  source 1..33: mol_type = other RNA
ctgttccttcccgtcagagaaggaagagggcac

SEQ ID NO: 115 - RNA, 33 nt, synthetic construct
  source 1..33: mol_type = other RNA
gtgccctcttccttctctgacgggaaggaacag

SEQ ID NO: 116 - RNA, 36 nt, synthetic construct
  source 1..36: mol_type = other RNA
atagcaatttcatctaatgccgttaggcgttgagca

SEQ ID NO: 117 - RNA, 36 nt, synthetic construct
  source 1..36: mol_type = other RNA
tgctcaacgcctaacggcattagatgaaattgctat

SEQ ID NO: 118 - RNA, 29 nt, synthetic construct
  source 1..29: mol_type = other RNA
ccccaagcccgcatgcgcgtgggctggac

SEQ ID NO: 119 - RNA, 29 nt, synthetic construct
  source 1..29: mol_type = other RNA
gtccagcccacgcgcatgcgggcttgggg

SEQ ID NO: 120 - RNA, 29 nt, synthetic construct
  source 1..29: mol_type = other RNA
taaaaggcccacattcgcgtgggctggac

SEQ ID NO: 121 - RNA, 29 nt, synthetic construct
  source 1..29: mol_type = other RNA
gtccagcccacgcgaatgtgggcctttta

SEQ ID NO: 122 - RNA, 29 nt, synthetic construct
  source 1..29: mol_type = other RNA
ccccaagccctcgcgcacgtgggccggac

SEQ ID NO: 123 - RNA, 29 nt, synthetic construct
  source 1..29: mol_type = other RNA
gtccggcccacgtgcgcgagggcttgggg

SEQ ID NO: 124 - RNA, 29 nt, synthetic construct
  source 1..29: mol_type = other RNA
ccccaaaccctcgcgcacgtgggctggac

SEQ ID NO: 125 - RNA, 29 nt, synthetic construct
  source 1..29: mol_type = other RNA
gtccagcccacgtgcgcgagggtttgggg

SEQ ID NO: 126 - RNA, 30 nt, synthetic construct
  source 1..30: mol_type = other RNA
ccccaagccctcgcgcacgtgggccggact

SEQ ID NO: 127 - RNA, 30 nt, synthetic construct
  source 1..30: mol_type = other RNA
agtccggcccacgtgcgcgagggcttgggg

SEQ ID NO: 128 - RNA, 23 nt, synthetic construct
  source 1..23: mol_type = other RNA
ccgaccacccccgcccgcgtggg

SEQ ID NO: 129 - RNA, 23 nt, synthetic construct
  source 1..23: mol_type = other RNA
cccacgcgggcgggggtggtcgg

SEQ ID NO: 130 - RNA, 23 nt, synthetic construct
  source 1..23: mol_type = other RNA
acgaccacccccgcccgcgtggg

SEQ ID NO: 131 - RNA, 23 nt, synthetic construct
  source 1..23: mol_type = other RNA
cccacgcgggcgggggtggtcgt

SEQ ID NO: 132 - RNA, 23 nt, synthetic construct
  source 1..23: mol_type = other RNA
gcaaacacactagcccgcgtggg

SEQ ID NO: 133 - RNA, 23 nt, synthetic construct
  source 1..23: mol_type = other RNA
cccacgcgggctagtgtgtttgc

SEQ ID NO: 134 - RNA, 23 nt, synthetic construct
  source 1..23: mol_type = other RNA
gcgaccacccccgcccgcgtggg

SEQ ID NO: 135 - RNA, 23 nt, synthetic construct
  source 1..23: mol_type = other RNA
cccacgcgggcgggggtggtcgc

SEQ ID NO: 136 - RNA, 29 nt, synthetic construct
  source 1..29: mol_type = other RNA
ccgaccacccccgcccgcgtgggcttgac

SEQ ID NO: 137 - RNA, 29 nt, synthetic construct
  source 1..29: mol_type = other RNA
gtcaagcccacgcgggcgggggtggtcgg

SEQ ID NO: 138 - RNA, 23 nt, synthetic construct
  source 1..23: mol_type = other RNA
caaccaaccaccgaccgcgtggg

SEQ ID NO: 139 - RNA, 23 nt, synthetic construct
  source 1..23: mol_type = other RNA
cccacgcggtcggtggttggttg

SEQ ID NO: 140 - RNA, 23 nt, synthetic construct
  source 1..23: mol_type = other RNA
ccgaccacccccgccagcgtggg

SEQ ID NO: 141 - RNA, 23 nt, synthetic construct
  source 1..23: mol_type = other RNA
cccacgctggcgggggtggtcgg

SEQ ID NO: 142 - RNA, 37 nt, synthetic construct
  source 1..37: mol_type = other RNA
gttggattcagccataaaatccagtaggtataaaacc

SEQ ID NO: 143 - RNA, 37 nt, synthetic construct
  source 1..37: mol_type = other RNA
ggttttatacctactggattttatggctgaatccaac

SEQ ID NO: 144 - RNA, 37 nt, synthetic construct
  source 1..37: mol_type = other RNA
gttggattcagccataaaatccagtaggtataaaact

SEQ ID NO: 145 - RNA, 37 nt, synthetic construct
  source 1..37: mol_type = other RNA
agttttatacctactggattttatggctgaatccaac

SEQ ID NO: 146 - RNA, 32 nt, synthetic construct
  source 1..32: mol_type = other RNA
gattcagccataaaatccagtaggtataaaac

SEQ ID NO: 147 - RNA, 32 nt, synthetic construct
  source 1..32: mol_type = other RNA
gttttatacctactggattttatggctgaatc

SEQ ID NO: 148 - RNA, 36 nt, synthetic construct
  source 1..36: mol_type = other RNA
gttggattcagccataaaatccagtaggtataaaac

SEQ ID NO: 149 - RNA, 36 nt, synthetic construct
  source 1..36: mol_type = other RNA
gttttatacctactggattttatggctgaatccaac

SEQ ID NO: 150 - RNA, 32 nt, synthetic construct
  source 1..32: mol_type = other RNA
gattcagccttcaaatccagttgttttctatt

SEQ ID NO: 151 - RNA, 32 nt, synthetic construct
  source 1..32: mol_type = other RNA
aatagaaaacaactggatttgaaggctgaatc

SEQ ID NO: 152 - RNA, 32 nt, synthetic construct
  source 1..32: mol_type = other RNA
gattcagcctacaaatccagtaggtgtaaaac

SEQ ID NO: 153 - RNA, 32 nt, synthetic construct
  source 1..32: mol_type = other RNA
gttttacacctactggatttgtaggctgaatc

SEQ ID NO: 154 - RNA, 32 nt, synthetic construct
  source 1..32: mol_type = other RNA
gattcagtcataaaatccagtaggtataaaac

SEQ ID NO: 155 - RNA, 32 nt, synthetic construct
  source 1..32: mol_type = other RNA
gttttatacctactggattttatgactgaatc

SEQ ID NO: 156 - RNA, 38 nt, synthetic construct
  source 1..38: mol_type = other RNA
gttggattcagccataaaatccagtaggtataaaaccg

SEQ ID NO: 157 - RNA, 38 nt, synthetic construct
  source 1..38: mol_type = other RNA
cggttttatacctactggattttatggctgaatccaac

SEQ ID NO: 158 - RNA, 23 nt, synthetic construct
  source 1..23: mol_type = other RNA
gttggattcagccataaaatcca

SEQ ID NO: 159 - RNA, 23 nt, synthetic construct
  source 1..23: mol_type = other RNA
tggattttatggctgaatccaac

SEQ ID NO: 160 - RNA, 23 nt, synthetic construct
  source 1..23: mol_type = other RNA
gttggattcagcctacaaatcca

SEQ ID NO: 161 - RNA, 23 nt, synthetic construct
  source 1..23: mol_type = other RNA
tggatttgtaggctgaatccaac

SEQ ID NO: 162 - RNA, 23 nt, synthetic construct
  source 1..23: mol_type = other RNA
gttggattcagtcataaaatcca

SEQ ID NO: 163 - RNA, 23 nt, synthetic construct
  source 1..23: mol_type = other RNA
tggattttatgactgaatccaac

SEQ ID NO: 164 - RNA, 23 nt, synthetic construct
  source 1..23: mol_type = other RNA
tggatttgaaggttgaatccaac

SEQ ID NO: 165 - RNA, 23 nt, synthetic construct
  source 1..23: mol_type = other RNA
gttggattcaaccttcaaatcca

SEQ ID NO: 166 - RNA, 23 nt, synthetic construct
  source 1..23: mol_type = other RNA
tgggtttgagggctgaatccaag

SEQ ID NO: 167 - RNA, 23 nt, synthetic construct
  source 1..23: mol_type = other RNA
cttggattcagccctcaaaccca

SEQ ID NO: 168 - RNA, 23 nt, synthetic construct
  source 1..23: mol_type = other RNA
tggatttgtagactgaatccaac

SEQ ID NO: 169 - RNA, 23 nt, synthetic construct
  source 1..23: mol_type = other RNA
gttggattcagtctacaaatcca

SEQ ID NO: 170 - RNA, 23 nt, synthetic construct
  source 1..23: mol_type = other RNA
tgactttgagggctgaagccaac

SEQ ID NO: 171 - RNA, 23 nt, synthetic construct
  source 1..23: mol_type = other RNA
gttggcttcagccctcaaagtca

SEQ ID NO: 172 - RNA, 42 nt, synthetic construct
  source 1..42: mol_type = other RNA
ggttttatacctactggattttatggctgaatccaaccgagc

SEQ ID NO: 173 - RNA, 42 nt, synthetic construct
  source 1..42: mol_type = other RNA
gctcggttggattcagccataaaatccagtaggtataaaacc

SEQ ID NO: 174 - RNA, 36 nt, synthetic construct
  source 1..36: mol_type = other RNA
cttccagagcctcccgatcggcttcgtagatcagac

SEQ ID NO: 175 - RNA, 36 nt, synthetic construct
  source 1..36: mol_type = other RNA
gtctgatctacgaagccgatcgggaggctctggaag

SEQ ID NO: 176 - RNA, 36 nt, synthetic construct
  source 1..36: mol_type = other RNA
tctccagagcctcccgatcggcttcgtagatcagac

SEQ ID NO: 177 - RNA, 36 nt, synthetic construct
  source 1..36: mol_type = other RNA
gtctgatctacgaagccgatcgggaggctctggaga

SEQ ID NO: 178 - RNA, 36 nt, synthetic construct
  source 1..36: mol_type = other RNA
cttccagagccttccgatcggcttcgtagatcagac

SEQ ID NO: 179 - RNA, 36 nt, synthetic construct
  source 1..36: mol_type = other RNA
gtctgatctacgaagccgatcggaaggctctggaag

SEQ ID NO: 180 - RNA, 36 nt, synthetic construct
  source 1..36: mol_type = other RNA
cttccagagcctcccgatcggcttcataggtcggac

SEQ ID NO: 181 - RNA, 36 nt, synthetic construct
  source 1..36: mol_type = other RNA
gtccgacctatgaagccgatcgggaggctctggaag

SEQ ID NO: 182 - RNA, 36 nt, synthetic construct
  source 1..36: mol_type = other RNA
cttccagagccccctgatcggcttcgtagatcagac

SEQ ID NO: 183 - RNA, 36 nt, synthetic construct
  source 1..36: mol_type = other RNA
gtctgatctacgaagccgatcagggggctctggaag

SEQ ID NO: 184 - RNA, 36 nt, synthetic construct
  source 1..36: mol_type = other RNA
cttccaaagcctcccgatcggcttcgtagatcagac

SEQ ID NO: 185 - RNA, 36 nt, synthetic construct
  source 1..36: mol_type = other RNA
gtctgatctacgaagccgatcgggaggctttggaag

SEQ ID NO: 186 - RNA, 36 nt, synthetic construct
  source 1..36: mol_type = other RNA
cttccagagcctcctgttcggcttcgtagatcagaa

SEQ ID NO: 187 - RNA, 36 nt, synthetic construct
  source 1..36: mol_type = other RNA
ttctgatctacgaagccgaacaggaggctctggaag

SEQ ID NO: 188 - RNA, 36 nt, synthetic construct
  source 1..36: mol_type = other RNA
cttccagagcctcctgatcggcttcgtaggtcagac

SEQ ID NO: 189 - RNA, 36 nt, synthetic construct
  source 1..36: mol_type = other RNA
gtctgacctacgaagccgatcaggaggctctggaag

SEQ ID NO: 190 - RNA, 36 nt, synthetic construct
  source 1..36: mol_type = other RNA
cttccagagccttctgatcggttcggtgctgggact

SEQ ID NO: 191 - RNA, 36 nt, synthetic construct
  source 1..36: mol_type = other RNA
agtcccagcaccgaaccgatcagaaggctctggaag

SEQ ID NO: 192 - RNA, 34 nt, synthetic construct
  source 1..34: mol_type = other RNA
tccagagcctcccgatcggcttcgtagatcagac

SEQ ID NO: 193 - RNA, 34 nt, synthetic construct
  source 1..34: mol_type = other RNA
gtctgatctacgaagccgatcgggaggctctgga

SEQ ID NO: 194 - RNA, 34 nt, synthetic construct
  source 1..34: mol_type = other RNA
tccagagccttccgatcggcttcgtagatcagac

SEQ ID NO: 195 - RNA, 34 nt, synthetic construct
  source 1..34: mol_type = other RNA
gtctgatctacgaagccgatcggaaggctctgga

SEQ ID NO: 196 - RNA, 34 nt, synthetic construct
  source 1..34: mol_type = other RNA
tccagagcctcccgatcggcttcataggtcggac

SEQ ID NO: 197 - RNA, 34 nt, synthetic construct
  source 1..34: mol_type = other RNA
gtccgacctatgaagccgatcgggaggctctgga

SEQ ID NO: 198 - RNA, 34 nt, synthetic construct
  source 1..34: mol_type = other RNA
tccagagccccctgatcggcttcgtagatcagac

SEQ ID NO: 199 - RNA, 34 nt, synthetic construct
  source 1..34: mol_type = other RNA
gtctgatctacgaagccgatcagggggctctgga

SEQ ID NO: 200 - RNA, 34 nt, synthetic construct
  source 1..34: mol_type = other RNA
tccaaagcctcccgatcggcttcgtagatcagac

SEQ ID NO: 201 - RNA, 34 nt, synthetic construct
  source 1..34: mol_type = other RNA
gtctgatctacgaagccgatcgggaggctttgga

SEQ ID NO: 202 - RNA, 34 nt, synthetic construct
  source 1..34: mol_type = other RNA
tccagagcctcctgttcggcttcgtagatcagaa

SEQ ID NO: 203 - RNA, 34 nt, synthetic construct
  source 1..34: mol_type = other RNA
ttctgatctacgaagccgaacaggaggctctgga

SEQ ID NO: 204 - RNA, 34 nt, synthetic construct
  source 1..34: mol_type = other RNA
tccagagcctcctgatcggcttcgtaggtcagac

SEQ ID NO: 205 - RNA, 34 nt, synthetic construct
  source 1..34: mol_type = other RNA
gtctgacctacgaagccgatcaggaggctctgga

SEQ ID NO: 206 - RNA, 30 nt, synthetic construct
  source 1..30: mol_type = other RNA
atttaaatagaaccatagtggaatgtaaat

SEQ ID NO: 207 - RNA, 30 nt, synthetic construct
  source 1..30: mol_type = other RNA
atttacattccactatggttctatttaaat

SEQ ID NO: 208 - RNA, 32 nt, synthetic construct
  source 1..32: mol_type = other RNA
ctttgcctccgcgcacacacacggattgcaac

SEQ ID NO: 209 - RNA, 32 nt, synthetic construct
  source 1..32: mol_type = other RNA
gttgcaatccgtgtgtgtgcgcggaggcaaag

SEQ ID NO: 210 - RNA, 32 nt, synthetic construct
  source 1..32: mol_type = other RNA
gtctgcctccgcgcacacacacggattgcaac

SEQ ID NO: 211 - RNA, 32 nt, synthetic construct
  source 1..32: mol_type = other RNA
gttgcaatccgtgtgtgtgcgcggaggcagac

SEQ ID NO: 212 - RNA, 17 nt, synthetic construct
  source 1..17: mol_type = other RNA
gaacatcctgaaccaca

SEQ ID NO: 213 - RNA, 17 nt, synthetic construct
  source 1..17: mol_type = other RNA
tgtggttcaggatgttc

SEQ ID NO: 214 - RNA, 23 nt, synthetic construct
  source 1..23: mol_type = other RNA
attaatttacatcattctcaaac

SEQ ID NO: 215 - RNA, 23 nt, synthetic construct
  source 1..23: mol_type = other RNA
gtttgagaatgatgtaaattaat

SEQ ID NO: 216 - RNA, 23 nt, synthetic construct
  source 1..23: mol_type = other RNA
ttcatattctatcattctcaaac

SEQ ID NO: 217 - RNA, 23 nt, synthetic construct
  source 1..23: mol_type = other RNA
gtttgagaatgatagaatatgaa

SEQ ID NO: 218 - RNA, 32 nt, synthetic construct
  source 1..32: mol_type = other RNA
gtctcaccttacacaggtgagtggattgaaat

SEQ ID NO: 219 - RNA, 32 nt, synthetic construct
  source 1..32: mol_type = other RNA
atttcaatccactcacctgtgtaaggtgagac

SEQ ID NO: 220 - RNA, 32 nt, synthetic construct
  source 1..32: mol_type = other RNA
gtctcaccttacataggtgagtggattgaaat

SEQ ID NO: 221 - RNA, 32 nt, synthetic construct
  source 1..32: mol_type = other RNA
atttcaatccactcacctatgtaaggtgagac

SEQ ID NO: 222 - RNA, 26 nt, synthetic construct
  source 1..26: mol_type = other RNA
tccacggcgttcagcagctagacatt

SEQ ID NO: 223 - RNA, 26 nt, synthetic construct
  source 1..26: mol_type = other RNA
aatgtctagctgctgaacgccgtgga

SEQ ID NO: 224 - RNA, 26 nt, synthetic construct
  source 1..26: mol_type = other RNA
tccacggcgtttagcagctagacatt

SEQ ID NO: 225 - RNA, 26 nt, synthetic construct
  source 1..26: mol_type = other RNA
aatgtctagctgctaaacgccgtgga

SEQ ID NO: 226 - RNA, 36 nt, synthetic construct
  source 1..36: mol_type = other RNA
gtttgagaatgatgtaaattaatatggttcttaatc

SEQ ID NO: 227 - RNA, 36 nt, synthetic construct
  source 1..36: mol_type = other RNA
gattaagaaccatattaatttacatcattctcaaac

SEQ ID NO: 228 - RNA, 36 nt, synthetic construct
  source 1..36: mol_type = other RNA
gtttgagaatgatgtaaatcaatatggttcttaatc

SEQ ID NO: 229 - RNA, 36 nt, synthetic construct
  source 1..36: mol_type = other RNA
gattaagaaccatattgatttacatcattctcaaac

SEQ ID NO: 230 - RNA, 36 nt, synthetic construct
  source 1..36: mol_type = other RNA
gtttgagaatgatgtaattcaatatggttacttaac

SEQ ID NO: 231 - RNA, 36 nt, synthetic construct
  source 1..36: mol_type = other RNA
gttaagtaaccatattgaattacatcattctcaaac

SEQ ID NO: 232 - RNA, 38 nt, synthetic construct
  source 1..38: mol_type = other RNA
agttacaatggcctctgccgtgtagcggcaagtggagg

SEQ ID NO: 233 - RNA, 38 nt, synthetic construct
  source 1..38: mol_type = other RNA
cctccacttgccgctacacggcagaggccattgtaact

SEQ ID NO: 234 - RNA, 38 nt, synthetic construct
  source 1..38: mol_type = other RNA
ggttacaatggcctctgccgtgtagcggcaagtggagg

SEQ ID NO: 235 - RNA, 38 nt, synthetic construct
  source 1..38: mol_type = other RNA
cctccacttgccgctacacggcagaggccattgtaacc

SEQ ID NO: 236 - RNA, 38 nt, synthetic construct
  source 1..38: mol_type = other RNA
cgttacaatggcctctgccgtgtagcggcaagtggagg

SEQ ID NO: 237 - RNA, 38 nt, synthetic construct
  source 1..38: mol_type = other RNA
cctccacttgccgctacacggcagaggccattgtaacg

SEQ ID NO: 238 - RNA, 38 nt, synthetic construct
  source 1..38: mol_type = other RNA
agttacaatggcctctgccgtgtagcggcaagtggagc

SEQ ID NO: 239 - RNA, 38 nt, synthetic construct
  source 1..38: mol_type = other RNA
gctccacttgccgctacacggcagaggccattgtaact

SEQ ID NO: 240 - RNA, 39 nt, synthetic construct
  source 1..39: mol_type = other RNA
gttacaatggcctctgccgtgtagcggcaagtggaggag

SEQ ID NO: 241 - RNA, 39 nt, synthetic construct
  source 1..39: mol_type = other RNA
ctcctccacttgccgctacacggcagaggccattgtaac

SEQ ID NO: 242 - RNA, 36 nt, synthetic construct
  source 1..36: mol_type = other RNA
gtctaatactttatattaatttctactattgtagat

SEQ ID NO: 243 - RNA, 36 nt, synthetic construct
  source 1..36: mol_type = other RNA
atctacaatagtagaaattaatataaagtattagac

SEQ ID NO: 244 - RNA, 35 nt, synthetic construct
  source 1..35: mol_type = other RNA
tctaatactttatattaatttctactattgtagat

SEQ ID NO: 245 - RNA, 35 nt, synthetic construct
  source 1..35: mol_type = other RNA
atctacaatagtagaaattaatataaagtattaga

SEQ ID NO: 246 - RNA, 37 nt, synthetic construct
  source 1..37: mol_type = other RNA
gttgcaatggtcaacagagcgtcgtggcaagtggagg

SEQ ID NO: 247 - RNA, 37 nt, synthetic construct
  source 1..37: mol_type = other RNA
cctccacttgccacgacgctctgttgaccattgcaac

SEQ ID NO: 248 - RNA, 37 nt, synthetic construct
  source 1..37: mol_type = other RNA
gttgcaatgggcaccgtggcatcgcggcaagtggagg

SEQ ID NO: 249 - RNA, 37 nt, synthetic construct
  source 1..37: mol_type = other RNA
cctccacttgccgcgatgccacggtgcccattgcaac

SEQ ID NO: 250 - RNA, 37 nt, synthetic construct
  source 1..37: mol_type = other RNA
cctgccgaacacatccgatcggatctcctgttcgacc

SEQ ID NO: 251 - RNA, 37 nt, synthetic construct
  source 1..37: mol_type = other RNA
ggtcgaacaggagatccgatcggatgtgttcggcagg

SEQ ID NO: 252 - RNA, 37 nt, synthetic construct
  source 1..37: mol_type = other RNA
cctgccgaacacatccgatcggatctcctgttcgacg

SEQ ID NO: 253 - RNA, 37 nt, synthetic construct
  source 1..37: mol_type = other RNA
cgtcgaacaggagatccgatcggatgtgttcggcagg

SEQ ID NO: 254 - RNA, 37 nt, synthetic construct
  source 1..37: mol_type = other RNA
cctgccgaacacatccgatcggatctcctgttcgaca

SEQ ID NO: 255 - RNA, 37 nt, synthetic construct
  source 1..37: mol_type = other RNA
tgtcgaacaggagatccgatcggatgtgttcggcagg

SEQ ID NO: 256 - RNA, 36 nt, synthetic construct
  source 1..36: mol_type = other RNA
cctgccgaacacatccgatcggatctcctgttcgac

SEQ ID NO: 257 - RNA, 36 nt, synthetic construct
  source 1..36: mol_type = other RNA
gtcgaacaggagatccgatcggatgtgttcggcagg

SEQ ID NO: 258 - RNA, 37 nt, synthetic construct
  source 1..37: mol_type = other RNA
atccaaagcacctcaatccccgcgaggggattacgac

SEQ ID NO: 259 - RNA, 37 nt, synthetic construct
  source 1..37: mol_type = other RNA
gtcgtaatcccctcgcggggattgaggtgctttggat

SEQ ID NO: 260 - RNA, 24 nt, synthetic construct
  source 1..24: mol_type = other RNA
ggtaataacgatcagaattggaag

SEQ ID NO: 261 - RNA, 24 nt, synthetic construct
  source 1..24: mol_type = other RNA
cttccaattctgatcgttattacc

SEQ ID NO: 262 - RNA, 24 nt, synthetic construct
  source 1..24: mol_type = other RNA
ggtagtaacgatcagaatttgaaa

SEQ ID NO: 263 - RNA, 24 nt, synthetic construct
  source 1..24: mol_type = other RNA
tttcaaattctgatcgttactacc

SEQ ID NO: 264 - RNA, 24 nt, synthetic construct
  source 1..24: mol_type = other RNA
ctttcagttcttcctagttgttac

SEQ ID NO: 265 - RNA, 24 nt, synthetic construct
  source 1..24: mol_type = other RNA
gtaacaactaggaagaactgaaag

SEQ ID NO: 266 - RNA, 24 nt, synthetic construct
  source 1..24: mol_type = other RNA
cttccaattctgatcgttgttacc

SEQ ID NO: 267 - RNA, 24 nt, synthetic construct
  source 1..24: mol_type = other RNA
ggtaacaacgatcagaattggaag

SEQ ID NO: 268 - RNA, 23 nt, synthetic construct
  source 1..23: mol_type = other RNA
atctgcaacagcagaaattttac

SEQ ID NO: 269 - RNA, 23 nt, synthetic construct
  source 1..23: mol_type = other RNA
gtaaaatttctgctgttgcagat

SEQ ID NO: 270 - RNA, 23 nt, synthetic construct
  source 1..23: mol_type = other RNA
acctgcgatagcaggaattggat

SEQ ID NO: 271 - RNA, 23 nt, synthetic construct
  source 1..23: mol_type = other RNA
atccaattcctgctatcgcaggt

SEQ ID NO: 272 - RNA, 23 nt, synthetic construct
  source 1..23: mol_type = other RNA
atctgcaacagcagaaatttgat

SEQ ID NO: 273 - RNA, 23 nt, synthetic construct
  source 1..23: mol_type = other RNA
atcaaatttctgctgttgcagat

SEQ ID NO: 274 - RNA, 23 nt, synthetic construct
  source 1..23: mol_type = other RNA
atctgcaacagcagaaatttgga

SEQ ID NO: 275 - RNA, 23 nt, synthetic construct
  source 1..23: mol_type = other RNA
tccaaatttctgctgttgcagat

SEQ ID NO: 276 - RNA, 23 nt, synthetic construct
  source 1..23: mol_type = other RNA
atctgcaacagcagaaatttcgc

SEQ ID NO: 277 - RNA, 23 nt, synthetic construct
  source 1..23: mol_type = other RNA
gcgaaatttctgctgttgcagat

SEQ ID NO: 278 - RNA, 23 nt, synthetic construct
  source 1..23: mol_type = other RNA
atctgcaacagcagaaatttaca

SEQ ID NO: 279 - RNA, 23 nt, synthetic construct
  source 1..23: mol_type = other RNA
tgtaaatttctgctgttgcagat

SEQ ID NO: 280 - RNA, 23 nt, synthetic construct
  source 1..23: mol_type = other RNA
atctgcgatagcagaaatttcgc

SEQ ID NO: 281 - RNA, 23 nt, synthetic construct
  source 1..23: mol_type = other RNA
gcgaaatttctgctatcgcagat

SEQ ID NO: 282 - RNA, 23 nt, synthetic construct
  source 1..23: mol_type = other RNA
atctgcaacagcagaaattttta

SEQ ID NO: 283 - RNA, 23 nt, synthetic construct
  source 1..23: mol_type = other RNA
taaaaatttctgctgttgcagat

SEQ ID NO: 284 - RNA, 23 nt, synthetic construct
  source 1..23: mol_type = other RNA
atcttcaacagcagaaatttggc

SEQ ID NO: 285 - RNA, 23 nt, synthetic construct
  source 1..23: mol_type = other RNA
gccaaatttctgctgttgaagat

SEQ ID NO: 286 - RNA, 23 nt, synthetic construct
  source 1..23: mol_type = other RNA
atctgcaacagcagaaattggca

SEQ ID NO: 287 - RNA, 23 nt, synthetic construct
  source 1..23: mol_type = other RNA
tgccaatttctgctgttgcagat

SEQ ID NO: 288 - RNA, 23 nt, synthetic construct
  source 1..23: mol_type = other RNA
atctgcaacagcagaaatttgag

SEQ ID NO: 289 - RNA, 23 nt, synthetic construct
  source 1..23: mol_type = other RNA
ctcaaatttctgctgttgcagat

SEQ ID NO: 290 - RNA, 20 nt, synthetic construct
  source 1..20: mol_type = other RNA
atctgcaacagcagaaattt

SEQ ID NO: 291 - RNA, 20 nt, synthetic construct
  source 1..20: mol_type = other RNA
aaatttctgctgttgcagat

SEQ ID NO: 292 - RNA, 19 nt, synthetic construct
  source 1..19: mol_type = other RNA
atctgcaacagcagaaatt

SEQ ID NO: 293 - RNA, 19 nt, synthetic construct
  source 1..19: mol_type = other RNA
aatttctgctgttgcagat

SEQ ID NO: 294 - RNA, 25 nt, synthetic construct
  source 1..25: mol_type = other RNA
ctttcaatattctattgaaatcaac

SEQ ID NO: 295 - RNA, 25 nt, synthetic construct
  source 1..25: mol_type = other RNA
gttgatttcaatagaatattgaaag

SEQ ID NO: 296 - RNA, 25 nt, synthetic construct
  source 1..25: mol_type = other RNA
ctttcaatattctactgaaatcaac

SEQ ID NO: 297 - RNA, 25 nt, synthetic construct
  source 1..25: mol_type = other RNA
gttgatttcagtagaatattgaaag

SEQ ID NO: 298 - RNA, 25 nt, synthetic construct
  source 1..25: mol_type = other RNA
ctttcgatattcctctggaatcatt

SEQ ID NO: 299 - RNA, 25 nt, synthetic construct
  source 1..25: mol_type = other RNA
aatgattccagaggaatatcgaaag

SEQ ID NO: 300 - RNA, 25 nt, synthetic construct
  source 1..25: mol_type = other RNA
ctttcaatattctattgaaattggc

SEQ ID NO: 301 - RNA, 25 nt, synthetic construct
  source 1..25: mol_type = other RNA
gccaatttcaatagaatattgaaag

SEQ ID NO: 302 - RNA, 25 nt, synthetic construct
  source 1..25: mol_type = other RNA
ctttcaatattccattgaaatcaac

SEQ ID NO: 303 - RNA, 25 nt, synthetic construct
  source 1..25: mol_type = other RNA
gttgatttcaatggaatattgaaag

SEQ ID NO: 304 - RNA, 25 nt, synthetic construct
  source 1..25: mol_type = other RNA
ctttcaatattctattgaaaatcaa

SEQ ID NO: 305 - RNA, 25 nt, synthetic construct
  source 1..25: mol_type = other RNA
ttgattttcaatagaatattgaaag

SEQ ID NO: 306 - RNA, 25 nt, synthetic construct
  source 1..25: mol_type = other RNA
gcttcaattcttctgttttagattc

SEQ ID NO: 307 - RNA, 25 nt, synthetic construct
  source 1..25: mol_type = other RNA
gaatctaaaacagaagaattgaagc

SEQ ID NO: 308 - RNA, 23 nt, synthetic construct
  source 1..23: mol_type = other RNA
tgatttcagaggaatattgaaac

SEQ ID NO: 309 - RNA, 23 nt, synthetic construct
  source 1..23: mol_type = other RNA
gtttcaatattcctctgaaatca

SEQ ID NO: 310 - RNA, 24 nt, synthetic construct
  source 1..24: mol_type = other RNA
ctttcagtcttatagaattgcttc

SEQ ID NO: 311 - RNA, 24 nt, synthetic construct
  source 1..24: mol_type = other RNA
gaagcaattctataagactgaaag

SEQ ID NO: 312 - RNA, 24 nt, synthetic construct
  source 1..24: mol_type = other RNA
ctttcagttttatagaattgcttc

SEQ ID NO: 313 - RNA, 24 nt, synthetic construct
  source 1..24: mol_type = other RNA
gaagcaattctataaaactgaaag

SEQ ID NO: 314 - RNA, 24 nt, synthetic construct
  source 1..24: mol_type = other RNA
ttttggtttttatagaattgcttc

SEQ ID NO: 315 - RNA, 24 nt, synthetic construct
  source 1..24: mol_type = other RNA
gaagcaattctataaaaaccaaaa

SEQ ID NO: 316 - RNA, 24 nt, synthetic construct
  source 1..24: mol_type = other RNA
ctttcattcttatagaattgcttc

SEQ ID NO: 317 - RNA, 24 nt, synthetic construct
  source 1..24: mol_type = other RNA
gaagcaattctataagaatgaaag

SEQ ID NO: 318 - RNA, 24 nt, synthetic construct
  source 1..24: mol_type = other RNA
ttttcagtcttatagaattgcttc

SEQ ID NO: 319 - RNA, 24 nt, synthetic construct
  source 1..24: mol_type = other RNA
gaagcaattctataagactgaaaa

SEQ ID NO: 320 - RNA, 24 nt, synthetic construct
  source 1..24: mol_type = other RNA
gtaacaactgaaagaaactaaaac

SEQ ID NO: 321 - RNA, 24 nt, synthetic construct
  source 1..24: mol_type = other RNA
gttttagtttctttcagttgttac

SEQ ID NO: 322 - RNA, 24 nt, synthetic construct
  source 1..24: mol_type = other RNA
ctttcaattctctatttgagatgc

SEQ ID NO: 323 - RNA, 24 nt, synthetic construct
  source 1..24: mol_type = other RNA
gcatctcaaatagagaattgaaag

SEQ ID NO: 324 - RNA, 32 nt, synthetic construct
  source 1..32: mol_type = other RNA
gtcgcacctctcgtaggtgcgtggattgaaat

SEQ ID NO: 325 - RNA, 32 nt, synthetic construct
  source 1..32: mol_type = other RNA
atttcaatccacgcacctacgagaggtgcgac

SEQ ID NO: 326 - RNA, 24 nt, synthetic construct
  source 1..24: mol_type = other RNA
ccatcagtatcaaagtaataccaa

SEQ ID NO: 327 - RNA, 24 nt, synthetic construct
  source 1..24: mol_type = other RNA
ttggtattactttgatactgatgg

SEQ ID NO: 328 - RNA, 25 nt, synthetic construct
  source 1..25: mol_type = other RNA
ggtactgcatctcatgctgaaggtg

SEQ ID NO: 329 - RNA, 25 nt, synthetic construct
  source 1..25: mol_type = other RNA
caccttcagcatgagatgcagtacc

SEQ ID NO: 330 - RNA, 25 nt, synthetic construct
  source 1..25: mol_type = other RNA
ggaaactctgcacatgctgaaggcg

SEQ ID NO: 331 - RNA, 25 nt, synthetic construct
  source 1..25: mol_type = other RNA
cgccttcagcatgtgcagagtttcc

SEQ ID NO: 332 - RNA, 25 nt, synthetic construct
  source 1..25: mol_type = other RNA
ggtagtgcatctcatgctgaaggtg

SEQ ID NO: 333 - RNA, 25 nt, synthetic construct
  source 1..25: mol_type = other RNA
caccttcagcatgagatgcactacc

SEQ ID NO: 334 - RNA, 25 nt, synthetic construct
  source 1..25: mol_type = other RNA
ggatacgcatctcatgcagagggtg

SEQ ID NO: 335 - RNA, 25 nt, synthetic construct
  source 1..25: mol_type = other RNA
caccctctgcatgagatgcgtatcc

SEQ ID NO: 336 - RNA, 25 nt, synthetic construct
  source 1..25: mol_type = other RNA
aatactcatgcacatgctgaaggtg

SEQ ID NO: 337 - RNA, 25 nt, synthetic construct
  source 1..25: mol_type = other RNA
caccttcagcatgtgcatgagtatt

SEQ ID NO: 338 - RNA, 25 nt, synthetic construct
  source 1..25: mol_type = other RNA
ggaaattactctcatgcggaaggtg

SEQ ID NO: 339 - RNA, 25 nt, synthetic construct
  source 1..25: mol_type = other RNA
caccttccgcatgagagtaatttcc

SEQ ID NO: 340 - RNA, 25 nt, synthetic construct
  source 1..25: mol_type = other RNA
aaacacgcatctcatgcagaaggtg

SEQ ID NO: 341 - RNA, 25 nt, synthetic construct
  source 1..25: mol_type = other RNA
caccttctgcatgagatgcgtgttt

SEQ ID NO: 342 - RNA, 25 nt, synthetic construct
  source 1..25: mol_type = other RNA
gctaatcacgcacatgcagaaggtg

SEQ ID NO: 343 - RNA, 25 nt, synthetic construct
  source 1..25: mol_type = other RNA
caccttctgcatgtgcgtgattagc

SEQ ID NO: 344 - RNA, 25 nt, synthetic construct
  source 1..25: mol_type = other RNA
ggtaaagcatcacacgcagaaggcg

SEQ ID NO: 345 - RNA, 25 nt, synthetic construct
  source 1..25: mol_type = other RNA
cgccttctgcgtgtgatgctttacc

SEQ ID NO: 346 - RNA, 25 nt, synthetic construct
  source 1..25: mol_type = other RNA
ggaagtttttctcatactcaaggta

SEQ ID NO: 347 - RNA, 25 nt, synthetic construct
  source 1..25: mol_type = other RNA
taccttgagtatgagaaaaacttcc

SEQ ID NO: 348 - RNA, 25 nt, synthetic construct
  source 1..25: mol_type = other RNA
ggtaatgcatctcatgctgaaggtg

SEQ ID NO: 349 - RNA, 25 nt, synthetic construct
  source 1..25: mol_type = other RNA
caccttcagcatgagatgcattacc

SEQ ID NO: 350 - RNA, 30 nt, synthetic construct
  source 1..30: mol_type = other RNA
gtttcagacggacccttgggcggttgaagc

SEQ ID NO: 351 - RNA, 30 nt, synthetic construct
  source 1..30: mol_type = other RNA
gcttcaaccgcccaagggtccgtctgaaac

SEQ ID NO: 352 - RNA, 30 nt, synthetic construct
  source 1..30: mol_type = other RNA
tttcagacggatcccttgggcggttgaagc

SEQ ID NO: 353 - RNA, 30 nt, synthetic construct
  source 1..30: mol_type = other RNA
gcttcaaccgcccaagggatccgtctgaaa

SEQ ID NO: 354 - RNA, 30 nt, synthetic construct
  source 1..30: mol_type = other RNA
gtttcagacggcctctggagtggccgaagc

SEQ ID NO: 355 - RNA, 30 nt, synthetic construct
  source 1..30: mol_type = other RNA
gcttcggccactccagaggccgtctgaaac

SEQ ID NO: 356 - RNA, 35 nt, synthetic construct
  source 1..35: mol_type = other RNA
gtttcaaccgcacgaggatccgtctgaaaccatgg

SEQ ID NO: 357 - RNA, 35 nt, synthetic construct
  source 1..35: mol_type = other RNA
ccatggtttcagacggatcctcgtgcggttgaaac

SEQ ID NO: 358 - RNA, 35 nt, synthetic construct
  source 1..35: mol_type = other RNA
gtttcaaccgcacgaggatccgtctgaaacatgga

SEQ ID NO: 359 - RNA, 35 nt, synthetic construct
  source 1..35: mol_type = other RNA
tccatgtttcagacggatcctcgtgcggttgaaac

SEQ ID NO: 360 - RNA, 28 nt, synthetic construct
  source 1..28: mol_type = other RNA
acccagacctcgacgccgactgccacgc

SEQ ID NO: 361 - RNA, 28 nt, synthetic construct
  source 1..28: mol_type = other RNA
gcgtggcagtcggcgtcgaggtctgggt

SEQ ID NO: 362 - RNA, 24 nt, synthetic construct
  source 1..24: mol_type = other RNA
gtcgccgaactcgtcgtcaccgcc

SEQ ID NO: 363 - RNA, 24 nt, synthetic construct
  source 1..24: mol_type = other RNA
ggcggtgacgacgagttcggcgac

SEQ ID NO: 364 - RNA, 30 nt, synthetic construct
  source 1..30: mol_type = other RNA
catttcaattccataaggtacaattaatac

SEQ ID NO: 365 - RNA, 30 nt, synthetic construct
  source 1..30: mol_type = other RNA
gtattaattgtaccttatggaattgaaatg

SEQ ID NO: 366 - RNA, 29 nt, synthetic construct
  source 1..29: mol_type = other RNA
gtattaattgtaccttatggaattgaaat

SEQ ID NO: 367 - RNA, 29 nt, synthetic construct
  source 1..29: mol_type = other RNA
atttcaattccataaggtacaattaatac

SEQ ID NO: 368 - RNA, 29 nt, synthetic construct
  source 1..29: mol_type = other RNA
gtattaattgtaccttatggaattaggac

SEQ ID NO: 369 - RNA, 29 nt, synthetic construct
  source 1..29: mol_type = other RNA
gtcctaattccataaggtacaattaatac

SEQ ID NO: 370 - RNA, 29 nt, synthetic construct
  source 1..29: mol_type = other RNA
gtattaattataccttatggaattgaaat

SEQ ID NO: 371 - RNA, 29 nt, synthetic construct
  source 1..29: mol_type = other RNA
atttcaattccataaggtataattaatac

SEQ ID NO: 372 - RNA, 54 nt, synthetic construct
  source 1..54: mol_type = other RNA
tttttctttgtcggggtagcgggattcgaacccacgaccccctgctcccaaagc

SEQ ID NO: 373 - RNA, 54 nt, synthetic construct
  source 1..54: mol_type = other RNA
gctttgggagcagggggtcgtgggttcgaatcccgctaccccgacaaagaaaaa

SEQ ID NO: 374 - RNA, 54 nt, synthetic construct
  source 1..54: mol_type = other RNA
tttttctttgtcggggtagcgggattcgaacccacgacccccagctcccaaagc

SEQ ID NO: 375 - RNA, 54 nt, synthetic construct
  source 1..54: mol_type = other RNA
gctttgggagctgggggtcgtgggttcgaatcccgctaccccgacaaagaaaaa

SEQ ID NO: 376 - RNA, 31 nt, synthetic construct
  source 1..31: mol_type = other RNA
tatttcaattccataaggtacaattaatact

SEQ ID NO: 377 - RNA, 31 nt, synthetic construct
  source 1..31: mol_type = other RNA
agtattaattgtaccttatggaattgaaata

SEQ ID NO: 378 - RNA, 31 nt, synthetic construct
  source 1..31: mol_type = other RNA
agtcctaattccataaggtacaattaatact

SEQ ID NO: 379 - RNA, 31 nt, synthetic construct
  source 1..31: mol_type = other RNA
agtattaattgtaccttatggaattaggact

SEQ ID NO: 380 - RNA, 29 nt, synthetic construct
  source 1..29: mol_type = other RNA
gtattaattgtaccttgtggaattgaaat

SEQ ID NO: 381 - RNA, 29 nt, synthetic construct
  source 1..29: mol_type = other RNA
atttcaattccacaaggtacaattaatac

SEQ ID NO: 382 - RNA, 29 nt, synthetic construct
  source 1..29: mol_type = other RNA
gtattaattgtacttatggaattgaaatt

SEQ ID NO: 383 - RNA, 29 nt, synthetic construct
  source 1..29: mol_type = other RNA
aatttcaattccataagtacaattaatac

SEQ ID NO: 384 - RNA, 30 nt, synthetic construct
  source 1..30: mol_type = other RNA
tgtattaattgtaccttatggaattgaaat

SEQ ID NO: 385 - RNA, 30 nt, synthetic construct
  source 1..30: mol_type = other RNA
atttcaattccataaggtacaattaataca

SEQ ID NO: 386 - RNA, 30 nt, synthetic construct
  source 1..30: mol_type = other RNA
ggtattaattgtaccttatggaattaggac

SEQ ID NO: 387 - RNA, 30 nt, synthetic construct
  source 1..30: mol_type = other RNA
gtcctaattccataaggtacaattaatacc

SEQ ID NO: 388 - RNA, 30 nt, synthetic construct
  source 1..30: mol_type = other RNA
ggtattaattgtaccttatggaattgaaat

SEQ ID NO: 389 - RNA, 30 nt, synthetic construct
  source 1..30: mol_type = other RNA
atttcaattccataaggtacaattaatacc

SEQ ID NO: 390 - RNA, 30 nt, synthetic construct
  source 1..30: mol_type = other RNA
agtattaattgtaccttatggaattgaaat

SEQ ID NO: 391 - RNA, 30 nt, synthetic construct
  source 1..30: mol_type = other RNA
atttcaattccataaggtacaattaatact

SEQ ID NO: 392 - RNA, 29 nt, synthetic construct
  source 1..29: mol_type = other RNA
gtattaattgtaccttatggatttgaaat

SEQ ID NO: 393 - RNA, 29 nt, synthetic construct
  source 1..29: mol_type = other RNA
atttcaaatccataaggtacaattaatac

SEQ ID NO: 394 - RNA, 29 nt, synthetic construct
  source 1..29: mol_type = other RNA
gtattaattgtatcttatggaattgaaat

SEQ ID NO: 395 - RNA, 29 nt, synthetic construct
  source 1..29: mol_type = other RNA
atttcaattccataagatacaattaatac

SEQ ID NO: 396 - RNA, 33 nt, synthetic construct
  source 1..33: mol_type = other RNA
aaagtattaattgtaccttatggaattgaaata

SEQ ID NO: 397 - RNA, 33 nt, synthetic construct
  source 1..33: mol_type = other RNA
tatttcaattccataaggtacaattaatacttt

SEQ ID NO: 398 - RNA, 24 nt, synthetic construct
  source 1..24: mol_type = other RNA
attcccaatatattgtgaatttga

SEQ ID NO: 399 - RNA, 24 nt, synthetic construct
  source 1..24: mol_type = other RNA
tcaaattcacaatatattgggaat

SEQ ID NO: 400 - RNA, 30 nt, synthetic construct
  source 1..30: mol_type = other RNA
gtttcaagcccttataggtattcaccaaac

SEQ ID NO: 401 - RNA, 30 nt, synthetic construct
  source 1..30: mol_type = other RNA
gtttggtgaatacctataagggcttgaaac

SEQ ID NO: 402 - RNA, 30 nt, synthetic construct
  source 1..30: mol_type = other RNA
tctcaaagcccttataggtattcatcaaac

SEQ ID NO: 403 - RNA, 30 nt, synthetic construct
  source 1..30: mol_type = other RNA
gtttgatgaatacctataagggctttgaga

SEQ ID NO: 404 - RNA, 30 nt, synthetic construct
  source 1..30: mol_type = other RNA
gtttcaagcccttataggcattcaccaaac

SEQ ID NO: 405 - RNA, 30 nt, synthetic construct
  source 1..30: mol_type = other RNA
gtttggtgaatgcctataagggcttgaaac

SEQ ID NO: 406 - RNA, 25 nt, synthetic construct
  source 1..25: mol_type = other RNA
gtttcccatgaaatgggtgttgaaa

SEQ ID NO: 407 - RNA, 25 nt, synthetic construct
  source 1..25: mol_type = other RNA
tttcaacacccatttcatgggaaac

SEQ ID NO: 408 - RNA, 47 nt, synthetic construct
  source 1..47: mol_type = other RNA
gttgttgcttatagtacaaaggtattaaaattcaagcaaatcacaac

SEQ ID NO: 409 - RNA, 47 nt, synthetic construct
  source 1..47: mol_type = other RNA
gttgtgatttgcttgaattttaatacctttgtactataagcaacaac

SEQ ID NO: 410 - RNA, 17 nt, synthetic construct
  source 1..17: mol_type = other RNA
cggcgactcagtcgccg

SEQ ID NO: 411 - RNA, 17 nt, synthetic construct
  source 1..17: mol_type = other RNA
cggcgactgagtcgccg

SEQ ID NO: 412 - RNA, 20 nt, synthetic construct
  source 1..20: mol_type = other RNA
aaacatcatacttattcaac

SEQ ID NO: 413 - RNA, 20 nt, synthetic construct
  source 1..20: mol_type = other RNA
gttgaataagtatgatgttt

SEQ ID NO: 414 - RNA, 36 nt, synthetic construct
  source 1..36: mol_type = other RNA
gtgcaacttgctgatgtttgtagtaccgaatggcgg

SEQ ID NO: 415 - RNA, 36 nt, synthetic construct
  source 1..36: mol_type = other RNA
ccgccattcggtactacaaacatcagcaagttgcac

SEQ ID NO: 416 - RNA, 36 nt, synthetic construct
  source 1..36: mol_type = other RNA
gtgcaacttgctgatgtttgtagtaccgaatggcga

SEQ ID NO: 417 - RNA, 36 nt, synthetic construct
  source 1..36: mol_type = other RNA
tcgccattcggtactacaaacatcagcaagttgcac

SEQ ID NO: 418 - RNA, 26 nt, synthetic construct
  source 1..26: mol_type = other RNA
agtaagaatttgcattggtaccaaac

SEQ ID NO: 419 - RNA, 26 nt, synthetic construct
  source 1..26: mol_type = other RNA
gtttggtaccaatgcaaattcttact

SEQ ID NO: 420 - RNA, 26 nt, synthetic construct
  source 1..26: mol_type = other RNA
agtaagaattggcacgggtaccaaac

SEQ ID NO: 421 - RNA, 26 nt, synthetic construct
  source 1..26: mol_type = other RNA
gtttggtacccgtgccaattcttact

SEQ ID NO: 422 - RNA, 26 nt, synthetic construct
  source 1..26: mol_type = other RNA
agtaagaatttacacggataccaaac

SEQ ID NO: 423 - RNA, 26 nt, synthetic construct
  source 1..26: mol_type = other RNA
gtttggtatccgtgtaaattcttact

SEQ ID NO: 424 - RNA, 26 nt, synthetic construct
  source 1..26: mol_type = other RNA
agtaagaattgtcacggggtaccaaa

SEQ ID NO: 425 - RNA, 26 nt, synthetic construct
  source 1..26: mol_type = other RNA
tttggtaccccgtgacaattcttact

SEQ ID NO: 426 - RNA, 26 nt, synthetic construct
  source 1..26: mol_type = other RNA
agcaagaatttacatgagttccaaac

SEQ ID NO: 427 - RNA, 26 nt, synthetic construct
  source 1..26: mol_type = other RNA
gtttggaactcatgtaaattcttgct

SEQ ID NO: 428 - RNA, 26 nt, synthetic construct
  source 1..26: mol_type = other RNA
agcaagaattgtcacgggtgccaaac

SEQ ID NO: 429 - RNA, 26 nt, synthetic construct
  source 1..26: mol_type = other RNA
gtttggcacccgtgacaattcttgct

SEQ ID NO: 430 - RNA, 26 nt, synthetic construct
  source 1..26: mol_type = other RNA
agtaagaatttacacgggtaccaaac

SEQ ID NO: 431 - RNA, 26 nt, synthetic construct
  source 1..26: mol_type = other RNA
gtttggtacccgtgtaaattcttact

SEQ ID NO: 432 - RNA, 26 nt, synthetic construct
  source 1..26: mol_type = other RNA
agtaaggatttacacgggtaccaaac

SEQ ID NO: 433 - RNA, 26 nt, synthetic construct
  source 1..26: mol_type = other RNA
gtttggtacccgtgtaaatccttact

SEQ ID NO: 434 - RNA, 26 nt, synthetic construct
  source 1..26: mol_type = other RNA
agtaagaatttacatgggtaccaaac

SEQ ID NO: 435 - RNA, 26 nt, synthetic construct
  source 1..26: mol_type = other RNA
gtttggtacccatgtaaattcttact

SEQ ID NO: 436 - RNA, 26 nt, synthetic construct
  source 1..26: mol_type = other RNA
agtaagaattgtcacggggcgccaaa

SEQ ID NO: 437 - RNA, 26 nt, synthetic construct
  source 1..26: mol_type = other RNA
tttggcgccccgtgacaattcttact

SEQ ID NO: 438 - RNA, 24 nt, synthetic construct
  source 1..24: mol_type = other RNA
ttgagtagtaagaatttacatggg

SEQ ID NO: 439 - RNA, 24 nt, synthetic construct
  source 1..24: mol_type = other RNA
cccatgtaaattcttactactcaa

SEQ ID NO: 440 - RNA, 24 nt, synthetic construct
  source 1..24: mol_type = other RNA
ttgagtagtaagaattgtcatggg

SEQ ID NO: 441 - RNA, 24 nt, synthetic construct
  source 1..24: mol_type = other RNA
cccatgacaattcttactactcaa

SEQ ID NO: 442 - RNA, 24 nt, synthetic construct
  source 1..24: mol_type = other RNA
ttgagcagtaagaatttacacggg

SEQ ID NO: 443 - RNA, 24 nt, synthetic construct
  source 1..24: mol_type = other RNA
cccgtgtaaattcttactgctcaa

SEQ ID NO: 444 - RNA, 24 nt, synthetic construct
  source 1..24: mol_type = other RNA
ttgagtagtaaaaattgttacggg

SEQ ID NO: 445 - RNA, 24 nt, synthetic construct
  source 1..24: mol_type = other RNA
cccgtaacaatttttactactcaa

SEQ ID NO: 446 - RNA, 24 nt, synthetic construct
  source 1..24: mol_type = other RNA
ttgagtagtaagaatatacacgag

SEQ ID NO: 447 - RNA, 24 nt, synthetic construct
  source 1..24: mol_type = other RNA
ctcgtgtatattcttactactcaa

SEQ ID NO: 448 - RNA, 24 nt, synthetic construct
  source 1..24: mol_type = other RNA
gttattgagtagtaagaatttaca

SEQ ID NO: 449 - RNA, 24 nt, synthetic construct
  source 1..24: mol_type = other RNA
tgtaaattcttactactcaataac

SEQ ID NO: 450 - RNA, 24 nt, synthetic construct
  source 1..24: mol_type = other RNA
gttgctgagtagcaagaaattaca

SEQ ID NO: 451 - RNA, 24 nt, synthetic construct
  source 1..24: mol_type = other RNA
tgtaatttcttgctactcagcaac

SEQ ID NO: 452 - RNA, 24 nt, synthetic construct
  source 1..24: mol_type = other RNA
gtttttgagcaataagaatttgca

SEQ ID NO: 453 - RNA, 24 nt, synthetic construct
  source 1..24: mol_type = other RNA
tgcaaattcttattgctcaaaaac

SEQ ID NO: 454 - RNA, 24 nt, synthetic construct
  source 1..24: mol_type = other RNA
gttgaagagccgcaagaattcgca

SEQ ID NO: 455 - RNA, 24 nt, synthetic construct
  source 1..24: mol_type = other RNA
tgcgaattcttgcggctcttcaac

SEQ ID NO: 456 - RNA, 23 nt, synthetic construct
  source 1..23: mol_type = other RNA
cttgaggcgctcgacctcctgtt

SEQ ID NO: 457 - RNA, 23 nt, synthetic construct
  source 1..23: mol_type = other RNA
aacaggaggtcgagcgcctcaag

SEQ ID NO: 458 - RNA, 23 nt, synthetic construct
  source 1..23: mol_type = other RNA
cttgagccgctcgacctgctgct

SEQ ID NO: 459 - RNA, 23 nt, synthetic construct
  source 1..23: mol_type = other RNA
agcagcaggtcgagcggctcaag

SEQ ID NO: 460 - RNA, 23 nt, synthetic construct
  source 1..23: mol_type = other RNA
gttgaggcgctcgacttcccgct

SEQ ID NO: 461 - RNA, 23 nt, synthetic construct
  source 1..23: mol_type = other RNA
agcgggaagtcgagcgcctcaac

SEQ ID NO: 462 - RNA, 23 nt, synthetic construct
  source 1..23: mol_type = other RNA
gttgaggtgctcgacctgctgct

SEQ ID NO: 463 - RNA, 23 nt, synthetic construct
  source 1..23: mol_type = other RNA
agcagcaggtcgagcacctcaac

SEQ ID NO: 464 - RNA, 23 nt, synthetic construct
  source 1..23: mol_type = other RNA
cttgaggcgctcgacctgctgct

SEQ ID NO: 465 - RNA, 23 nt, synthetic construct
  source 1..23: mol_type = other RNA
agcagcaggtcgagcgcctcaag

SEQ ID NO: 466 - RNA, 23 nt, synthetic construct
  source 1..23: mol_type = other RNA
cttgaggcgctcgacctcctgct

SEQ ID NO: 467 - RNA, 23 nt, synthetic construct
  source 1..23: mol_type = other RNA
agcaggaggtcgagcgcctcaag

SEQ ID NO: 468 - RNA, 23 nt, synthetic construct
  source 1..23: mol_type = other RNA
ctccaagcgctggacctcctcct

SEQ ID NO: 469 - RNA, 23 nt, synthetic construct
  source 1..23: mol_type = other RNA
aggaggaggtccagcgcttggag

SEQ ID NO: 470 - RNA, 23 nt, synthetic construct
  source 1..23: mol_type = other RNA
cttgaggcgctcgacctcctcct

SEQ ID NO: 471 - RNA, 23 nt, synthetic construct
  source 1..23: mol_type = other RNA
aggaggaggtcgagcgcctcaag

SEQ ID NO: 472 - RNA, 23 nt, synthetic construct
  source 1..23: mol_type = other RNA
gtcgagaagcttgagctgctgct

SEQ ID NO: 473 - RNA, 23 nt, synthetic construct
  source 1..23: mol_type = other RNA
agcagcagctcaagcttctcgac

SEQ ID NO: 474 - RNA, 23 nt, synthetic construct
  source 1..23: mol_type = other RNA
cctgagccgctccaccttctgct

SEQ ID NO: 475 - RNA, 23 nt, synthetic construct
  source 1..23: mol_type = other RNA
agcagaaggtggagcggctcagg

SEQ ID NO: 476 - RNA, 29 nt, synthetic construct
  source 1..29: mol_type = other RNA
cgtcccgcccacgcacgcgagggaacggc

SEQ ID NO: 477 - RNA, 29 nt, synthetic construct
  source 1..29: mol_type = other RNA
gccgttccctcgcgtgcgtgggcgggacg

SEQ ID NO: 478 - RNA, 29 nt, synthetic construct
  source 1..29: mol_type = other RNA
tgttccgcccacgcacgcgagggaacggc

SEQ ID NO: 479 - RNA, 29 nt, synthetic construct
  source 1..29: mol_type = other RNA
gccgttccctcgcgtgcgtgggcggaaca

SEQ ID NO: 480 - RNA, 29 nt, synthetic construct
  source 1..29: mol_type = other RNA
cgttccgcccacgcacgcgagggaacggc

SEQ ID NO: 481 - RNA, 29 nt, synthetic construct
  source 1..29: mol_type = other RNA
gccgttccctcgcgtgcgtgggcggaacg

SEQ ID NO: 482 - RNA, 29 nt, synthetic construct
  source 1..29: mol_type = other RNA
ggtctctcccacgcactcgagggaacgtc

SEQ ID NO: 483 - RNA, 29 nt, synthetic construct
  source 1..29: mol_type = other RNA
gacgttccctcgagtgcgtgggagagacc

SEQ ID NO: 484 - RNA, 28 nt, synthetic construct
  source 1..28: mol_type = other RNA
gtcccgcccacgcacgcgagggaacggc

SEQ ID NO: 485 - RNA, 28 nt, synthetic construct
  source 1..28: mol_type = other RNA
gccgttccctcgcgtgcgtgggcgggac

SEQ ID NO: 486 - RNA, 28 nt, synthetic construct
  source 1..28: mol_type = other RNA
gttccgcccacgcacgcgagggaacggc

SEQ ID NO: 487 - RNA, 28 nt, synthetic construct
  source 1..28: mol_type = other RNA
gccgttccctcgcgtgcgtgggcggaac

SEQ ID NO: 488 - RNA, 28 nt, synthetic construct
  source 1..28: mol_type = other RNA
gtctctcccacgcacgcgagggaacggc

SEQ ID NO: 489 - RNA, 28 nt, synthetic construct
  source 1..28: mol_type = other RNA
gccgttccctcgcgtgcgtgggagagac

SEQ ID NO: 490 - RNA, 28 nt, synthetic construct
  source 1..28: mol_type = other RNA
gtcccgcccacgcacacgagggaacggc

SEQ ID NO: 491 - RNA, 28 nt, synthetic construct
  source 1..28: mol_type = other RNA
gccgttccctcgtgtgcgtgggcgggac

SEQ ID NO: 492 - RNA, 28 nt, synthetic construct
  source 1..28: mol_type = other RNA
gcctcgcccacgcgtcctaggggacatc

SEQ ID NO: 493 - RNA, 28 nt, synthetic construct
  source 1..28: mol_type = other RNA
gatgtcccctaggacgcgtgggcgaggc

SEQ ID NO: 494 - RNA, 24 nt, synthetic construct
  source 1..24: mol_type = other RNA
gccgttccctcgcgtgcgtgggcg

SEQ ID NO: 495 - RNA, 24 nt, synthetic construct
  source 1..24: mol_type = other RNA
cgcccacgcacgcgagggaacggc

SEQ ID NO: 496 - RNA, 24 nt, synthetic construct
  source 1..24: mol_type = other RNA
gccgttccctcgcgtgcgtgggag

SEQ ID NO: 497 - RNA, 24 nt, synthetic construct
  source 1..24: mol_type = other RNA
ctcccacgcacgcgagggaacggc

SEQ ID NO: 498 - RNA, 28 nt, synthetic construct
  source 1..28: mol_type = other RNA
gtctcgcccacgcacacgaggggacggc

SEQ ID NO: 499 - RNA, 28 nt, synthetic construct
  source 1..28: mol_type = other RNA
gccgtcccctcgtgtgcgtgggcgagac

SEQ ID NO: 500 - RNA, 28 nt, synthetic construct
  source 1..28: mol_type = other RNA
gtctcgctcacgcacgcgagggaacggc

SEQ ID NO: 501 - RNA, 28 nt, synthetic construct
  source 1..28: mol_type = other RNA
gccgttccctcgcgtgcgtgagcgagac

SEQ ID NO: 502 - RNA, 28 nt, synthetic construct
  source 1..28: mol_type = other RNA
gtctcgcccacgcacacgagggggcgtc

SEQ ID NO: 503 - RNA, 28 nt, synthetic construct
  source 1..28: mol_type = other RNA
gacgccccctcgtgtgcgtgggcgagac

SEQ ID NO: 504 - RNA, 28 nt, synthetic construct
  source 1..28: mol_type = other RNA
gtcccgcccacgcacacgcacacgaggg

SEQ ID NO: 505 - RNA, 28 nt, synthetic construct
  source 1..28: mol_type = other RNA
ccctcgtgtgcgtgtgcgtgggcgggac

SEQ ID NO: 506 - RNA, 28 nt, synthetic construct
  source 1..28: mol_type = other RNA
cccacgcacacgcacacgaggggacggc

SEQ ID NO: 507 - RNA, 28 nt, synthetic construct
  source 1..28: mol_type = other RNA
gccgtcccctcgtgtgcgtgtgcgtggg

SEQ ID NO: 508 - RNA, 25 nt, synthetic construct
  source 1..25: mol_type = other RNA
ccgcccacgcacgcgagggaacggc

SEQ ID NO: 509 - RNA, 25 nt, synthetic construct
  source 1..25: mol_type = other RNA
gccgttccctcgcgtgcgtgggcgg

SEQ ID NO: 510 - RNA, 37 nt, synthetic construct
  source 1..37: mol_type = other RNA
gtcatcccccgcgagcgagcgggggccgcattgaagc

SEQ ID NO: 511 - RNA, 37 nt, synthetic construct
  source 1..37: mol_type = other RNA
gcttcaatgcggcccccgctcgctcgcgggggatgac

SEQ ID NO: 512 - RNA, 37 nt, synthetic construct
  source 1..37: mol_type = other RNA
gtcatcccccgcgagcgagcgggggccgcattgaagg

SEQ ID NO: 513 - RNA, 37 nt, synthetic construct
  source 1..37: mol_type = other RNA
ccttcaatgcggcccccgctcgctcgcgggggatgac

SEQ ID NO: 514 - RNA, 36 nt, synthetic construct
  source 1..36: mol_type = other RNA
gttgcaatcccaaggtaatgcgtctcccattgacgc

SEQ ID NO: 515 - RNA, 36 nt, synthetic construct
  source 1..36: mol_type = other RNA
gcgtcaatgggagacgcattaccttgggattgcaac

SEQ ID NO: 516 - RNA, 36 nt, synthetic construct
  source 1..36: mol_type = other RNA
gaattgatcccgttgtaatgcgtctcccattgacgc

SEQ ID NO: 517 - RNA, 36 nt, synthetic construct
  source 1..36: mol_type = other RNA
gcgtcaatgggagacgcattacaacgggatcaattc

SEQ ID NO: 518 - RNA, 36 nt, synthetic construct
  source 1..36: mol_type = other RNA
gcgtcaatgggagacgcattactttaggattgcaac

SEQ ID NO: 519 - RNA, 36 nt, synthetic construct
  source 1..36: mol_type = other RNA
gttgcaatcctaaagtaatgcgtctcccattgacgc

SEQ ID NO: 520 - RNA, 36 nt, synthetic construct
  source 1..36: mol_type = other RNA
gcgtcaatgggagacgcattactttgggattgcaac

SEQ ID NO: 521 - RNA, 36 nt, synthetic construct
  source 1..36: mol_type = other RNA
gttgcaatcccaaagtaatgcgtctcccattgacgc

SEQ ID NO: 522 - RNA, 36 nt, synthetic construct
  source 1..36: mol_type = other RNA
gcgtcaatgggagacgcattactttaggattgcatc

SEQ ID NO: 523 - RNA, 36 nt, synthetic construct
  source 1..36: mol_type = other RNA
gatgcaatcctaaagtaatgcgtctcccattgacgc

SEQ ID NO: 524 - RNA, 36 nt, synthetic construct
  source 1..36: mol_type = other RNA
gcgtcaatgggagacgcattaactttgggattgcaa

SEQ ID NO: 525 - RNA, 36 nt, synthetic construct
  source 1..36: mol_type = other RNA
ttgcaatcccaaagttaatgcgtctcccattgacgc

SEQ ID NO: 526 - RNA, 36 nt, synthetic construct
  source 1..36: mol_type = other RNA
gcgtcaatgggagacgcattactttggaattgcaac

SEQ ID NO: 527 - RNA, 36 nt, synthetic construct
  source 1..36: mol_type = other RNA
gttgcaattccaaagtaatgcgtctcccattgacgc

SEQ ID NO: 528 - RNA, 23 nt, synthetic construct
  source 1..23: mol_type = other RNA
ggcgtcaatgggagacgcattac

SEQ ID NO: 529 - RNA, 23 nt, synthetic construct
  source 1..23: mol_type = other RNA
gtaatgcgtctcccattgacgcc

SEQ ID NO: 530 - RNA, 23 nt, synthetic construct
  source 1..23: mol_type = other RNA
agcgtcaatgggagacgcattac

SEQ ID NO: 531 - RNA, 23 nt, synthetic construct
  source 1..23: mol_type = other RNA
gtaatgcgtctcccattgacgct

SEQ ID NO: 532 - RNA, 23 nt, synthetic construct
  source 1..23: mol_type = other RNA
ggcgtcaatgggagacgcattaa

SEQ ID NO: 533 - RNA, 23 nt, synthetic construct
  source 1..23: mol_type = other RNA
ttaatgcgtctcccattgacgcc

SEQ ID NO: 534 - RNA, 36 nt, synthetic construct
  source 1..36: mol_type = other RNA
atcgcaacatctcagaaacccgtcctaagttgacgg

SEQ ID NO: 535 - RNA, 36 nt, synthetic construct
  source 1..36: mol_type = other RNA
ccgtcaacttaggacgggtttctgagatgttgcgat

SEQ ID NO: 536 - RNA, 36 nt, synthetic construct
  source 1..36: mol_type = other RNA
ctcgcaacatctcagaaacccgtcctaagttgacgg

SEQ ID NO: 537 - RNA, 36 nt, synthetic construct
  source 1..36: mol_type = other RNA
ccgtcaacttaggacgggtttctgagatgttgcgag

SEQ ID NO: 538 - RNA, 36 nt, synthetic construct
  source 1..36: mol_type = other RNA
ctcgcaacatctcagaaagccgtcctaagttgacgg

SEQ ID NO: 539 - RNA, 36 nt, synthetic construct
  source 1..36: mol_type = other RNA
ccgtcaacttaggacggctttctgagatgttgcgag

SEQ ID NO: 540 - RNA, 36 nt, synthetic construct
  source 1..36: mol_type = other RNA
atcgcaacatcttagaaacccgtcctaagttgacgg

SEQ ID NO: 541 - RNA, 36 nt, synthetic construct
  source 1..36: mol_type = other RNA
ccgtcaacttaggacgggtttctaagatgttgcgat

SEQ ID NO: 542 - RNA, 36 nt, synthetic construct
  source 1..36: mol_type = other RNA
ctcgaaccatctcagaaatccgtcctaagctgagga

SEQ ID NO: 543 - RNA, 36 nt, synthetic construct
  source 1..36: mol_type = other RNA
tcctcagcttaggacggatttctgagatggttcgag

SEQ ID NO: 544 - RNA, 35 nt, synthetic construct
  source 1..35: mol_type = other RNA
tcgcaacatctcagaaacccgtcctaagttgacgg

SEQ ID NO: 545 - RNA, 35 nt, synthetic construct
  source 1..35: mol_type = other RNA
ccgtcaacttaggacgggtttctgagatgttgcga

SEQ ID NO: 546 - RNA, 35 nt, synthetic construct
  source 1..35: mol_type = other RNA
tcgcaacatctcagaaagccgtcctaagttgacgg

SEQ ID NO: 547 - RNA, 35 nt, synthetic construct
  source 1..35: mol_type = other RNA
ccgtcaacttaggacggctttctgagatgttgcga

SEQ ID NO: 548 - RNA, 35 nt, synthetic construct
  source 1..35: mol_type = other RNA
tcgcaacatcttagaaacccgtcctaagttgacgg

SEQ ID NO: 549 - RNA, 35 nt, synthetic construct
  source 1..35: mol_type = other RNA
ccgtcaacttaggacgggtttctaagatgttgcga

SEQ ID NO: 550 - RNA, 35 nt, synthetic construct
  source 1..35: mol_type = other RNA
tcgaaccatctcagaaatccgtcctaagctgagga

SEQ ID NO: 551 - RNA, 35 nt, synthetic construct
  source 1..35: mol_type = other RNA
tcctcagcttaggacggatttctgagatggttcga

SEQ ID NO: 552 - RNA, 36 nt, synthetic construct
  source 1..36: mol_type = other RNA
gtgcattgaccgctccctgacggaaccagccagcac

SEQ ID NO: 553 - RNA, 36 nt, synthetic construct
  source 1..36: mol_type = other RNA
gtgctggctggttccgtcagggagcggtcaatgcac

SEQ ID NO: 554 - RNA, 36 nt, synthetic construct
  source 1..36: mol_type = other RNA
gtgccttggccgacccctgacggaaccggccagcac

SEQ ID NO: 555 - RNA, 36 nt, synthetic construct
  source 1..36: mol_type = other RNA
gtgctggccggttccgtcaggggtcggccaaggcac

SEQ ID NO: 556 - RNA, 36 nt, synthetic construct
  source 1..36: mol_type = other RNA
gtgctttagttggcccctgacggaaccgaccagcac

SEQ ID NO: 557 - RNA, 36 nt, synthetic construct
  source 1..36: mol_type = other RNA
gtgctggtcggttccgtcaggggccaactaaagcac

SEQ ID NO: 558 - RNA, 36 nt, synthetic construct
  source 1..36: mol_type = other RNA
gtgccttgatcgacccctgacggaaccgaccagcac

SEQ ID NO: 559 - RNA, 36 nt, synthetic construct
  source 1..36: mol_type = other RNA
gtgctggtcggttccgtcaggggtcgatcaaggcac

SEQ ID NO: 560 - RNA, 36 nt, synthetic construct
  source 1..36: mol_type = other RNA
gtgccttgaccggcccctgacggaaccggtcagcac

SEQ ID NO: 561 - RNA, 36 nt, synthetic construct
  source 1..36: mol_type = other RNA
gtgctgaccggttccgtcaggggccggtcaaggcac

SEQ ID NO: 562 - RNA, 36 nt, synthetic construct
  source 1..36: mol_type = other RNA
gcgccttgactgacccctgacggaaccggccagcac

SEQ ID NO: 563 - RNA, 36 nt, synthetic construct
  source 1..36: mol_type = other RNA
gtgctggccggttccgtcaggggtcagtcaaggcgc

SEQ ID NO: 564 - RNA, 36 nt, synthetic construct
  source 1..36: mol_type = other RNA
gcgccttgaccgacccctgacggaacctgccagcac

SEQ ID NO: 565 - RNA, 36 nt, synthetic construct
  source 1..36: mol_type = other RNA
gtgctggcaggttccgtcaggggtcggtcaaggcgc

SEQ ID NO: 566 - RNA, 36 nt, synthetic construct
  source 1..36: mol_type = other RNA
gtgccttgaccgccccctaatggaaccggtcagcac

SEQ ID NO: 567 - RNA, 36 nt, synthetic construct
  source 1..36: mol_type = other RNA
gtgctgaccggttccattagggggcggtcaaggcac

SEQ ID NO: 568 - RNA, 36 nt, synthetic construct
  source 1..36: mol_type = other RNA
gtgccttgaccgccccctaatggaaccggccagcac

SEQ ID NO: 569 - RNA, 36 nt, synthetic construct
  source 1..36: mol_type = other RNA
gtgctggccggttccattagggggcggtcaaggcac

SEQ ID NO: 570 - RNA, 36 nt, synthetic construct
  source 1..36: mol_type = other RNA
gtgccttgactgacccctaacggaaccagccagcac

SEQ ID NO: 571 - RNA, 36 nt, synthetic construct
  source 1..36: mol_type = other RNA
gtgctggctggttccgttaggggtcagtcaaggcac

SEQ ID NO: 572 - RNA, 36 nt, synthetic construct
  source 1..36: mol_type = other RNA
gtgccttgactgaccactgacggaaccagccagcac

SEQ ID NO: 573 - RNA, 36 nt, synthetic construct
  source 1..36: mol_type = other RNA
gtgctggctggttccgtcagtggtcagtcaaggcac

SEQ ID NO: 574 - RNA, 36 nt, synthetic construct
  source 1..36: mol_type = other RNA
gtgccttgactgacccctgacggaaccagccagcac

SEQ ID NO: 575 - RNA, 36 nt, synthetic construct
  source 1..36: mol_type = other RNA
gtgctggctggttccgtcaggggtcagtcaaggcac

SEQ ID NO: 576 - RNA, 36 nt, synthetic construct
  source 1..36: mol_type = other RNA
gtgccttggccgaccccttacggaaccggccagcac

SEQ ID NO: 577 - RNA, 36 nt, synthetic construct
  source 1..36: mol_type = other RNA
gtgctggccggttccgtaaggggtcggccaaggcac

SEQ ID NO: 578 - RNA, 53 nt, synthetic construct
  source 1..53: mol_type = other RNA
gaagccctctgggacaatgaaggcggtgccagccccggcaagggcggcaaggc

SEQ ID NO: 579 - RNA, 53 nt, synthetic construct
  source 1..53: mol_type = other RNA
gccttgccgcccttgccggggctggcaccgccttcattgtcccagagggcttc

SEQ ID NO: 580 - RNA, 23 nt, synthetic construct
  source 1..23: mol_type = other RNA
tggccgccgggcatgccgatcat

SEQ ID NO: 581 - RNA, 23 nt, synthetic construct
  source 1..23: mol_type = other RNA
atgatcggcatgcccggcggcca

SEQ ID NO: 582 - RNA, 23 nt, synthetic construct
  source 1..23: mol_type = other RNA
tggcccccgggcatgccgatcat

SEQ ID NO: 583 - RNA, 23 nt, synthetic construct
  source 1..23: mol_type = other RNA
atgatcggcatgcccgggggcca

SEQ ID NO: 584 - RNA, 124 nt, synthetic construct
  source 1..124: mol_type = other RNA
ttctctcccggccagccttggctctcagctcaggccgatccagctcgaatccctgatagccacagatgagccggaaatccccgtccttcatcaactggagctttgcgccgcccggagcccacgc

SEQ ID NO: 585 - RNA, 124 nt, synthetic construct
  source 1..124: mol_type = other RNA
tggctatgtcgagttcaagctgattgggaaaaaactcaagcaaaacgcaaaggggaatagcaagcgcggccttgatgcatcgcaatggtacatcatcaagcaactgcaatcgggtgcgtgggct

SEQ ID NO: 586 - RNA, 79 nt, synthetic construct
  source 1..79: mol_type = other RNA
aacacatcgacattgctgcgccccctgaccgtggcatgcaacgcaccattctcgccgctctgcacattgatgctggctg

SEQ ID NO: 587 - RNA, 132 nt, synthetic construct
  source 1..132: mol_type = other RNA
aacgtagcagccgcgggtgaggatgtgaaggtgcggccagccggacttgtggagttccaggaacgccatgtattcgagtcgaggatagttgcggcggagccttcgcagcaaggccgtccagcgcccgcgcat

SEQ ID NO: 588 - RNA, 121 nt, synthetic construct
  source 1..121: mol_type = other RNA
ccgcgtccgactctccaaggcccgcgcccaggccgccgctggcaagccagagcgcatcatcacgctcactacacgcccccgcccaggtcttagcatcccctgtgccgtgcgctggatgcgc

SEQ ID NO: 589 - RNA, 133 nt, synthetic construct
  source 1..133: mol_type = other RNA
gcgatccgggagaaggagcaggtcttcgcgcagacgtggaaccgatcgacgctcgacagcctgcgcgacacgctctccgacggggtgctggagggcgagaacaaggaagagctcacggcccgcgtgcgcgagg

SEQ ID NO: 590 - RNA, 124 nt, synthetic construct
  source 1..124: mol_type = other RNA
tcctcgccccatatgtcccaagaccaaatgcgcagcttgcaggcgcgcgtgtcaatctcgacgcggcccggactgctgttcggcttgataccaggacagtcgatcctggccgagaagtccggcc

SEQ ID NO: 591 - RNA, 124 nt, synthetic construct
  source 1..124: mol_type = other RNA
cgaaagagcatggctaaaaaaccaccgaccattcgaaccacacttcagcacattctggataacgtgctcatcgccaaaaccagagcagagggcgacggcgtgattacgctggtccggccggact

SEQ ID NO: 592 - RNA, 128 nt, synthetic construct
  source 1..128: mol_type = other RNA
gcgccccgatctgcggcgtttcgtcgacgcgcgtcagagcatggtgcacctgtacggcttgcagacctatgccgacatcatgagcgaattcgcatccggtgagcgctacgtaaatcgggtgtggtcgg

SEQ ID NO: 593 - RNA, 126 nt, synthetic construct
  source 1..126: mol_type = other RNA
ggacgacgcggccctgatcgcgggcggaggcgagaaaggtctcgaggttctgctgcacgacgcggtagagaacggtgtcctcgggcttgcgccgctggtacccgagcgcaccggcggggtggtcgg

SEQ ID NO: 594 - RNA, 128 nt, synthetic construct
  source 1..128: mol_type = other RNA
ggagtgaccaaagtgttgtttgccgcggaccgcaaccgtgactgggcattccggaattgctcgacggccttaccgagataggtctcggcctccccgtcgtaaccatcggcagaagccgaccacacccg

SEQ ID NO: 595 - RNA, 126 nt, synthetic construct
  source 1..126: mol_type = other RNA
aatgatgttcttacctacaggttttagcctgaactgtgcataaaaactggcaacaccatacatgtcgctaagttttaagtttgtttccttttcaagcttcaggaacgcatcacgcggtataaaacc

SEQ ID NO: 596 - RNA, 126 nt, synthetic construct
  source 1..126: mol_type = other RNA
agcggaggcttacaacaatcgaggcaacacactacatgctcttcagcaatatcaggcggccctggatagctatgacaaggccatccatctcaagccggagtttgcggatgcctattccaaccgagc

SEQ ID NO: 597 - RNA, 126 nt, synthetic construct
  source 1..126: mol_type = other RNA
atgagggcaaacaggatgaagccggcgaacacaacatcgagcttgtcgaagcgggagaagatgcggcggtagcctttgagccgacggaagaggcgttcgatttcatttctgcggcggtataaaacc

SEQ ID NO: 598 - RNA, 129 nt, synthetic construct
  source 1..129: mol_type = other RNA
caaggttaccaacgcctttcagccaccggggcgctcctgccggctgcgcttcgtccgtctttccccgaaattgccgtcgattgtggcgatctccccgagaggcttgctctgcgggggttggagtcagcc

SEQ ID NO: 599 - RNA, 68 nt, synthetic construct
  source 1..68: mol_type = other RNA
cagaacaccgttccagccgcgcccagaaccacggcgcggatttcgcggttgcggccgatttcctccag

SEQ ID NO: 600 - RNA, 125 nt, synthetic construct
  source 1..125: mol_type = other RNA
cgcatgatctcatcgcgcttctcgcgggcagcctctccccccagcgcctcgaccatctcgtctcggaacagtcgccgatacacgtggcggatcgatccgggactccgggggaactcctcccgatc

SEQ ID NO: 601 - RNA, 125 nt, synthetic construct
  source 1..125: mol_type = other RNA
tcgctgccgtcagcacgaggagacgagcaggaagctccacgagtccctctccaagcatgagaaggatgctcggaaggccttcaagacgctgaacctcgacccctcgatcatctgggatcgggagg

SEQ ID NO: 602 - RNA, 139 nt, synthetic construct
  source 1..139: mol_type = other RNA
ctcccgatcggcttcgtagatcagacctgacgcagaaatggccggtagctcggtgtccgactccccatagcctcctgaatggcttcgtaattcagactggatctatcgccactgggcctcccgattggcttcgtagatc

SEQ ID NO: 603 - RNA, 125 nt, synthetic construct
  source 1..125: mol_type = other RNA
actcatgattaaagataaaagttctacagtaacacttgcaaaataatattataaaaaggagagtgaaactctccttaaaatttaagtaattatatttccgttattatctgtgaaagttctattta

SEQ ID NO: 604 - RNA, 124 nt, synthetic construct
  source 1..124: mol_type = other RNA
ttatttaaaggtcttaaagattttaactcagcttgtaaatcataaatatctttaaaaaaaacgctcatttcctactccttttatttactataattatttatatcatatcatataatatttaaat

SEQ ID NO: 605 - RNA, 124 nt, synthetic construct
  source 1..124: mol_type = other RNA
tatttaaaggtcttaaagattttaactcagcttgtaaatcataaatatctttaaaaaaaacgctcatttcctactccttttatttactataattatttatatcatatcatataatatttaaata

SEQ ID NO: 606 - RNA, 132 nt, synthetic construct
  source 1..132: mol_type = other RNA
acgcttggcatagcagagagcaccgtagagtcgcagatgcgcattgcgctgcgcacgttgcgtcgcagcttcgccgtgtaacagcccatgtcgcaagacggacaataaccccgaccacacacattgattgca

SEQ ID NO: 607 - RNA, 132 nt, synthetic construct
  source 1..132: mol_type = other RNA
tcaggctctctattcattgttgatgttgtctgcctgtggcagaacaggcggcgcaaggattgttatcggtgcggcgcagtgattgtgataatgtcctctttggtgttgtgttgtgtgcaatcaatgtgtgtg

SEQ ID NO: 608 - RNA, 123 nt, synthetic construct
  source 1..123: mol_type = other RNA
gttgcgagcatgggaatccgcagtgcgacccataagcgcgcagaataagagtatagcattcgcactgcaatcaatcggtcgattgtccgtccgaggctgtcgttaatgacatcataggatgtt

SEQ ID NO: 609 - RNA, 126 nt, synthetic construct
  source 1..126: mol_type = other RNA
cgataattccgcggcaccatcgctatttaacggcgattttgaaggtgcactaaatgaaagcttcgagcgtttccgttttggtggagtgacgccaagtaagcaagaagtgttctttattaatttaca

SEQ ID NO: 610 - RNA, 126 nt, synthetic construct
  source 1..126: mol_type = other RNA
atcggtaatcgcgatggagtagctaccatgagcgcgcacgaataattccgcattgtaaaaattatcgaaatagttgatcggttgctgcgtaccaaaacgaatgccgcgaatttcttgtaaattaat

SEQ ID NO: 611 - RNA, 132 nt, synthetic construct
  source 1..132: mol_type = other RNA
accaactcggcattcacgaactccacggcaccaaaatcgtaaaactagcagaataacccaaccaacctccctaaagcccctgcgaaaaggtcgcgcagaagcttggggaggttggtttacatcattctcaaa

SEQ ID NO: 612 - RNA, 124 nt, synthetic construct
  source 1..124: mol_type = other RNA
agtattgcgcggatataattttgtagatccttgatataatgcattttcaatcgtatatcgttcttgatacaaaatatgaagtgcccgatacacatcttccaattgataagtagattgatgtaaa

SEQ ID NO: 613 - RNA, 124 nt, synthetic construct
  source 1..124: mol_type = other RNA
gacgtttggctgctactgcttggttcgctcccttgccaccacctgcagaaaagatttcttttgtatgcatcgtttcaccaatttgtggcatatgacttaagcgaatcgtacggtctaaattaat

SEQ ID NO: 614 - RNA, 14 nt, synthetic construct
  source 1..14: mol_type = other RNA
tcttaaaatagcac

SEQ ID NO: 615 - RNA, 126 nt, synthetic construct
  source 1..126: mol_type = other RNA
cgataattccgcggcaccatcgctatttaacggcgattttgaaggcgcactgaatgaaagtttcgagcgtttccgttttggtggagtgacaccaagtaagcaagaagtgttctttattaatttaca

SEQ ID NO: 616 - RNA, 126 nt, synthetic construct
  source 1..126: mol_type = other RNA
atcggtaatcgcgatggagtagctaccatgagcacgcacgaataattccgcattgtaaaaattatcgaaatagttgatcggttgctgcgtaccaaaacgaatgcctcgtatttcttgtaaattaat

SEQ ID NO: 617 - RNA, 124 nt, synthetic construct
  source 1..124: mol_type = other RNA
gacgtttggctgctactgcttggttcgctcccttgccaccacctgcagaaaagatttcctttgtatgcatcgtttcaccaatttgtggcatatgacttaagcgaatcgtacggtctaaattaat

SEQ ID NO: 618 - RNA, 134 nt, synthetic construct
  source 1..134: mol_type = other RNA
aaacaacgattaaagcaagcaaggataaattaaccattgcttcttataatattgaaaacttctcagcaaataaagcgtccacaagtgatgaaaaagttcaacgcattgcccaatcgtttgtgaatgatttaaat

SEQ ID NO: 619 - RNA, 132 nt, synthetic construct
  source 1..132: mol_type = other RNA
cgcaggatacgctgtctgcagcgattgtcggcagtagtatcggttctacgaacgcccagagccatcggcgggtggcgtgccagaggcgccaatgcggtctggctggggctggcgcgtagtggcaagtggagg

SEQ ID NO: 620 - RNA, 132 nt, synthetic construct
  source 1..132: mol_type = other RNA
actcggcgctgctggtgctgcgcgtgctggaaacgctgggtgaggggtgaggggtgagaggcactggcgaatagtggcgaccccgactgggctcgaaccagtaaccttcagctcccctccacttgccactac

SEQ ID NO: 621 - RNA, 125 nt, synthetic construct
  source 1..125: mol_type = other RNA
ccgagttgcggcttgttagcccctcgcacagcgcgtgccagtcgcgctcgccggcccagatgcgccgcgtggcatcggcaatctgccagccgtttgcctcaagacgtgggaggcgctcctccact

SEQ ID NO: 622 - RNA, 124 nt, synthetic construct
  source 1..124: mol_type = other RNA
cgggataggacccgtggaattttgtgcttgccggagctctgaagaagtcgcagttaggcgagagcaagaactcgagaagcttatctgctccttctctcttgatcttatccttgaaaatttctac

SEQ ID NO: 623 - RNA, 124 nt, synthetic construct
  source 1..124: mol_type = other RNA
ataaggctttattaaaacaaaacactattatataagaaaaaaaggagaaaacattatgacaaacaataacattaacaacaacacaatcgatagagaagcggtacaggcccgtttcgtagaaatt

SEQ ID NO: 624 - RNA, 124 nt, synthetic construct
  source 1..124: mol_type = other RNA
agaaaaaacaacatgccgaattacgattacatcgacagacaaaagttagggataggcaaggcggacagaaatgcgtttgccgttcccgagtacgcagacggttggaacggcgcgatagaaatta

SEQ ID NO: 625 - RNA, 131 nt, synthetic construct
  source 1..131: mol_type = other RNA
cgcgagcgcaagggccgcgtgaaatgtccagggcctgtggccggacagcgtggaagcagtcggatcgatatctcgtcgctttgggacaaccaggccgagcagatgtgattgcgaaagcgtcgtggcaagtg

SEQ ID NO: 626 - RNA, 131 nt, synthetic construct
  source 1..131: mol_type = other RNA
cagagctgctacccgtgaggtagatggcagcacctgtagtatatgtcaacagctcgttgctggcaaccagacaagtcctgattatagaatagggattcgaacccccgacacccctcacttgccacgacgct

SEQ ID NO: 627 - RNA, 130 nt, synthetic construct
  source 1..130: mol_type = other RNA
gcgaggatccacggcaagttggtcgacaagctggacctgtcccgcgtcggcgacatgaagggcgacacgctccgccgcgaaatccgcgtggtcatcgaacacctctgcgacgccgacgacgcgctgttga

SEQ ID NO: 628 - RNA, 125 nt, synthetic construct
  source 1..125: mol_type = other RNA
cgcgggcggccttcagatccttcttggtgaaattcccgaccggcaggggcgtacacagggacagcacctcccggaagctccgcccgaactcgaccagttccttcgacggcttgccgttcggcagg

SEQ ID NO: 629 - RNA, 125 nt, synthetic construct
  source 1..125: mol_type = other RNA
ccgtgctggcggagttggccgggctggcggagccccccggccgtcctgccggggggctgctgacggtcggcgggttcgtgcggcggttcatggagcacgcgaaggtgtactaccgcctgccgaac

SEQ ID NO: 630 - RNA, 126 nt, synthetic construct
  source 1..126: mol_type = other RNA
catgtcccggagttgtcgtcgcaagtctttgatgtccgttcgctcccatttctcagtcctcttctggggttgaggtttcattcgatccggcccatttgtcatccaccagctcgaccccctcgcggg

SEQ ID NO: 631 - RNA, 124 nt, synthetic construct
  source 1..124: mol_type = other RNA
ttttaagcgatgcaagatacgctgatcaagtcgagaagtataacctattgaaaacagttaatccctcgaggataatcagcctactcgacagactagccgataacggaataattaataggaagaa

SEQ ID NO: 632 - RNA, 124 nt, synthetic construct
  source 1..124: mol_type = other RNA
tccaagtagcgagccaagggttccggaaaggtaggcaattggtactccgtaaaccgggttatcaacgagtagtattgttgttaaaacagctgttaatgaaggtatgaatcccgggacaacgatc

SEQ ID NO: 633 - RNA, 139 nt, synthetic construct
  source 1..139: mol_type = other RNA
acaaaaagtaataatccaggcatatctacgacaccgcctagcactttcagttcttcctagttgttacgcagaatcataggaaacattgaatggcttgaacacctagcagaacaatctttcagttcttcctagttgttac

SEQ ID NO: 634 - RNA, 135 nt, synthetic construct
  source 1..135: mol_type = other RNA
gaagctgggctacaccatcaagcagggcggcaagcgtgtctccgataagaccctaaaggaagctcaggacgacggtacaggacagttcatgctgggcctgtagcaaaacacctacaaatttctgctgttgcagat

SEQ ID NO: 635 - RNA, 134 nt, synthetic construct
  source 1..134: mol_type = other RNA
aagctgggctacaccatcaagcagggcggcaagcgtgtctccgataagaccctaaaggaagctcaggacgacggtacaggacagttcatgctgggcctgtagcaaaacacctacaaatttctgctgttgcagat

SEQ ID NO: 636 - RNA, 134 nt, synthetic construct
  source 1..134: mol_type = other RNA
tgagtggtcattccccgagaagggtctcgaaagattgctcctaatccctacaagatgtgcattttgtggggcaaaggagcgggggccatcgggtttccacgtaatatcctttaatatctgcaacagcagaaatt

SEQ ID NO: 637 - RNA, 124 nt, synthetic construct
  source 1..124: mol_type = other RNA
caagtggctaatgaactaacaaagacaccatcaatcataatcactgaggaacttggtgagaacccgcaggagtcgatgattgaggatgttgggaaggacgagttgaggcaccgcataaaacaga

SEQ ID NO: 638 - RNA, 124 nt, synthetic construct
  source 1..124: mol_type = other RNA
cgttgcgaataatgttacgggtgcgaataaactccagaggttattctacaataagtataggctggagtacccaagccttaactcacaattaatcatccaagcaatcaggcaggcatctgaaatc

SEQ ID NO: 639 - RNA, 124 nt, synthetic construct
  source 1..124: mol_type = other RNA
cttgtgaagtgtattgggcataccctactgtttctgtatgatgatacgtggaatagtttggatccgcgctccaaagccttatcctccacagccctcaccaacgccttgaatggtgtctgtttta

SEQ ID NO: 640 - RNA, 124 nt, synthetic construct
  source 1..124: mol_type = other RNA
acttttctgcttggaggatttgtcgccggaataccgatcattgtttacgatgaacctataaacgctttattcgagggaatatcggcaattacaacgaccggattatctagtttgaatcagaatt

SEQ ID NO: 641 - RNA, 124 nt, synthetic construct
  source 1..124: mol_type = other RNA
atattataggccgccgatcctggtgatactaggaacgatacagtaaggagcgctattccaagccctcctatccattggtaatatgatctgagaaaatgtactccaggggttagagaattctgat

SEQ ID NO: 642 - RNA, 124 nt, synthetic construct
  source 1..124: mol_type = other RNA
actcatagtaacccctgaccacttactcgtagacggggatactcttgaatggaaacaagcctttgaatttaagaaaggggataaagtactttcaatacaaaaaataccgggacacaacaacgat

SEQ ID NO: 643 - RNA, 129 nt, synthetic construct
  source 1..129: mol_type = other RNA
aaaagatcttcagaaaaataagtgagattctcaatacaaatctttcctcctcaaagctctgcgaaactctcatcacgatcagagatgttctcatgaagagtgatgatgatttcatcagaagatttgaag

SEQ ID NO: 644 - RNA, 124 nt, synthetic construct
  source 1..124: mol_type = other RNA
agtttataagcttcttaacaactattgttattgggatagtaaaaatatgatagacatggttaaagaaggcatcaaagaggatcttgtgaagctatatgacaacatatcctcatcatcagttgtt

SEQ ID NO: 645 - RNA, 125 nt, synthetic construct
  source 1..125: mol_type = other RNA
ctgatcgatgctcctataaggcttgaggttggcgatatgatatttctagaatgttcatctaaatatcttgagatccttaagaaggcatcggcatacagctcatatctatcgttcacatctcaaat

SEQ ID NO: 646 - RNA, 124 nt, synthetic construct
  source 1..124: mol_type = other RNA
gagagagatgctgagagattctgaaagctaagaaggcagtcccaagataatgttgaagacctgaagtcgagtagaacttcgggtttgaggctatgataggaaaatagaagtcctcaacaactga

SEQ ID NO: 647 - RNA, 64 nt, synthetic construct
  source 1..64: mol_type = other RNA
ggtacaaaaaccagttgtgtatccaaagcttcttctaaacatggcatcagagcctgatgatgtt

SEQ ID NO: 648 - RNA, 127 nt, synthetic construct
  source 1..127: mol_type = other RNA
cttgttttatacaatgagagcaatggctatgcagctatcaaagagcttgattatttaatgaatcttagaagtgcaaaagagagatttaagcaagtttatgacgagggatttgtagttgatactgatg

SEQ ID NO: 649 - RNA, 124 nt, synthetic construct
  source 1..124: mol_type = other RNA
tgttacctttatactaataccccttgtatgagctgcatctgtatataaagtataacgcccaccattaacatttaccttatttacaggctcttttgaattaccataataaaacttagtattactt

SEQ ID NO: 650 - RNA, 126 nt, synthetic construct
  source 1..126: mol_type = other RNA
cagaacctatttataaaatatcaattaattctgatttagatgtagataagctacctaaggctagagtatttgagcctgaagaattcaataaaggttggaaaactgtaaataactcttggtattact

SEQ ID NO: 651 - RNA, 123 nt, synthetic construct
  source 1..123: mol_type = other RNA
tcaacaataataatattattaatgtcagtaacaaatgcaccagcatagcttatattgctactaccaccaactaatactttaggcttttcaataaatttgcgtgcgtaaagaataccaccttca

SEQ ID NO: 652 - RNA, 123 nt, synthetic construct
  source 1..123: mol_type = other RNA
aagctatgctggtgcatttgttactgacattaataatattattattgttgatgctaatggctacatactgatagagggttaatgaatagaggtatgttttaaatgacacaactaaatgcatta

SEQ ID NO: 653 - RNA, 130 nt, synthetic construct
  source 1..130: mol_type = other RNA
aactgctgatgaccctgaccaaaagattcgttctaatggttatgtagttcaagttggggcatatggtaagagttctattatgacaggtgcaaaatctcaaaatgtaggtaagaagtctcatactgaaggt

SEQ ID NO: 654 - RNA, 127 nt, synthetic construct
  source 1..127: mol_type = other RNA
tctcggtatcgacgagtttcgtgacttttagcttctgcacgcggtagctaatacgctggcagtagtggcggcttgctgctgatcgttcgtagaatgtggcgtcgatagcagcatgttcagacggatc

SEQ ID NO: 655 - RNA, 127 nt, synthetic construct
  source 1..127: mol_type = other RNA
ggagatcggcctcagcgcggccgatctcccttcgccgtccacgttgtgtaaagcgttcgaccggatcgagatgagcgtctgtcgagtgctactgcgccagtcggcgcagttgcacgatccgtctgaa

SEQ ID NO: 656 - RNA, 127 nt, synthetic construct
  source 1..127: mol_type = other RNA
accggtcgatcgcgacgaggcctgcggcctccagatccgccacgtagcgatcgatactggcgtcggcgtagtcgatctgggtatctcgcttcagcgcccgcactgagcgctcgctgtcggcgtcgag

SEQ ID NO: 657 - RNA, 126 nt, synthetic construct
  source 1..126: mol_type = other RNA
acgcagcctcctggaggccatatcaaacagcacgcaccgccaacacgaccctacggcgttattttcgagatcgccaacgagaccgatttcttcgagatcccgcccgatcgctactacgagttcggc

SEQ ID NO: 658 - RNA, 66 nt, synthetic construct
  source 1..66: mol_type = other RNA
atgctgtcggcgctgttcgcgagcgatgagccactcgatcgacaggcgctcatcgaagtcacgagc

SEQ ID NO: 659 - RNA, 125 nt, synthetic construct
  source 1..125: mol_type = other RNA
tttcctaatacaagaatcactagtaatcagctcaaaagaaagcctaaagcatgaataggatgcaaattgtttgatatatagaaaaatcgctaacttatactaaagataaaagtatccttatggaa

SEQ ID NO: 660 - RNA, 130 nt, synthetic construct
  source 1..130: mol_type = other RNA
aaaacgcggaagaagcctaaactcctggttattatagtgatataatgaatcgttacgatattggcctccaaaccagaaaccaatgtccatcaccgtcccattatttagagatttgatttcatttccataa

SEQ ID NO: 661 - RNA, 127 nt, synthetic construct
  source 1..127: mol_type = other RNA
aaaatgacttagcatatttggatagtcgtatgagcgttttgattcaagaaatgttctcatctgatttgtgcgctgttgtgatgacgaaggatcctgtagaactagaagaagtctttggaattgaaat

SEQ ID NO: 662 - RNA, 129 nt, synthetic construct
  source 1..129: mol_type = other RNA
aaagagaataatgattacgggagctgccggttcaattgggcgtgaaatggtgaggcagatagccggattgaatccatataaattaattttggttgatcaggcagaatcacctttgcataatgtacaatt

SEQ ID NO: 663 - RNA, 118 nt, synthetic construct
  source 1..118: mol_type = other RNA
aaatttattgatatgtatgccggacgcctgcggaatcaagtctcttttatgttgagtgcctgcaacttctatatgcctatctttgaggaggcccttgatgcgtataatttaccattgg

SEQ ID NO: 664 - RNA, 126 nt, synthetic construct
  source 1..126: mol_type = other RNA
aaaaatagaatctttcaaagccaatgctaactctaaggcttgatcgagataaaacaaagcttccttttcttttccttcaacaacacgcacccatcccatattcgaaagagaatacattaatacttt

SEQ ID NO: 665 - RNA, 126 nt, synthetic construct
  source 1..126: mol_type = other RNA
aaacatagtggcaagccccatgcccataccattaatggccgaggaagtcgtaccgagtgtaggacacataccaagcaggagcacaaatgtcggattctctttaacaatcccattcattaatacttt

SEQ ID NO: 666 - RNA, 126 nt, synthetic construct
  source 1..126: mol_type = other RNA
aaagaagctgacgcctacaaatccctctttgaaaaaatgggtattgaaaacattgtctataacatagcaatgtgctccaaaaaccattattgcaaatatgaatctcaacgatgttaaagtattaat

SEQ ID NO: 667 - RNA, 126 nt, synthetic construct
  source 1..126: mol_type = other RNA
aagcatacttcttgattcatactaactatactttccatatatttgcagtattcaacacacacatcacatctttaatgatgaaaataaaaaaacgataagacaatacgaaattatgattaatacttt

SEQ ID NO: 668 - RNA, 102 nt, synthetic construct
  source 1..102: mol_type = other RNA
aaggaaatttattgttttgacgatttacaaattaattgtccgaaggaaccattcttcgggacaataagtcacaaatacccggaacatagttgtctatgtctc

SEQ ID NO: 669 - RNA, 126 nt, synthetic construct
  source 1..126: mol_type = other RNA
caaggggttaactttgctttatttccaatatatctacgactctccaaatcaaacatcttataccccaaaagagtgacatctatatcagttcgattatagacttcttgtaatgacaatttcaattcc

SEQ ID NO: 670 - RNA, 126 nt, synthetic construct
  source 1..126: mol_type = other RNA
cagataattgtgttttccgataccttcattgtctgccgacatattgaataggatttccgccccttgtaaagctagcgatgagctgggaggaatcgtggaccatagatcttcacaaatttcaattcc

SEQ ID NO: 671 - RNA, 126 nt, synthetic construct
  source 1..126: mol_type = other RNA
cagctattatccctgcaacaattcaaaaatatgtaacgaccaattatcccgatgctaaaatcctgaaaatagagagggataaaaaagattatgaagtaaaactgtccaaccgtacggaattgaaat

SEQ ID NO: 672 - RNA, 126 nt, synthetic construct
  source 1..126: mol_type = other RNA
cccaaatcatcttaccaagagaaccataatcattcttcaaggcgtctacatgattaccaccagccgcagctattacttcgtccttagatactggcaatcttcttggattattaccggaattgaaat

SEQ ID NO: 673 - RNA, 113 nt, synthetic construct
  source 1..113: mol_type = other RNA
cgtaaaccggcagacacacatgtaaattcgcgggtaaacacgttgacggatagatgcttccaaaagcgcatagcagcaccaatgttccaaccatgcgtatcatattccgccat

SEQ ID NO: 674 - RNA, 126 nt, synthetic construct
  source 1..126: mol_type = other RNA
ctttagaaataatgtgtcgatcaagaataatataaaaaacataggttagcgacataggtactaaacatctatatatcaacatgtcatagagcgtttccgttactttaccattgataattcacaata

SEQ ID NO: 675 - RNA, 125 nt, synthetic construct
  source 1..125: mol_type = other RNA
cctaaaccaatacagaaggtccttgaaacactgataaaatgccctagatgcggaagccaaccaagctatggagaaaaatactgcaaacaatgcggagcaagaatcccaacaaaagcatgggaaac

SEQ ID NO: 676 - RNA, 129 nt, synthetic construct
  source 1..129: mol_type = other RNA
cctctaccgaggttgccagtttagatgctgagcgcataacctccctctcaaaaaccctctcatccacatccaacaacgccagcctaatagcctctctcctgaaggcttcaagaggaacacccatatcat

SEQ ID NO: 677 - RNA, 129 nt, synthetic construct
  source 1..129: mol_type = other RNA
ggcgaaaaaccgcagccgcagcagccagctccgcctacaaggggggtaacggctcctgagcctgttcctgcaggggttgattgggagcctgatgaagacatggttgaggcttttgatgatatgggtgtt

SEQ ID NO: 678 - RNA, 126 nt, synthetic construct
  source 1..126: mol_type = other RNA
acgagtaagaaacgaacacgaggcctacggattgcattttgcggaagtttggttgcaactgcccgactacgacaactacgaactgcaagccaccgtcgtacttgacagtttgctcactgagtcgcc

SEQ ID NO: 679 - RNA, 125 nt, synthetic construct
  source 1..125: mol_type = other RNA
cctctgcagctgagattgttacaggtgcgatacaagaccaagacagaggtatggtggtgggaagacgttcctttggtaagggacttgtacagcgcccggttgagtttcaggatggaagtatgatg

SEQ ID NO: 680 - RNA, 124 nt, synthetic construct
  source 1..124: mol_type = other RNA
cgacgtacaatatcttctcttgacatcttcacccctgcgatagcggtatcgtttaccataacaatacggtcgccggcaagtatccccaccttctcagaaggtccgttggtaaccggttgaataa

SEQ ID NO: 681 - RNA, 129 nt, synthetic construct
  source 1..129: mol_type = other RNA
aacacattgtctgaacttcttctaattcctgttctgttgtaataaacaaagttggttcatttgttctgattttaatccatccaaaatcactataaatttcactacaagagaaataacaagcatcagcaa

SEQ ID NO: 682 - RNA, 129 nt, synthetic construct
  source 1..129: mol_type = other RNA
gaagtaggagttcctttatatggacctttaattaacacagtaactagaggcgcaagattaaagaaattctatctgcggtccgcagcttctggagtcggcaaatcaagaacaatgattgctgatgcttgt

SEQ ID NO: 683 - RNA, 129 nt, synthetic construct
  source 1..129: mol_type = other RNA
ttacggatttccacaacgtcgtctgttacaagacggtgaccgcgctttacaagttccaaagcagcctcagatttaccgatgccgctctcaccagtaatcaatacaccttcaccgtaaacatcaacaagt

SEQ ID NO: 684 - RNA, 125 nt, synthetic construct
  source 1..125: mol_type = other RNA
caccttatccatggcaatttgctcttcggaaagcgggccgagcggtttaccttgttcagaaggagaacggcgagcagcaaaggagaacagaccggcggaatcagcaggagcccctttgctgatgt

SEQ ID NO: 685 - RNA, 125 nt, synthetic construct
  source 1..125: mol_type = other RNA
gaatgtgcctacgctgcgaataaggcggtgggtgaggttttgcctgtaccccggactcagggtgaccgaggcggaaagaagtatctggtggaactgtggcccaccaagcagcaatacatcagcaa

SEQ ID NO: 686 - RNA, 124 nt, synthetic construct
  source 1..124: mol_type = other RNA
tcctgaaaaagacgatgcgtatcgtagatggcatcatagggagagtactgtgcattctgtcgcaaatcatcatcctcaaattcagcattgatgatgcgaccttggtaaattctgttgatgtttg

SEQ ID NO: 687 - RNA, 137 nt, synthetic construct
  source 1..137: mol_type = other RNA
agcttcattccgtggaagtgccccaaaaaggttgcacggcatagtcggatttggttcccgtgcaattcttgctactcaccagccggcgtgccccaccggatactcaggctccatatttggtgcccgtgcaaattctt

SEQ ID NO: 688 - RNA, 137 nt, synthetic construct
  source 1..137: mol_type = other RNA
gtcgttttcatagtataattggcgcgggcactcacagaatagtgctggataaaagagtggcgccttcctccttcttcgaaaaataagagatacggggtttgcgttgttgagtagcaagaatttgcacgggcaccaaa

SEQ ID NO: 689 - RNA, 124 nt, synthetic construct
  source 1..124: mol_type = other RNA
tgaaaaaattatttgtggttgtcaacacagatacccaacgggccattcgcgcttttgtgagcgagtcccgagcggatgattacgctgacgatctatacgaaaaaacgaaccaggatacccgtgt

SEQ ID NO: 690 - RNA, 127 nt, synthetic construct
  source 1..127: mol_type = other RNA
cgcgcgggaggcctggacggacaagatcgcctcggacaccgtcaagacggccctgcggctcggggtgagcgtcatcgcggtgtacaaggacgaggactccaccccctcgcaggtgcgtcccgcccac

SEQ ID NO: 691 - RNA, 127 nt, synthetic construct
  source 1..127: mol_type = other RNA
cccggtggccgacgcccttgctgacgaccttgacctcgatgccgtgcagcggcgccaccagggcgatctggtcggcgatcgcacggcgcgcctcggtggccagacgccggttgatgtgggcgggacg

SEQ ID NO: 692 - RNA, 125 nt, synthetic construct
  source 1..125: mol_type = other RNA
cgggaccttcagcaccgcggcggtcacccgccgctcctgggcaagggcgagggctgcgagcccgccgccgaagctgacgccgtggatgtcgatgcggcgcaggtcagggtacagggcgtgggcgg

SEQ ID NO: 693 - RNA, 125 nt, synthetic construct
  source 1..125: mol_type = other RNA
agcgtccagccggacgtgcccgacgtcgtggccgagcacgtcctgcacggcatcgcctcgcgcgagacgtacatcatcggcgggtgcgtccaaggcgtgtgggccgcggtctcagccgcccacgc

SEQ ID NO: 694 - RNA, 66 nt, synthetic construct
  source 1..66: mol_type = other RNA
aggtacatggccacgtggtagatcgcctggatgtccgtcttggtcgggtcggacgtgtagtagatc

SEQ ID NO: 695 - RNA, 131 nt, synthetic construct
  source 1..131: mol_type = other RNA
catggtgaaactggcagactcccactgaaccattgggaacaggatacccgtgctggccgagctttgccaggatagcaggcgccagcaactggccttttgctgtaggtataccgtccttcaatgcggccccc

SEQ ID NO: 696 - protein, 1139 aa, synthetic construct
IFVVLSVNQFRCNPNAFRQASMKTDDEKKDTAIKSYTSWLLPNDRKEKDMVRSFLALDQGSRFFFDLMQAWYGGLTPDIIKSVTKERDLVDLWCAIYWFRPMKKELASHPIDRVDLAKTFQRYYGGPASDVVQEYLSASIGEDCCWNDCRQKYQEFCKNLGVDFTPDLKTLVREKLIAVALNDGSQAAISNLFGNGGKEDRNVKVNICKKILIALEKAGKSVKYVRDVQSIILKCANAKDREDFNRIYADKNGRPGTLLLLLDRKGENTYDAEVLKRYLRKTIKSKNAPLVWNYNQKLFEYIERGIRNLLRRTINYDAWAWGEMWRVGHTPLQTKATRNYHFAQEQLKRHSDIAAASQSSHAIAVALNEFFESPFFDGENPFTICPHHLGKNLEKLFKAWADEKNQTDEEDAGETAITDYCAEFKDGFDREPIRNLLRYVYASLRSKYSAKELIQAAKYNQQFERYQRQKAHPVTPDNQGYTWPEAVIKPSKAERKNRENSLDTRIWVSVKLLQKDGTWEKHHIPFYNLRFFEEVYAAASIAEDMPSPTFRNSRFGFKLPKLLNTHAKINKKKKDGKKDKKAVNAAKREARIYLAAKEGRLPAPSVPLDKLSAVIARVNGKFQVTVPVKFKVNKQPKYPLPQLGQIILGYDQNLTANHAWALFEVVTEDTPGAHFCRNQYLRVLKTGQVRSITKTKDGQEIDQLSYDGLEYKEYGEWRKQAKKFASQWYITTKVRKGKETTLLSQPALERFESIEKYKPALYRFNKEYARLLLAVIRRKTLNELEEIRPEIFRLVEQGFGICRFGSLSLSSFEAIRAAKAVIYGYFSTALKHDHNTPITDDERQAFDPELFGLLNKLETLRQNKGEEKINRAANALIRIALENKADFIRGEGDLPTTNKSVKKGQNSRSMDWLARGLFNKICQLAVMHNIIPTAANPHSTSHQDPFEHNKDFDDPQPAMKCRYAEFKIEDIGDSVLERLGTSLRNAKAGQTGAYYYKGAQDFLAHYGLQDIEEELKKCRRGRKANMPCWELQKRLIQKLGSKDAVVYIPMRGGRIYLATHSVTTGAKPIIFNGEEVWVSNADEIAAVNIGLTIIPTSKKDEEHPDRENDDKAIRKSVRRPRKSGERRSGDKMPATARKT

SEQ ID NO: 697 - DNA, 9375 bp, synthetic construct
  source 1..9375: mol_type = other DNA
gacggatcgggagatctcccgatcccctatggtgcactctcagtacaatctgctctgatgccgcatagttaagccagtatctgctccctgcttgtgtgttggaggtcgctgagtagtgcgcgagcaaaatttaagctacaacaaggcaaggcttgaccgacaattgcatgaagaatctgcttagggttaggcgttttgcgctgcttcgcgatgtacgggccagatatacgcgttgacattgattattgactagttattaatagtaatcaattacggggtcattagttcatagcccatatatggagttccgcgttacataacttacggtaaatggcccgcctggctgaccgcccaacgacccccgcccattgacgtcaataatgacgtatgttcccatagtaacgccaatagggactttccattgacgtcaatgggtggagtatttacggtaaactgcccacttggcagtacatcaagtgtatcatatgccaagtacgccccctattgacgtcaatgacggtaaatggcccgcctggcattatgcccagtacatgaccttatgggactttcctacttggcagtacatctacgtattagtcatcgctattaccatggtgatgcggttttggcagtacatcaatgggcgtggatagcggtttgactcacggggatttccaagtctccaccccattgacgtcaatgggagtttgttttggcaccaaaatcaacgggactttccaaaatgtcgtaacaactccgccccattgacgcaaatgggcggtaggcgtgtacggtgggaggtctatataagcagagctctctggctaactagagaacccactgcttactggcttatcgaaattaatacgactcactatagggagacccaagctggctagcgtttaaacttaagcttaccggtgccaccatgccggcagctaagaaaaagaaactggatggcagcgtcgacatcttcgtggtgctgagcgtgaatcagttcagatgcaaccccaacgccttcagacaagcctccatgaaaaccgacgacgagaagaaggacaccgccatcaagagctacacaagctggctgctgcccaacgacagaaaggagaaggacatggtgcggagcttcctggccctggaccaaggcagcagattctttttcgacctgatgcaagcctggtacggcggcctcacccccgacatcatcaagagcgtgaccaaggagcgggacctggtggacctgtggtgcgccatctactggttcagacccatgaagaaggagctggcctcccaccccatcgacagagtggacctggccaagacctttcagagatactacggcggccccgcctccgacgtggtgcaagagtacctgagcgcctccatcggcgaggactgctgctggaacgactgcagacagaagtaccaagagttctgcaagaacctcggggtggacttcacccccgacctcaagaccctggtgagagagaagctgatcgccgtggccctgaacgacggcagccaagccgccatcagcaacctgttcggcaacggcggcaaggaggacagaaacgtgaaggtgaacatctgcaagaagatcctgattgctctggagaaggccggcaaatccgtgaagtacgtgcgggacgtgcagagcatcatcctgaagtgcgccaacgccaaggacagagaggacttcaacagaatctacgccgacaagaacggcagacccggcaccctgctcctgctcctggacagaaagggcgagaacacctacgacgccgaggtgctgaagagatacctgagaaagaccatcaagagcaagaacgcccccctggtgtggaactacaatcagaagctgttcgagtacatcgagagaggcatccggaatctgctgagaagaaccatcaactacgacgcctgggcctggggcgagatgtggagagtgggccacacccccctgcagaccaaggccacaagaaactaccacttcgcccaagagcagctgaagagacacagcgacatcgccgccgcttcccaaagcagccacgccatcgccgtcgctctgaacgagttcttcgagagccccttcttcgacggcgagaaccccttcaccatctgcccccaccacctgggcaagaacctggaaaagctgttcaaggcctgggccgacgaaaaaaatcagaccgacgaggaggacgccggcgaaaccgccatcaccgactactgcgccgagttcaaggacggcttcgacagagagcccattagaaacctgctgagatacgtgtacgcttccctgagaagcaagtacagcgccaaggagctgatccaagccgccaagtacaatcagcagttcgagagatatcagagacagaaggcccaccccgtgacccccgacaaccaaggctacacctggcccgaggccgtgatcaagcctagcaaggccgagagaaagaacagagagaacagcctggacacaagaatctgggtgagcgtgaagctgctgcaaaaggacggcacctgggagaagcaccacatccccttctacaacctgagattcttcgaagaggtgtacgccgctgcctccatcgccgaggacatgcctagccccaccttcagaaacagcagattcggcttcaagctgcccaagctgctgaacacccacgccaagatcaacaagaaaaagaaggacggcaagaaggacaagaaggccgtgaacgccgccaagagagaggctagaatctacctcgctgccaaggagggcagactgcccgccccctccgtgcccctggacaagctgagcgccgtgatcgctagagtgaacggcaagttccaagtgaccgtgcccgtgaagttcaaggtgaacaagcagcccaagtaccccctgcctcagctggggcagatcatcctgggctacgatcagaacctgaccgccaaccacgcctgggccctgttcgaggtggtgaccgaggacacccccggcgcccacttctgcagaaatcagtacctgagagtgctcaagaccggccaagtgagaagcatcaccaagaccaaggacggccaagagatcgatcagctgagctacgacggcctggagtacaaggagtacggcgagtggagaaagcaagccaagaagttcgcctcccaatggtacatcaccaccaaggtgagaaagggcaaggaaaccaccctgctgagccaacccgccctggagagattcgagagcatcgagaagtacaagcccgccctgtacagattcaacaaggaatacgcccggctgctcctggccgtcatcagaagaaagaccctgaacgagctggaggagatcagacccgagatcttcagactggtggagcaaggcttcggcatctgcagattcggcagcctgagcctgagcagcttcgaggccatcagagccgccaaggccgtgatctacggctacttcagcaccgccctgaagcacgaccacaacacccccatcacagatgacgagagacaagccttcgaccccgagctgttcggcctgctgaacaagctggaaaccctgagacagaacaagggcgaggagaagatcaacagagccgctaacgccctgatcagaatcgccctggagaacaaggccgacttcatcagaggcgagggcgacctgcccaccaccaacaagagcgtcaagaaggggcagaacagcagaagcatggactggctggctagaggcctgttcaacaagatctgtcagctggccgtgatgcacaacatcattcccaccgccgccaacccccacagcacaagccaccaagaccccttcgagcacaacaaggacttcgacgaccctcagcccgccatgaagtgcagatacgctgagttcaagatcgaggacatcggcgacagcgtgctggagagactgggcacctccctgagaaatgccaaggccgggcagaccggcgcctactattacaagggcgcccaagacttcctggcccactacggcctgcaagacatcgaggaagagctgaagaagtgcagaagaggcagaaaggccaacatgccctgctgggagctgcagaagagactgattcagaagctgggcagcaaggacgccgtggtgtacatccccatgagaggcggccggatctacctggctacacacagcgtgaccaccggcgccaagcccatcatcttcaacggcgaagaggtgtgggtgagcaacgccgacgagatcgccgccgtgaacatcggcctgaccatcatccccacaagcaagaaggacgaggagcaccccgacagagagaacgacgacaaggccatcagaaagagcgtcagacggcctagaaagagcggcgagagaagaagcggcgacaagatgcccgccaccgctagaaagaccacaggcggcggccccggcggcggcgccgccgccggcagcggcagccctaagaaaaaacgaaaagttggcagcggaagcaaaaggccggcggccacgaaaaaggccggccaggcaaaaaagaaaaagctcgagtacccatacgatgttccagattacgcttgagaattccccttgagcatctgacttctggctaataaaggaaatttattttcattgcaatagtgtgttggaattttttgtgtctctcaggtaccaaaaacggctcggagatcatcattgcggcgtcaatgggagacgcattacggtgtttcgtcctttccacaagatatataaagccaagaaatcgaaatactttcaagttacggtaagcatatgatagtccattttaaaacataattttaaaactgcaaactacccaagaaattattactttctacgtcacgtattttgtactaatatctttgtgtttacagtcaaattaattccaattatctctctaacagccttgtatcgtatatgcaaatatgaaggaatcatgggaaataggccctctagagggcccgtttaaacccgctgatcagcctcgactgtgccttctagttgccagccatctgttgtttgcccctcccccgtgccttccttgaccctggaaggtgccactcccactgtcctttcctaataaaatgaggaaattgcatcgcattgtctgagtaggtgtcattctattctggggggtggggtggggcaggacagcaagggggaggattgggaagacaatagcaggcatgctggggatgcggtgggctctatggcttctgaggcggaaagaaccagctggggctctagggggtatccccacgcgccctgtagcggcgcattaagcgcggcgggtgtggtggttacgcgcagcgtgaccgctacacttgccagcgccctagcgcccgctcctttcgctttcttcccttcctttctcgccacgttcgccggctttccccgtcaagctctaaatcgggggctccctttagggttccgatttagtgctttacggcacctcgaccccaaaaaacttgattagggtgatggttcacgtagtgggccatcgccctgatagacggtttttcgccctttgacgttggagtccacgttctttaatagtggactcttgttccaaactggaacaacactcaaccctatctcggtctattcttttgatttataagggattttgccgatttcggcctattggttaaaaaatgagctgatttaacaaaaatttaacgcgaattaattctgtggaatgtgtgtcagttagggtgtggaaagtccccaggctccccagcaggcagaagtatgcaaagcatgcatctcaattagtcagcaaccaggtgtggaaagtccccaggctccccagcaggcagaagtatgcaaagcatgcatctcaattagtcagcaaccatagtcccgcccctaactccgcccatcccgcccctaactccgcccagttccgcccattctccgccccatggctgactaattttttttatttatgcagaggccgaggccgcctctgcctctgagctattccagaagtagtgaggaggcttttttggaggcctaggcttttgcaaaaagctcccgggagcttgtatatccattttcggatctgatcaagagacaggatgaggatcgtttcgcatgattgaacaagatggattgcacgcaggttctccggccgcttgggtggagaggctattcggctatgactgggcacaacagacaatcggctgctctgatgccgccgtgttccggctgtcagcgcaggggcgcccggttctttttgtcaagaccgacctgtccggtgccctgaatgaactgcaggacgaggcagcgcggctatcgtggctggccacgacgggcgttccttgcgcagctgtgctcgacgttgtcactgaagcgggaagggactggctgctattgggcgaagtgccggggcaggatctcctgtcatctcaccttgctcctgccgagaaagtatccatcatggctgatgcaatgcggcggctgcatacgcttgatccggctacctgcccattcgaccaccaagcgaaacatcgcatcgagcgagcacgtactcggatggaagccggtcttgtcgatcaggatgatctggacgaagagcatcaggggctcgcgccagccgaactgttcgccaggctcaaggcgcgcatgcccgacggcgaggatctcgtcgtgacccatggcgatgcctgcttgccgaatatcatggtggaaaatggccgcttttctggattcatcgactgtggccggctgggtgtggcggaccgctatcaggacatagcgttggctacccgtgatattgctgaagagcttggcggcgaatgggctgaccgcttcctcgtgctttacggtatcgccgctcccgattcgcagcgcatcgccttctatcgccttcttgacgagttcttctgagcgggactctggggttcgaaatgaccgaccaagcgacgcccaacctgccatcacgagatttcgattccaccgccgccttctatgaaaggttgggcttcggaatcgttttccgggacgccggctggatgatcctccagcgcggggatctcatgctggagttcttcgcccaccccaacttgtttattgcagcttataatggttacaaataaagcaatagcatcacaaatttcacaaataaagcatttttttcactgcattctagttgtggtttgtccaaactcatcaatgtatcttatcatgtctgtataccgtcgacctctagctagagcttggcgtaatcatggtcatagctgtttcctgtgtgaaattgttatccgctcacaattccacacaacatacgagccggaagcataaagtgtaaagcctggggtgcctaatgagtgagctaactcacattaattgcgttgcgctcactgcccgctttccagtcgggaaacctgtcgtgccagctgcattaatgaatcggccaacgcgcggggagaggcggtttgcgtattgggcgctcttccgcttcctcgctcactgactcgctgcgctcggtcgttcggctgcggcgagcggtatcagctcactcaaaggcggtaatacggttatccacagaatcaggggataacgcaggaaagaacatgtgagcaaaaggccagcaaaaggccaggaaccgtaaaaaggccgcgttgctggcgtttttccataggctccgcccccctgacgagcatcacaaaaatcgacgctcaagtcagaggtggcgaaacccgacaggactataaagataccaggcgtttccccctggaagctccctcgtgcgctctcctgttccgaccctgccgcttaccggatacctgtccgcctttctcccttcgggaagcgtggcgctttctcatagctcacgctgtaggtatctcagttcggtgtaggtcgttcgctccaagctgggctgtgtgcacgaaccccccgttcagcccgaccgctgcgccttatccggtaactatcgtcttgagtccaacccggtaagacacgacttatcgccactggcagcagccactggtaacaggattagcagagcgaggtatgtaggcggtgctacagagttcttgaagtggtggcctaactacggctacactagaagaacagtatttggtatctgcgctctgctgaagccagttaccttcggaaaaagagttggtagctcttgatccggcaaacaaaccaccgctggtagcggtttttttgtttgcaagcagcagattacgcgcagaaaaaaaggatctcaagaagatcctttgatcttttctacggggtctgacgctcagtggaacgaaaactcacgttaagggattttggtcatgagattatcaaaaaggatcttcacctagatccttttaaattaaaaatgaagttttaaatcaatctaaagtatatatgagtaaacttggtctgacagttaccaatgcttaatcagtgaggcacctatctcagcgatctgtctatttcgttcatccatagttgcctgactccccgtcgtgtagataactacgatacgggagggcttaccatctggccccagtgctgcaatgataccgcgagacccacgctcaccggctccagatttatcagcaataaaccagccagccggaagggccgagcgcagaagtggtcctgcaactttatccgcctccatccagtctattaattgttgccgggaagctagagtaagtagttcgccagttaatagtttgcgcaacgttgttgccattgctacaggcatcgtggtgtcacgctcgtcgtttggtatggcttcattcagctccggttcccaacgatcaaggcgagttacatgatcccccatgttgtgcaaaaaagcggttagctccttcggtcctccgatcgttgtcagaagtaagttggccgcagtgttatcactcatggttatggcagcactgcataattctcttactgtcatgccatccgtaagatgcttttctgtgactggtgagtactcaaccaagtcattctgagaatagtgtatgcggcgaccgagttgctcttgcccggcgtcaatacgggataataccgcgccacatagcagaactttaaaagtgctcatcattggaaaacgttcttcggggcgaaaactctcaaggatcttaccgctgttgagatccagttcgatgtaacccactcgtgcacccaactgatcttcagcatcttttactttcaccagcgtttctgggtgagcaaaaacaggaaggcaaaatgccgcaaaaaagggaataagggcgacacggaaatgttgaatactcatactcttcctttttcaatattattgaagcatttatcagggttattgtctcatgagcggatacatatttgaatgtatttagaaaaataaacaaataggggttccgcgcacatttccccgaaaagtgccacctgacgtc

SEQ ID NO: 698 - DNA, 8956 bp, synthetic construct
  source 1..8956: mol_type = other DNA
tggcgaatgggacgcgccctgtagcggcgcattaagcgcggcgggtgtggtggttacgcgcagcgtgaccgctacacttgccagcgccctagcgcccgctcctttcgctttcttcccttcctttctcgccacgttcgccggctttccccgtcaagctctaaatcgggggctccctttagggttccgatttagtgctttacggcacctcgaccccaaaaaacttgattagggtgatggttcacgtagtgggccatcgccctgatagacggtttttcgccctttgacgttggagtccacgttctttaatagtggactcttgttccaaactggaacaacactcaaccctatctcggtctattcttttgatttataagggattttgccgatttcggcctattggttaaaaaatgagctgatttaacaaaaatttaacgcgaattttaacaaaatattaacgtttacaatttcaggtggcacttttcggggaaatgtgcgcggaacccctatttgtttatttttctaaatacattcaaatatgtatccgctcatgaattaattcttagaaaaactcatcgagcatcaaatgaaactgcaatttattcatatcaggattatcaataccatatttttgaaaaagccgtttctgtaatgaaggagaaaactcaccgaggcagttccataggatggcaagatcctggtatcggtctgcgattccgactcgtccaacatcaatacaacctattaatttcccctcgtcaaaaataaggttatcaagtgagaaatcaccatgagtgacgactgaatccggtgagaatggcaaaagtttatgcatttctttccagacttgttcaacaggccagccattacgctcgtcatcaaaatcactcgcatcaaccaaaccgttattcattcgtgattgcgcctgagcgagacgaaatacgcgatcgctgttaaaaggacaattacaaacaggaatcgaatgcaaccggcgcaggaacactgccagcgcatcaacaatattttcacctgaatcaggatattcttctaatacctggaatgctgttttcccggggatcgcagtggtgagtaaccatgcatcatcaggagtacggataaaatgcttgatggtcggaagaggcataaattccgtcagccagtttagtctgaccatctcatctgtaacatcattggcaacgctacctttgccatgtttcagaaacaactctggcgcatcgggcttcccatacaatcgatagattgtcgcacctgattgcccgacattatcgcgagcccatttatacccatataaatcagcatccatgttggaatttaatcgcggcctagagcaagacgtttcccgttgaatatggctcataacaccccttgtattactgtttatgtaagcagacagttttattgttcatgaccaaaatcccttaacgtgagttttcgttccactgagcgtcagaccccgtagaaaagatcaaaggatcttcttgagatcctttttttctgcgcgtaatctgctgcttgcaaacaaaaaaaccaccgctaccagcggtggtttgtttgccggatcaagagctaccaactctttttccgaaggtaactggcttcagcagagcgcagataccaaatactgtccttctagtgtagccgtagttaggccaccacttcaagaactctgtagcaccgcctacatacctcgctctgctaatcctgttaccagtggctgctgccagtggcgataagtcgtgtcttaccgggttggactcaagacgatagttaccggataaggcgcagcggtcgggctgaacggggggttcgtgcacacagcccagcttggagcgaacgacctacaccgaactgagatacctacagcgtgagctatgagaaagcgccacgcttcccgaagggagaaaggcggacaggtatccggtaagcggcagggtcggaacaggagagcgcacgagggagcttccagggggaaacgcctggtatctttatagtcctgtcgggtttcgccacctctgacttgagcgtcgatttttgtgatgctcgtcaggggggcggagcctatggaaaaacgccagcaacgcggcctttttacggttcctggccttttgctggccttttgctcacatgttctttcctgcgttatcccctgattctgtggataaccgtattaccgcctttgagtgagctgataccgctcgccgcagccgaacgaccgagcgcagcgagtcagtgagcgaggaagcggaagagcgcctgatgcggtattttctccttacgcatctgtgcggtatttcacaccgcatatatggtgcactctcagtacaatctgctctgatgccgcatagttaagccagtatacactccgctatcgctacgtgactgggtcatggctgcgccccgacacccgccaacacccgctgacgcgccctgacgggcttgtctgctcccggcatccgcttacagacaagctgtgaccgtctccgggagctgcatgtgtcagaggttttcaccgtcatcaccgaaacgcgcgaggcagctgcggtaaagctcatcagcgtggtcgtgaagcgattcacagatgtctgcctgttcatccgcgtccagctcgttgagtttctccagaagcgttaatgtctggcttctgataaagcgggccatgttaagggcggttttttcctgtttggtcactgatgcctccgtgtaagggggatttctgttcatgggggtaatgataccgatgaaacgagagaggatgctcacgatacgggttactgatgatgaacatgcccggttactggaacgttgtgagggtaaacaactggcggtatggatgcggcgggaccagagaaaaatcactcagggtcaatgccagcgcttcgttaatacagatgtaggtgttccacagggtagccagcagcatcctgcgatgcagatccggaacataatggtgcagggcgctgacttccgcgtttccagactttacgaaacacggaaaccgaagaccattcatgttgttgctcaggtcgcagacgttttgcagcagcagtcgcttcacgttcgctcgcgtatcggtgattcattctgctaaccagtaaggcaaccccgccagcctagccgggtcctcaacgacaggagcacgatcatgcgcacccgtggggccgccatgccggcgataatggcctgcttctcgccgaaacgtttggtggcgggaccagtgacgaaggcttgagcgagggcgtgcaagattccgaataccgcaagcgacaggccgatcatcgtcgcgctccagcgaaagcggtcctcgccgaaaatgacccagagcgctgccggcacctgtcctacgagttgcatgataaagaagacagtcataagtgcggcgacgatagtcatgccccgcgcccaccggaaggagctgactgggttgaaggctctcaagggcatcggtcgagatcccggtgcctaatgagtgagctaacttacattaattgcgttgcgctcactgcccgctttccagtcgggaaacctgtcgtgccagctgcattaatgaatcggccaacgcgcggggagaggcggtttgcgtattgggcgccagggtggtttttcttttcaccagtgagacgggcaacagctgattgcccttcaccgcctggccctgagagagttgcagcaagcggtccacgctggtttgccccagcaggcgaaaatcctgtttgatggtggttaacggcgggatataacatgagctgtcttcggtatcgtcgtatcccactaccgagatatccgcaccaacgcgcagcccggactcggtaatggcgcgcattgcgcccagcgccatctgatcgttggcaaccagcatcgcagtgggaacgatgccctcattcagcatttgcatggtttgttgaaaaccggacatggcactccagtcgccttcccgttccgctatcggctgaatttgattgcgagtgagatatttatgccagccagccagacgcagacgcgccgagacagaacttaatgggcccgctaacagcgcgatttgctggtgacccaatgcgaccagatgctccacgcccagtcgcgtaccgtcttcatgggagaaaataatactgttgatgggtgtctggtcagagacatcaagaaataacgccggaacattagtgcaggcagcttccacagcaatggcatcctggtcatccagcggatagttaatgatcagcccactgacgcgttgcgcgagaagattgtgcaccgccgctttacaggcttcgacgccgcttcgttctaccatcgacaccaccacgctggcacccagttgatcggcgcgagatttaatcgccgcgacaatttgcgacggcgcgtgcagggccagactggaggtggcaacgccaatcagcaacgactgtttgcccgccagttgttgtgccacgcggttgggaatgtaattcagctccgccatcgccgcttccactttttcccgcgttttcgcagaaacgtggctggcctggttcaccacgcgggaaacggtctgataagagacaccggcatactctgcgacatcgtataacgttactggtttcacattcaccaccctgaattgactctcttccgggcgctatcatgccataccgcgaaaggttttgcgccattcgatggtgtccgggatctcgacgctctcccttatgcgactcctgcattaggaagcagcccagtagtaggttgaggccgttgagcaccgccgccgcaaggaatggtgcatgcaaggagatggcgcccaacagtcccccggccacggggcctgccaccatacccacgccgaaacaagcgctcatgagcccgaagtggcgagcccgatcttccccatcggtgatgtcggcgatataggcgccagcaaccgcacctgtggcgccggtgatgccggccacgatgcgtccggcgtagaggatcgagatctcgatcccgcgaaattaatacgactcactataggggaattgtgagcggataacaattcccctctagaaataattttgtttaactttaagaaggagatataccatgggcagcagccatcatcatcatcatcacagcagcggcctggtgccgcgcggcagccatatggctagcatgactggtggacagcaaatgggtcgcggatccatgccggcagctaagaaaaagaaactggatggcagcgtcgacatcttcgtggtgctgagcgtgaatcagttcagatgcaaccccaacgccttcagacaagcctccatgaaaaccgacgacgagaagaaggacaccgccatcaagagctacacaagctggctgctgcccaacgacagaaaggagaaggacatggtgcggagcttcctggccctggaccaaggcagcagattctttttcgacctgatgcaagcctggtacggcggcctcacccccgacatcatcaagagcgtgaccaaggagcgggacctggtggacctgtggtgcgccatctactggttcagacccatgaagaaggagctggcctcccaccccatcgacagagtggacctggccaagacctttcagagatactacggcggccccgcctccgacgtggtgcaagagtacctgagcgcctccatcggcgaggactgctgctggaacgactgcagacagaagtaccaagagttctgcaagaacctcggggtggacttcacccccgacctcaagaccctggtgagagagaagctgatcgccgtggccctgaacgacggcagccaagccgccatcagcaacctgttcggcaacggcggcaaggaggacagaaacgtgaaggtgaacatctgcaagaagatcctgattgctctggagaaggccggcaaatccgtgaagtacgtgcgggacgtgcagagcatcatcctgaagtgcgccaacgccaaggacagagaggacttcaacagaatctacgccgacaagaacggcagacccggcaccctgctcctgctcctggacagaaagggcgagaacacctacgacgccgaggtgctgaagagatacctgagaaagaccatcaagagcaagaacgcccccctggtgtggaactacaatcagaagctgttcgagtacatcgagagaggcatccggaatctgctgagaagaaccatcaactacgacgcctgggcctggggcgagatgtggagagtgggccacacccccctgcagaccaaggccacaagaaactaccacttcgcccaagagcagctgaagagacacagcgacatcgccgccgcttcccaaagcagccacgccatcgccgtcgctctgaacgagttcttcgagagccccttcttcgacggcgagaaccccttcaccatctgcccccaccacctgggcaagaacctggaaaagctgttcaaggcctgggccgacgaaaaaaatcagaccgacgaggaggacgccggcgaaaccgccatcaccgactactgcgccgagttcaaggacggcttcgacagagagcccattagaaacctgctgagatacgtgtacgcttccctgagaagcaagtacagcgccaaggagctgatccaagccgccaagtacaatcagcagttcgagagatatcagagacagaaggcccaccccgtgacccccgacaaccaaggctacacctggcccgaggccgtgatcaagcctagcaaggccgagagaaagaacagagagaacagcctggacacaagaatctgggtgagcgtgaagctgctgcaaaaggacggcacctgggagaagcaccacatccccttctacaacctgagattcttcgaagaggtgtacgccgctgcctccatcgccgaggacatgcctagccccaccttcagaaacagcagattcggcttcaagctgcccaagctgctgaacacccacgccaagatcaacaagaaaaagaaggacggcaagaaggacaagaaggccgtgaacgccgccaagagagaggctagaatctacctcgctgccaaggagggcagactgcccgccccctccgtgcccctggacaagctgagcgccgtgatcgctagagtgaacggcaagttccaagtgaccgtgcccgtgaagttcaaggtgaacaagcagcccaagtaccccctgcctcagctggggcagatcatcctgggctacgatcagaacctgaccgccaaccacgcctgggccctgttcgaggtggtgaccgaggacacccccggcgcccacttctgcagaaatcagtacctgagagtgctcaagaccggccaagtgagaagcatcaccaagaccaaggacggccaagagatcgatcagctgagctacgacggcctggagtacaaggagtacggcgagtggagaaagcaagccaagaagttcgcctcccaatggtacatcaccaccaaggtgagaaagggcaaggaaaccaccctgctgagccaacccgccctggagagattcgagagcatcgagaagtacaagcccgccctgtacagattcaacaaggaatacgcccggctgctcctggccgtcatcagaagaaagaccctgaacgagctggaggagatcagacccgagatcttcagactggtggagcaaggcttcggcatctgcagattcggcagcctgagcctgagcagcttcgaggccatcagagccgccaaggccgtgatctacggctacttcagcaccgccctgaagcacgaccacaacacccccatcacagatgacgagagacaagccttcgaccccgagctgttcggcctgctgaacaagctggaaaccctgagacagaacaagggcgaggagaagatcaacagagccgctaacgccctgatcagaatcgccctggagaacaaggccgacttcatcagaggcgagggcgacctgcccaccaccaacaagagcgtcaagaaggggcagaacagcagaagcatggactggctggctagaggcctgttcaacaagatctgtcagctggccgtgatgcacaacatcattcccaccgccgccaacccccacagcacaagccaccaagaccccttcgagcacaacaaggacttcgacgaccctcagcccgccatgaagtgcagatacgctgagttcaagatcgaggacatcggcgacagcgtgctggagagactgggcacctccctgagaaatgccaaggccgggcagaccggcgcctactattacaagggcgcccaagacttcctggcccactacggcctgcaagacatcgaggaagagctgaagaagtgcagaagaggcagaaaggccaacatgccctgctgggagctgcagaagagactgattcagaagctgggcagcaaggacgccgtggtgtacatccccatgagaggcggccggatctacctggctacacacagcgtgaccaccggcgccaagcccatcatcttcaacggcgaagaggtgtgggtgagcaacgccgacgagatcgccgccgtgaacatcggcctgaccatcatccccacaagcaagaaggacgaggagcaccccgacagagagaacgacgacaaggccatcagaaagagcgtcagacggcctagaaagagcggcgagagaagaagcggcgacaagatgcccgccaccgctagaaagaccacaggcggcggccccggcggcggcgccgccgccggcagcggcagccctaagaaaaaacgaaaagttggcagcggaagcaaaaggccggcggccacgaaaaaggccggccaggcaaaaaagaaaaagctcgagtacccatacgatgttccagattacgcttgactcgagcaccaccaccaccaccactgagatccggctgctaacaaagcccgaaaggaagctgagttggctgctgccaccgctgagcaataactagcataaccccttggggcctctaaacgggtcttgaggggttttttgctgaaaggaggaactatatccggat

SEQ ID NO: 699 - DNA, 51 bp, synthetic construct
  source 1..51: mol_type = other DNA
tggacagcaaatgggtcgcggatccatgccggcagctaagaaaaagaaact

SEQ ID NO: 700 - DNA, 55 bp, synthetic construct
  source 1..55: mol_type = other DNA
tctcagtggtggtggtggtggtgctcgagtcaagcgtaatctggaacatcgtatg

SEQ ID NO: 701 - DNA, 273 bp, synthetic construct
  source 1..273: mol_type = other DNA
ggagttcagacgtgtgctcttccgatctcagcacaaaaggaaactcaccctaactgtaaagtaattgtgtgttttgagactataaatatgcatgcgagaaaagccttgtttgccaccatggaacggctcggagatcatcattgcgnnnnnnngtgagcaagggcgaggagctgttcaccggggtggtgcccatcctggtcgagctggacggcgacgtaaacggccacaagttcagcgtgtccggcagatcggaagagcacacgtctgaactcc

SEQ ID NO: 702 - RNA, 46 nt, synthetic construct
  source 1..46: mol_type = other RNA
gtaatgcgtctcccattgacgcgtgagcaagggcgaggagctgttc

SEQ ID NO: 703 - RNA, 48 nt, synthetic construct
  source 1..48: mol_type = other RNA
gtaatgcgtctcccattgacgccgcaatgatgatctccgagccgttcc

SEQ ID NO: 704 - RNA, 22 nt, synthetic construct
  source 1..22: mol_type = other RNA
gtaatgcgtctcccattgacgc

SEQ ID NO: 705 - DNA, 59 bp, synthetic construct
  source 1..59: mol_type = other DNA
gttgacatgctggattgagacttcctacactctttccctacacgacgctcttccgatct

SEQ ID NO: 706 - DNA, 58 bp, synthetic construct
  source 1..58: mol_type = other DNA
gatcggaagagcgtcgtgtagggaaagagtgtaggaagtctcaatccagcatgtcaac

SEQ ID NO: 707 - DNA, 19 bp, synthetic construct
  source 1..19: mol_type = other DNA
ggagttcagacgtgtgctc

SEQ ID NO: 708 - DNA, 24 bp, synthetic construct
  source 1..24: mol_type = other DNA
gttgacatgctggattgagacttc

SEQ ID NO: 709 - DNA, 58 bp, synthetic construct
  source 1..58: mol_type = other DNA
aatgatacggcgaccaccgagatctacactatagcctacactctttccctacacgacg

SEQ ID NO: 710 - DNA, 57 bp, synthetic construct
  source 1..57: mol_type = other DNA
caagcagaagacggcatacgagatcgagtaatgtgactggagttcagacgtgtgctc

SEQ ID NO: 711 - DNA, 8057 bp, synthetic construct
  source 1..8057: mol_type = other DNA
tgtagtcttatgcaatactcttgtagtcttgcaacatggtaacgatgagttagcaacatgccttacaaggagagaaaaagcaccgtgcatgccgattggtggaagtaaggtggtacgatcgtgccttattaggaaggcaacagacgggtctgacatggattggacgaaccactgaattgccgcattgcagagatattgtatttaagtgcctagctcgatacataaacgggtctctctggttagaccagatctgagcctgggagctctctggctaactagggaacccactgcttaagcctcaataaagcttgccttgagtgcttcaagtagtgtgtgcccgtctgttgtgtgactctggtaactagagatccctcagacccttttagtcagtgtggaaaatctctagcagtggcgcccgaacagggacttgaaagcgaaagggaaaccagaggagctctctcgacgcaggactcggcttgctgaagcgcgcacggcaagaggcgaggggcggcgactggtgagtacgccaaaaattttgactagcggaggctagaaggagagagatgggtgcgagagcgtcagtattaagcgggggagaattagatcgcgatgggaaaaaattcggttaaggccagggggaaagaaaaaatataaattaaaacatatagtatgggcaagcagggagctagaacgattcgcagttaatcctggcctgttagaaacatcagaaggctgtagacaaatactgggacagctacaaccatcccttcagacaggatcagaagaacttagatcattatataatacagtagcaaccctctattgtgtgcatcaaaggatagagataaaagacaccaaggaagctttagacaagatagaggaagagcaaaacaaaagtaagaccaccgcacagcaagcggccactgatcttcagacctggaggaggagatatgagggacaattggagaagtgaattatataaatataaagtagtaaaaattgaaccattaggagtagcacccaccaaggcaaagagaagagtggtgcagagagaaaaaagagcagtgggaataggagctttgttccttgggttcttgggagcagcaggaagcactatgggcgcagcgtcaatgacgctgacggtacaggccagacaattattgtctggtatagtgcagcagcagaacaatttgctgagggctattgaggcgcaacagcatctgttgcaactcacagtctggggcatcaagcagctccaggcaagaatcctggctgtggaaagatacctaaaggatcaacagctcctggggatttggggttgctctggaaaactcatttgcaccactgctgtgccttggaatgctagttggagtaataaatctctggaacagatttggaatcacacgacctggatggagtgggacagagaaattaacaattacacaagcttaatacactccttaattgaagaatcgcaaaaccagcaagaaaagaatgaacaagaattattggaattagataaatgggcaagtttgtggaattggtttaacataacaaattggctgtggtatataaaattattcataatgatagtaggaggcttggtaggtttaagaatagtttttgctgtactttctatagtgaatagagttaggcagggatattcaccattatcgtttcagacccacctcccaaccccgaggggacccgacaggcccgaaggaatagaagaagaaggtggagagagagacagagacagatccattcgattagtgaacggatctcgacggtatcggttaacttttaaaagaaaaggggggattggggggtacagtgcaggggaaagaatagtagacataatagcaacagacatacaaactaaagaattacaaaaacaaattacaaaattcaaaattttatcgatactagtattatgcccagtacatgaccttatgggactttcctacttggcagtacatctacgtattagtcatcgctattaccatggtgatgcggttttggcagtacatcaatgggcgtggatagcggtttgactcacggggatttccaagtctccaccccattgacgtcaatgggagtttgttttggcaccaaaatcaacgggactttccaaaatgtcgtaacaactccgccccattgacgcaaatgggcggtaggcgtgtacggtgggaggtttatataagcagagctcgtttagtgaaccgtcagatcgcctggagacgccatccacgctgttttgacctccatagaagattctagagctagcgaattgggatccctagagatccgacgccgccatctctaggcccgcgccggccccctcgcacagacttgtgggagaagctcggctactcccctgccccggttaatttgcatataatatttcctagtaactatagaggcttaatgtgcgataaaagacagataatctgttctttttaatactagctacattttacatgataggcttggatttctataagagatacaaatactaaattattattttaaaaaacagcacaaaaggaaactcaccctaactgtaaagtaattgtgtgttttgagactataaatatgcatgcgagaaaagccttgtttgccaccatggaacggctcggagatatccagcgtacggctctcatcaactccactggggaagaagtggccatgcgcaagctggtgcgctcagtgactgtggttgaggacgacgaggatgaggatggagatgacctgctccatcaccaccacggctcccactgcagcagctcgggggaccccgctgagtacaacctgcgctcgcgcaccgtgctgtgcgggacctgcgggcagcctgccgacaaggcatctgccagcggctcaggagcccaggtgggcggacccatctcctctggctcttctgcctccagtgtcacggtcactcgcagctaccgcagtgtggggggcagtgggggtggcagcttcggggacaatctggtcacccgctcctacctcctgggcaactccagcccccgaacccagagcccccagaactgcagcatcatgtaatctgtctagaagaattcctcgaggcggccgctaaatagttgaatttaaatagatctccagcacagtggtaaatagttgattcgaacaaggatctgcgatcgctccggtgcccgtcagtgggcagagcgcacatcgcccacagtccccgagaagttggggggaggggtcggcaattgaacgggtgcctagagaaggtggcgcggggtaaactgggaaagtgatgtcgtgtactggctccgcctttttcccgagggtgggggagaaccgtatataagtgcagtagtcgccgtgaacgttctttttcgcaacgggtttgccgccagaacacagctgaagcttcgaggggctcgcatctctccttcacgcgcccgccgccctacctgaggccgccatccacgccggttgagtcgcgttctgccgcctcccgcctgtggtgcctcctgaactgcgtccgccgtctaggtaagtttaaagctcaggtcgagaccgggcctttgtccggcgctcccttggagcctacctagactcagccggctctccacgctttgcctgaccctgcttgctcaactctacgtctttgtttcgttttctgttctgcgccgttacagatccaagctgtgaccggcgcctacgcccatgggcatggccaagcctttgtctcaagaagaatccaccctcattgaaagagcaacggctacaatcaacagcatccccatctctgaagactacagcgtcgccagcgcagctctctctagcgacggccgcatcttcactggtgtcaatgtatatcattttactgggggaccttgtgcagaactcgtggtgctgggcactgctgctgctgcggcagctggcaacctgacttgtatcgtcgcgatcggaaatgagaacaggggcatcttgagcccctgcggacggtgccgacaggtgcttctcgatctgcatcctgggatcaaagccatagtgaaggacagtgatggacagccgacggcagttgggattcgtgaattgctgccctctggttatgtgtgggagggctaagcacaattcgagctcgcgtcgacaatcaacctctggattacaaaatttgtgaaagattgactggtattcttaactatgttgctccttttacgctatgtggatacgctgctttaatgcctttgtatcatgctattgcttcccgtatggctttcattttctcctccttgtataaatcctggttgctgtctctttatgaggagttgtggcccgttgtcaggcaacgtggcgtggtgtgcactgtgtttgctgacgcaacccccactggttggggcattgccaccacctgtcagctcctttccgggactttcgctttccccctccctattgccacggcggaactcatcgccgcctgccttgcccgctgctggacaggggctcggctgttgggcactgacaattccgtggtgttgtcggggaaatcatcgtcctttccttggctgctcgcctgtgttgccacctggattctgcgcgggacgtccttctgctacgtcccttcggccctcaatccagcggaccttccttcccgcggcctgctgccggctctgcggcctcttccgcgtcttcgccttcgccctcagacgagtcggatctccctttgggccgcctccccgcctggtacctttaagaccaatgacttacaaggcagctgtagatcttagccactttttaaaagaaaaggggggactggaagggctaattcactcccaacgaagataagatctgctttttgcttgtactgggtctctctggttagaccagatctgagcctgggagctctctggctaactagggaacccactgcttaagcctcaataaagcttgccttgagtgcttcaagtagtgtgtgcccgtctgttgtgtgactctggtaactagagatccctcagacccttttagtcagtgtggaaaatctctagcagtagtagttcatgtcatcttattattcagtatttataacttgcaaagaaatgaatatcagagagtgagaggaacttgtttattgcagcttataatggttacaaataaagcaatagcatcacaaatttcacaaataaagcatttttttcactgcattctagttgtggtttgtccaaactcatcaatgtatcttatcatgtctggctctagctatcccgcccctaactccgcccatcccgcccctaactccgcccagttccgcccattctccgccccatggctgactaattttttttatttatgcagaggccgaggccgcctcggcctctgagctattccagaagtagtgaggaggcttttttggaggcctagacttttgcagagaccaaattcgtaatcatgtcatagctgtttcctgtgtgaaattgttatccgctcacaattccacacaacatacgagccggaagcataaagtgtaaagcctggggtgcctaatgagtgagctaactcacattaattgcgttgcgctcactgcccgctttccagtcgggaaacctgtcgtgccagctgcattaatgaatcggccaacgcgcggggagaggcggtttgcgtattgggcgctcttccgcttcctcgctcactgactcgctgcgctcggtcgttcggctgcggcgagcggtatcagctcactcaaaggcggtaatacggttatccacagaatcaggggataacgcaggaaagaacatgtgagcaaaaggccagcaaaaggccaggaaccgtaaaaaggccgcgttgctggcgtttttccataggctccgcccccctgacgagcatcacaaaaatcgacgctcaagtcagaggtggcgaaacccgacaggactataaagataccaggcgtttccccctggaagctccctcgtgcgctctcctgttccgaccctgccgcttaccggatacctgtccgcctttctcccttcgggaagcgtggcgctttctcatagctcacgctgtaggtatctcagttcggtgtaggtcgttcgctccaagctgggctgtgtgcacgaaccccccgttcagcccgaccgctgcgccttatccggtaactatcgtcttgagtccaacccggtaagacacgacttatcgccactggcagcagccactggtaacaggattagcagagcgaggtatgtaggcggtgctacagagttcttgaagtggtggcctaactacggctacactagaagaacagtatttggtatctgcgctctgctgaagccagttaccttcggaaaaagagttggtagctcttgatccggcaaacaaaccaccgctggtagcggtggtttttttgtttgcaagcagcagattacgcgcagaaaaaaaggatctcaagaagatcctttgatcttttctacggggtctgacgctcagtggaacgaaaactcacgttaagggattttggtcatgagattatcaaaaaggatcttcacctagatccttttaaattaaaaatgaagttttaaatcaatctaaagtatatatgagtaaacttggtctgacagttaccaatgcttaatcagtgaggcacctatctcagcgatctgtctatttcgttcatccatagttgcctgactccccgtcgtgtagataactacgatacgggagggcttaccatctggccccagtgctgcaatgataccgcgagacccacgctcaccggctccagatttatcagcaataaaccagccagccggaagggccgagcgcagaagtggtcctgcaactttatccgcctccatccagtctattaattgttgccgggaagctagagtaagtagttcgccagttaatagtttgcgcaacgttgttgccattgctacaggcatcgtggtgtcacgctcgtcgtttggtatggcttcattcagctccggttcccaacgatcaaggcgagttacatgatcccccatgttgtgcaaaaaagcggttagctccttcggtcctccgatcgttgtcagaagtaagttggccgcagtgttatcactcatggttatggcagcactgcataattctcttactgtcatgccatccgtaagatgcttttctgtgactggtgagtactcaaccaagtcattctgagaatagtgtatgcggcgaccgagttgctcttgcccggcgtcaatacgggataataccgcgccacatagcagaactttaaaagtgctcatcattggaaaacgttcttcggggcgaaaactctcaaggatcttaccgctgttgagatccagttcgatgtaacccactcgtgcacccaactgatcttcagcatcttttactttcaccagcgtttctgggtgagcaaaaacaggaaggcaaaatgccgcaaaaaagggaataagggcgacacggaaatgttgaatactcatactcttcctttttcaatattattgaagcatttatcagggttattgtctcatgagcggatacatatttgaatgtatttagaaaaataaacaaataggggttccgcgcacatttccccgaaaagtgccacctgacgtctaagaaaccattattatcatgacattaacctataaaaataggcgtatcacgaggccctttcgtctcgcgcgtttcggtgatgacggtgaaaacctctgacacatgcagctcccggagacggtcacagcttgtctgtaagcggatgccgggagcagacaagcccgtcagggcgcgtcagcgggtgttggcgggtgtcggggctggcttaactatgcggcatcagagcagattgtactgagagtgcaccatatgcggtgtgaaataccgcacagatgcgtaaggagaaaataccgcatcaggcgccattcgccattcaggctgcgcaactgttgggaagggcgatcggtgcgggcctcttcgctattacgccagctggcgaaagggggatgtgctgcaaggcgattaagttgggtaacgccagggttttcccagtcacgacgttgtaaaacgacggccagtgccaagctgacgcg

SEQ ID NO: 712 - DNA, 8131 bp, synthetic construct
  source 1..8131: mol_type = other DNA
acgcgtgtagtcttatgcaatactcttgtagtcttgcaacatggtaacgatgagttagcaacatgccttacaaggagagaaaaagcaccgtgcatgccgattggtggaagtaaggtggtacgatcgtgccttattaggaaggcaacagacgggtctgacatggattggacgaaccactgaattgccgcattgcagagatattgtatttaagtgcctagctcgatacaataaacgggtctctctggttagaccagatctgagcctgggagctctctggctaactagggaacccactgcttaagcctcaataaagcttgccttgagtgcttcaagtagtgtgtgcccgtctgttgtgtgactctggtaactagagatccctcagacccttttagtcagtgtggaaaatctctagcagtggcgcccgaacagggacctgaaagcgaaagggaaaccagagctctctcgacgcaggactcggcttgctgaagcgcgcacggcaagaggcgaggggcggcgactggtgagtacgccaaaaattttgactagcggaggctagaaggagagagatgggtgcgagagcgtcagtattaagcgggggagaattagatcgcgatgggaaaaaattcggttaaggccagggggaaagaaaaaatataaattaaaacatatagtatgggcaagcagggagctagaacgattcgcagttaatcctggcctgttagaaacatcagaaggctgtagacaaatactgggacagctacaaccatcccttcagacaggatcagaagaacttagatcattatataatacagtagcaaccctctattgtgtgcatcaaaggatagagataaaagacaccaaggaagctttagacaagatagaggaagagcaaaacaaaagtaagaccaccgcacagcaagcggccactgatcttcagacctggaggaggagatatgagggacaattggagaagtgaattatataaatataaagtagtaaaaattgaaccattaggagtagcacccaccaaggcaaagagaagagtggtgcagagagaaaaaagagcagtgggaataggagctttgttccttgggttcttgggagcagcaggaagcactatgggcgcagcctcaatgacgctgacggtacaggccagacaattattgtctggtatagtgcagcagcagaacaatttgctgagggctattgaggcgcaacagcatctgttgcaactcacagtctggggcatcaagcagctccaggcaagaatcctggctgtggaaagatacctaaaggatcaacagctcctggggatttggggttgctctggaaaactcatttgcaccactgctgtgccttggaatgctagttggagtaataaatctctggaacagattggaatcacacgacctggatggagtgggacagagaaattaacaattacacaagcttaatacactccttaattgaagaatcgcaaaaccagcaagaaaagaatgaacaagaattattggaattagataaatgggcaagtttgtggaattggtttaacataacaaattggctgtggtatataaaattattcataatgatagtaggaggcttggtaggtttaagaatagtttttgctgtactttctatagtgaatagagttaggcagggatattcaccattatcgtttcagacccacctcccaaccccgaggggacccgacaggcccgaaggaatagaagaagaaggtggagagagagacagagacagatccattcgattagtgaacggatctcgacggtatcggttaacttttaaaagaaaaggggggattggggggtacagtgcaggggaaagaatagtagacataatagcaacagacatacaaactaaagaattacaaaaacaaattacaaaattcaaaattttatcgatactagtattatgcccagtacatgaccttatgggactttcctacttggcagtacatctacgtattagtcatcgctattaccatggtgatgcggttttggcagtacatcaatgggcgtggatagcggtttgactcacggggatttccaagtctccaccccattgacgtcaatgggagtttgttttggcaccaaaatcaacgggactttccaaaatgtcgtaacaactccgccccattgacgcaaatgggcggtaggcgtgtacggtgggaggtttatataagcagagctcgtttagtgaaccgtcagatcgcctggagacgccatccacgctgttttgacctccatagaagattctagagcgagaaaagccttgtttgccaccatggaacggctcggagatcatcattgcgtcgcgaggtgagcaagggcgaggagctgttcaccggggtggtgcccatcctggtcgagctggacggcgacgtaaacggccacaagttcagcgtgtccggcgagggcgagggcgatgccacctacggcaagctgaccctgaagttcatctgcaccaccggcaagctgcccgtgccctggcccaccctcgtgaccaccctgacctacggcgtgcagtgcttcagccgctaccccgaccacatgaagcagcacgacttcttcaagtccgccatgcccgaaggctacgtccaggagcgcaccatcttcttcaaggacgacggcaactacaagacccgcgccgaggtgaagttcgagggcgacaccctggtgaaccgcatcgagctgaagggcatcgacttcaaggaggacggcaacatcctggggcacaagctggagtacaactacaacagccacaacgtctatatcatggccgacaagcagaagaacggcatcaaggtgaacttcaagatccgccacaacatcgaggacggcagcgtgcagctcgccgaccactaccagcagaacacccccatcggcgacggccccgtgctgctgcccgacaaccactacctgagcacccagtccaagctgagcaaagaccccaacgagaagcgcgatcacatggtcctgctggagttcgtgaccgccgccgggatcactctcggcatggacgagctgtacaagtaagcggccgcgaaggatctgcgatcgctccggtgcccgtcagtgggcagagcgcacatcgcccacagtccccgagaagttggggggaggggtcggcaattgaacgggtgcctagagaaggtggcgcggggtaaactgggaaagtgatgtcgtgtactggctccgcctttttcccgagggtgggggagaaccgtatataagtgcagtagtcgccgtgaacgttctttttcgcaacgggtttgccgccagaacacagctgaagcttcgaggggctcgcatctctccttcacgcgcccgccgccctacctgaggccgccatccacgccggttgagtcgcgttctgccgcctcccgcctgtggtgcctcctgaactgcgtccgccgtctaggtaagtttaaagctcaggtcgagaccgggcctttgtccggcgctcccttggagcctacctagactcagccggctctccacgctttgcctgaccctgcttgctcaactctacgtctttgtttcgttttctgttctgcgccgttacagatccaagctgtgaccggcgcctacgctagatgaccgagtacaagcccacggtgcgcctcgccacccgcgacgacgtccccagggccgtacgcaccctcgccgccgcgttcgccgactaccccgccacgcgccacaccgtcgatccggaccgccacatcgagcgggtcaccgagctgcaagaactcttcctcacgcgcgtcgggctcgacatcggcaaggtgtgggtcgcggacgacggcgccgcggtggcggtctggaccacgccggagagcgtcgaagcgggggcggtgttcgccgagatcggcccgcgcatggccgagttgagcggttcccggctggccgcgcagcaacagatggaaggcctcctggcgccgcaccggcccaaggagcccgcgtggttcctggccaccgtcggcgtctcgcccgaccaccagggcaagggtctgggcagcgccgtcgtgctccccggagtggaggcggccgagcgcgccggggtgcccgccttcctggagacctccgcgccccgcaacctccccttctacgagcggctcggcttcaccgtcaccgccgacgtcgaggtgcccgaaggaccgcgcacctggtgcatgacccgcaagcccggtgcctgagtcgacaatcaacctctggattacaaaatttgtgaaagattgactggtattcttaactatgttgctccttttacgctatgtggatacgctgctttaatgcctttgtatcatgctattgcttcccgtatggctttcattttctcctccttgtataaatcctggttgctgtctctttatgaggagttgtggcccgttgtcaggcaacgtggcgtggtgtgcactgtgtttgctgacgcaacccccactggttggggcattgccaccacctgtcagctcctttccgggactttcgctttccccctccctattgccacggcggaactcatcgccgcctgccttgcccgctgctggacaggggctcggctgttgggcactgacaattccgtggtgttgtcggggaaatcatcgtcctttccttggctgctcgcctgtgttgccacctggattctgcgcgggacgtccttctgctacgtcccttcggccctcaatccagcggaccttccttcccgcggcctgctgccggctctgcggcctcttccgcgtcttcgccttcgccctcagacgagtcggatctccctttgggccgcctccccgcctggtacctttaagaccaatgacttacaaggcagctgtagatcttagccactttttaaaagaaaaggggggactggaagggctaattcactcccaacgaaaataagatctgctttttgcttgtactgggtctctctggttagaccagatctgagcctgggagctctctggctaactagggaacccactgcttaagcctcaataaagcttgccttgagtgcttcaagtagtgtgtgcccgtctgttgtgtgactctggtaactagagatccctcagacccttttagtcagtgtggaaaatctctagcagtagtagttcatgtcatcttattattcagtatttataacttgcaaagaaatgaatatcagagagtgagaggaacttgtttattgcagcttataatggttacaaataaagcaatagcatcacaaatttcacaaataaagcatttttttcactgcattctagttgtggtttgtccaaactcatcaatgtatcttatcatgtctggctctagctatcccgcccctaactccgcccagttccgcccattctccgccccatggctgactaattttttttatttatgcagaggccgaggccgcctcggcctctgagctattccagaagtagtgaggaggcttttttggaggcctagacttttgcagagacggcccaaattcgtaatcatggtcatagctgtttcctgtgtgaaattgttatccgctcacaattccacacaacatacgagccggaagcataaagtgtaaagcctggggtgcctaatgagtgagctaactcacattaattgcgttgcgctcactgcccgctttccagtcgggaaacctgtcgtgccagctgcattaatgaatcggccaacgcgcggggagaggcggtttgcgtattgggcgctcttccgcttcctcgctcactgactcgctgcgctcggtcgttcggctgcggcgagcggtatcagctcactcaaaggcggtaatacggttatccacagaatcaggggataacgcaggaaagaacatgtgagcaaaaggccagcaaaaggccaggaaccgtaaaaaggccgcgttgctggcgtttttccataggctccgcccccctgacgagcatcacaaaaatcgacgctcaagtcagaggtggcgaaacccgacaggactataaagataccaggcgtttccccctggaagctccctcgtgcgctctcctgttccgaccctgccgcttaccggatacctgtccgcctttctcccttcgggaagcgtggcgctttctcatagctcacgctgtaggtatctcagttcggtgtaggtcgttcgctccaagctgggctgtgtgcacgaaccccccgttcagcccgaccgctgcgccttatccggtaactatcgtcttgagtccaacccggtaagacacgacttatcgccactggcagcagccactggtaacaggattagcagagcgaggtatgtaggcggtgctacagagttcttgaagtggtggcctaactacggctacactagaaggacagtatttggtatctgcgctctgctgaagccagttaccttcggaaaaagagttggtagctcttgatccggcaaacaaaccaccgctggtagcggtggtttttttgtttgcaagcagcagattacgcgcagaaaaaaaggatctcaagaagatcctttgatcttttctacggggtctgacgctcagtggaacgaaaactcacgttaagggattttggtcatgagattatcaaaaaggatcttcacctagatccttttaaattaaaaatgaagttttaaatcaatctaaagtatatatgagtaaacttggtctgacagttaccaatgcttaatcagtgaggcacctatctcagcgatctgtctatttcgttcatccatagttgcctgactccccgtcgtgtagataactacgatacgggagggcttaccatctggccccagtgctgcaatgataccgcgagacccacgctcaccggctccagatttatcagcaataaaccagccagccggaagggccgagcgcagaagtggtcctgcaactttatccgcctccatccagtctattaattgttgccgggaagctagagtaagtagttcgccagttaatagtttgcgcaacgttgttgccattgctacaggcatcgtggtgtcacgctcgtcgtttggtatggcttcattcagctccggttcccaacgatcaaggcgagttacatgatcccccatgttgtgcaaaaaagcggttagctccttcggtcctccgatcgttgtcagaagtaagttggccgcagtgttatcactcatggttatggcagcactgcataattctcttactgtcatgccatccgtaagatgcttttctgtgactggtgagtactcaaccaagtcattctgagaatagtgtatgcggcgaccgagttgctcttgcccggcgtcaatacgggataataccgcgccacatagcagaactttaaaagtgctcatcattggaaaacgttcttcggggcgaaaactctcaaggatcttaccgctgttgagatccagttcgatgtaacccactcgtgcacccaactgatcttcagcatcttttactttcaccagcgtttctgggtgagcaaaaacaggaaggcaaaatgccgcaaaaaagggaataagggcgacacggaaatgttgaatactcatactcttcctttttcaatattattgaagcatttatcagggttattgtctcatgagcggatacatatttgaatgtatttagaaaaataaacaaataggggttccgcgcacatttccccgaaaagtgccacctgacgtctaagaaaccattattatcatgacattaacctataaaaataggcgtatcacgaggccctttcgtctcgcgcgtttcggtgatgacggtgaaaacctctgacacatgcagctcccggagacggtcacagcttgtctgtaagcggatgccgggagcagacaagcccgtcagggcgcgtcagcgggtgttggcgggtgtcggggctggcttaactatgcggcatcagagcagattgtactgagagtgcaccatatgcggtgtgaaataccgcacagatgcgtaaggagaaaataccgcatcaggcgccattcgccattcaggctgcgcaactgttgggaagggcgatcggtgcgggcctcttcgctattacgccagctggcgaaagggggatgtgctgcaaggcgattaagttgggtaacgccagggttttcccagtcacgacgttgtaaaacgacggccagtgccaagctg

SEQ ID NO: 713 - DNA, 8231 bp, synthetic construct
  source 1..8231: mol_type = other DNA
tgtagtcttatgcaatactcttgtagtcttgcaacatggtaacgatgagttagcaacatgccttacaaggagagaaaaagcaccgtgcatgccgattggtggaagtaaggtggtacgatcgtgccttattaggaaggcaacagacgggtctgacatggattggacgaaccactgaattgccgcattgcagagatattgtatttaagtgcctagctcgatacataaacgggtctctctggttagaccagatctgagcctgggagctctctggctaactagggaacccactgcttaagcctcaataaagcttgccttgagtgcttcaagtagtgtgtgcccgtctgttgtgtgactctggtaactagagatccctcagacccttttagtcagtgtggaaaatctctagcagtggcgcccgaacagggacttgaaagcgaaagggaaaccagaggagctctctcgacgcaggactcggcttgctgaagcgcgcacggcaagaggcgaggggcggcgactggtgagtacgccaaaaattttgactagcggaggctagaaggagagagatgggtgcgagagcgtcagtattaagcgggggagaattagatcgcgatgggaaaaaattcggttaaggccagggggaaagaaaaaatataaattaaaacatatagtatgggcaagcagggagctagaacgattcgcagttaatcctggcctgttagaaacatcagaaggctgtagacaaatactgggacagctacaaccatcccttcagacaggatcagaagaacttagatcattatataatacagtagcaaccctctattgtgtgcatcaaaggatagagataaaagacaccaaggaagctttagacaagatagaggaagagcaaaacaaaagtaagaccaccgcacagcaagcggccactgatcttcagacctggaggaggagatatgagggacaattggagaagtgaattatataaatataaagtagtaaaaattgaaccattaggagtagcacccaccaaggcaaagagaagagtggtgcagagagaaaaaagagcagtgggaataggagctttgttccttgggttcttgggagcagcaggaagcactatgggcgcagcgtcaatgacgctgacggtacaggccagacaattattgtctggtatagtgcagcagcagaacaatttgctgagggctattgaggcgcaacagcatctgttgcaactcacagtctggggcatcaagcagctccaggcaagaatcctggctgtggaaagatacctaaaggatcaacagctcctggggatttggggttgctctggaaaactcatttgcaccactgctgtgccttggaatgctagttggagtaataaatctctggaacagatttggaatcacacgacctggatggagtgggacagagaaattaacaattacacaagcttaatacactccttaattgaagaatcgcaaaaccagcaagaaaagaatgaacaagaattattggaattagataaatgggcaagtttgtggaattggtttaacataacaaattggctgtggtatataaaattattcataatgatagtaggaggcttggtaggtttaagaatagtttttgctgtactttctatagtgaatagagttaggcagggatattcaccattatcgtttcagacccacctcccaaccccgaggggacccgacaggcccgaaggaatagaagaagaaggtggagagagagacagagacagatccattcgattagtgaacggatctcgacggtatcggttaacttttaaaagaaaaggggggattggggggtacagtgcaggggaaagaatagtagacataatagcaacagacatacaaactaaagaattacaaaaacaaattacaaaattcaaaattttatcgatactagtattatgcccagtacatgaccttatgggactttcctacttggcagtacatctacgtattagtcatcgctattaccatggtgatgcggttttggcagtacatcaatgggcgtggatagcggtttgactcacggggatttccaagtctccaccccattgacgtcaatgggagtttgttttggcaccaaaatcaacgggactttccaaaatgtcgtaacaactccgccccattgacgcaaatgggcggtaggcgtgtacggtgggaggtttatataagcagagctcgtttagtgaaccgtcagatcgcctggagacgccatccacgctgttttgacctccatagaagattctagagctagcgaattgggatccctagagatccgacgccgccatctctaggcccgcgccggccccctcgcacagacttgtgggagaagctcggctactcccctgccccggttaatttgcatataatatttcctagtaactatagaggcttaatgtgcgataaaagacagataatctgttctttttaatactagctacattttacatgataggcttggatttctataagagatacaaatactaaattattattttaaaaaacagcacaaaaggaaactcaccctaactgtaaagtaattgtgtgttttgagactataaatatgcatgcgagaaaagccttgtttgccaccatggaacggctcggagatcatcattgcgnnnnnnnaccgagtacaagcccacggtgcgcctcgccacccgcgacgacgtccccagggccgtacgcaccctcgccgccgcgttcgccgactaccccgccacgcgccacaccgtcgatccggaccgccacatcgagcgggtcaccgagctgcaagaactcttcctcacgcgcgtcgggctcgacatcggcaaggtgtgggtcgcggacgacggcgccgcggtggcggtctggaccacgccggagagcgtcgaagcgggggcggtgttcgccgagatcggcccgcgcatggccgagttgagcggttcccggctggccgcgcagcaacagatggaaggcctcctggcgccgcaccggcccaaggagcccgcgtggttcctggccaccgtcggcgtctcgcccgaccaccagggcaagggtctgggcagcgccgtcgtgctccccggagtggaggcggccgagcgcgccggggtgcccgccttcctggagacctccgcgccccgcaacctccccttctacgagcggctcggcttcaccgtcaccgccgacgtcgaggtgcccgaaggaccgcgcacctggtgcatgacccgcaagcccggtgcctgactcgaggcggccgctaaatagttgaatttaaatagatctccagcacagtggtaaatagttgattcgaacaaggatctgcgatcgctccggtgcccgtcagtgggcagagcgcacatcgcccacagtccccgagaagttggggggaggggtcggcaattgaacgggtgcctagagaaggtggcgcggggtaaactgggaaagtgatgtcgtgtactggctccgcctttttcccgagggtgggggagaaccgtatataagtgcagtagtcgccgtgaacgttctttttcgcaacgggtttgccgccagaacacagctgaagcttcgaggggctcgcatctctccttcacgcgcccgccgccctacctgaggccgccatccacgccggttgagtcgcgttctgccgcctcccgcctgtggtgcctcctgaactgcgtccgccgtctaggtaagtttaaagctcaggtcgagaccgggcctttgtccggcgctcccttggagcctacctagactcagccggctctccacgctttgcctgaccctgcttgctcaactctacgtctttgtttcgttttctgttctgcgccgttacagatccaagctgtgaccggcgcctacgcccatgggcatggccaagcctttgtctcaagaagaatccaccctcattgaaagagcaacggctacaatcaacagcatccccatctctgaagactacagcgtcgccagcgcagctctctctagcgacggccgcatcttcactggtgtcaatgtatatcattttactgggggaccttgtgcagaactcgtggtgctgggcactgctgctgctgcggcagctggcaacctgacttgtatcgtcgcgatcggaaatgagaacaggggcatcttgagcccctgcggacggtgccgacaggtgcttctcgatctgcatcctgggatcaaagccatagtgaaggacagtgatggacagccgacggcagttgggattcgtgaattgctgccctctggttatgtgtgggagggctaagcacaattcgagctcgcgtcgacaatcaacctctggattacaaaatttgtgaaagattgactggtattcttaactatgttgctccttttacgctatgtggatacgctgctttaatgcctttgtatcatgctattgcttcccgtatggctttcattttctcctccttgtataaatcctggttgctgtctctttatgaggagttgtggcccgttgtcaggcaacgtggcgtggtgtgcactgtgtttgctgacgcaacccccactggttggggcattgccaccacctgtcagctcctttccgggactttcgctttccccctccctattgccacggcggaactcatcgccgcctgccttgcccgctgctggacaggggctcggctgttgggcactgacaattccgtggtgttgtcggggaaatcatcgtcctttccttggctgctcgcctgtgttgccacctggattctgcgcgggacgtccttctgctacgtcccttcggccctcaatccagcggaccttccttcccgcggcctgctgccggctctgcggcctcttccgcgtcttcgccttcgccctcagacgagtcggatctccctttgggccgcctccccgcctggtacctttaagaccaatgacttacaaggcagctgtagatcttagccactttttaaaagaaaaggggggactggaagggctaattcactcccaacgaagataagatctgctttttgcttgtactgggtctctctggttagaccagatctgagcctgggagctctctggctaactagggaacccactgcttaagcctcaataaagcttgccttgagtgcttcaagtagtgtgtgcccgtctgttgtgtgactctggtaactagagatccctcagacccttttagtcagtgtggaaaatctctagcagtagtagttcatgtcatcttattattcagtatttataacttgcaaagaaatgaatatcagagagtgagaggaacttgtttattgcagcttataatggttacaaataaagcaatagcatcacaaatttcacaaataaagcatttttttcactgcattctagttgtggtttgtccaaactcatcaatgtatcttatcatgtctggctctagctatcccgcccctaactccgcccatcccgcccctaactccgcccagttccgcccattctccgccccatggctgactaattttttttatttatgcagaggccgaggccgcctcggcctctgagctattccagaagtagtgaggaggcttttttggaggcctagacttttgcagagaccaaattcgtaatcatgtcatagctgtttcctgtgtgaaattgttatccgctcacaattccacacaacatacgagccggaagcataaagtgtaaagcctggggtgcctaatgagtgagctaactcacattaattgcgttgcgctcactgcccgctttccagtcgggaaacctgtcgtgccagctgcattaatgaatcggccaacgcgcggggagaggcggtttgcgtattgggcgctcttccgcttcctcgctcactgactcgctgcgctcggtcgttcggctgcggcgagcggtatcagctcactcaaaggcggtaatacggttatccacagaatcaggggataacgcaggaaagaacatgtgagcaaaaggccagcaaaaggccaggaaccgtaaaaaggccgcgttgctggcgtttttccataggctccgcccccctgacgagcatcacaaaaatcgacgctcaagtcagaggtggcgaaacccgacaggactataaagataccaggcgtttccccctggaagctccctcgtgcgctctcctgttccgaccctgccgcttaccggatacctgtccgcctttctcccttcgggaagcgtggcgctttctcatagctcacgctgtaggtatctcagttcggtgtaggtcgttcgctccaagctgggctgtgtgcacgaaccccccgttcagcccgaccgctgcgccttatccggtaactatcgtcttgagtccaacccggtaagacacgacttatcgccactggcagcagccactggtaacaggattagcagagcgaggtatgtaggcggtgctacagagttcttgaagtggtggcctaactacggctacactagaagaacagtatttggtatctgcgctctgctgaagccagttaccttcggaaaaagagttggtagctcttgatccggcaaacaaaccaccgctggtagcggtggtttttttgtttgcaagcagcagattacgcgcagaaaaaaaggatctcaagaagatcctttgatcttttctacggggtctgacgctcagtggaacgaaaactcacgttaagggattttggtcatgagattatcaaaaaggatcttcacctagatccttttaaattaaaaatgaagttttaaatcaatctaaagtatatatgagtaaacttggtctgacagttaccaatgcttaatcagtgaggcacctatctcagcgatctgtctatttcgttcatccatagttgcctgactccccgtcgtgtagataactacgatacgggagggcttaccatctggccccagtgctgcaatgataccgcgagacccacgctcaccggctccagatttatcagcaataaaccagccagccggaagggccgagcgcagaagtggtcctgcaactttatccgcctccatccagtctattaattgttgccgggaagctagagtaagtagttcgccagttaatagtttgcgcaacgttgttgccattgctacaggcatcgtggtgtcacgctcgtcgtttggtatggcttcattcagctccggttcccaacgatcaaggcgagttacatgatcccccatgttgtgcaaaaaagcggttagctccttcggtcctccgatcgttgtcagaagtaagttggccgcagtgttatcactcatggttatggcagcactgcataattctcttactgtcatgccatccgtaagatgcttttctgtgactggtgagtactcaaccaagtcattctgagaatagtgtatgcggcgaccgagttgctcttgcccggcgtcaatacgggataataccgcgccacatagcagaactttaaaagtgctcatcattggaaaacgttcttcggggcgaaaactctcaaggatcttaccgctgttgagatccagttcgatgtaacccactcgtgcacccaactgatcttcagcatcttttactttcaccagcgtttctgggtgagcaaaaacaggaaggcaaaatgccgcaaaaaagggaataagggcgacacggaaatgttgaatactcatactcttcctttttcaatattattgaagcatttatcagggttattgtctcatgagcggatacatatttgaatgtatttagaaaaataaacaaataggggttccgcgcacatttccccgaaaagtgccacctgacgtctaagaaaccattattatcatgacattaacctataaaaataggcgtatcacgaggccctttcgtctcgcgcgtttcggtgatgacggtgaaaacctctgacacatgcagctcccggagacggtcacagcttgtctgtaagcggatgccgggagcagacaagcccgtcagggcgcgtcagcgggtgttggcgggtgtcggggctggcttaactatgcggcatcagagcagattgtactgagagtgcaccatatgcggtgtgaaataccgcacagatgcgtaaggagaaaataccgcatcaggcgccattcgccattcaggctgcgcaactgttgggaagggcgatcggtgcgggcctcttcgctattacgccagctggcgaaagggggatgtgctgcaaggcgattaagttgggtaacgccagggttttcccagtcacgacgttgtaaaacgacggccagtgccaagctgacgcg

SEQ ID NO: 714 - DNA, 68 bp, synthetic construct
  source 1..68: mol_type = other DNA
tgtttgccaccatggaacggctcggagatcatcattgcgnnnnnnnaccgagtacaagcccacggtgc

SEQ ID NO: 715 - DNA, 52 bp, synthetic construct
  source 1..52: mol_type = other DNA
taaattcaactatttagcggccgcctcgagtcaggcaccgggcttgcgggtc

SEQ ID NO: 716 - DNA, 2322 bp, synthetic construct
  source 1..2322: mol_type = other DNA
atcataagatgatcttcttgagatcgttttggtctgcgcgtaatctcttgctctgaaaacgaaaaaaccgccttgcagggcggtttttcgaaggttctctgagctaccaactctttgaaccgaggtaactggcttggaggagcgcagtcaccaaaacttgtcctttcagtttagccttaaccggcgcatgacttcaagactaactcctctaaatcaattaccagtggctgctgccagtggtgcttttgcatgtctttccgggttggactcaagacgatagttaccggataaggcgcagcggtcggactgaacggggggttcgtgcatacagtccagcttggagcgaactgcctacccggaactgagtgtcaggcgtggaatgagacaaacgcggccataacagcggaatgacaccggtaaaccgaaaggcaggaacaggagagcgcacgagggagccgccagggggaaacgcctggtatctttatagtcctgtcgggtttcgccaccactgatttgagcgtcagatttcgtgatgcttgtcaggggggcggagcctatggaaaaacggctttgccgcggccctctcacttccctgttaagtatcttcctggcatcttccaggaaatctccgccccgttcgtaagccatttccgctcgccgcagtcgaacgaccgagcgtagcgagtcagtgagcgaggaagcggaatatatcctgtatcacatattctgctgacgcaccggtgcagccttttttctcctgccacatgaagcacttcactgacaccctcatcagtgccaacatagtaagccagtatacactccgctagcgctgatgtccggcggtgcttttgccgttacgcaccaccccgtcagtagctgaacaggagggacagctgatagaaacagaagccactggagcacctcaaaaacaccatcatacactaaatcagtaagttggcagcatcacccgacgcactttgcgccgaataaatacctgtgacggaagatcacttcgcagaataaataaatcctggtgtccctgttgataccgggaagccccgggccaacttttggcgaaaatgagacgttgatcggcacgtaagaggttccaactttcaccataatgaaataagatcactaccgggcgtattttttgagttatcgagattttcaggagctaaggaagctaaaatggagaaaaaaatcactggatataccaccgttgatatatcccaatggcatcgtaaagaacattttgaggcatttcagtcagttgctcaatgtacctataaccagaccgttcagctggatattacggcctttttaaagaccgtaaagaaaaataagcacaagttttatccggcctttattcacattcttgcccgcctgatgaatgctcatccggaattccgtatggcaatgaaagacggtgagctggtgatatgggatagtgttcacccttgttacaccgttttccatgagcaaactgaaacgttttcatcgctctggagtgaataccacgacgatttccggcagtttctacacatatattcgcaagatgtggcgtgttacggtgaaaacctggcctatttccctaaagggtttattgagaatatgtttttcgtctcagccaatccctgggtgagtttcaccagttttgatttaaacgtggccaatatggacaacttcttcgcccccgttttcaccatgggcaaatattatacgcaaggcgacaaggtgctgatgccgctggcgattcaggttcatcatgccgtttgtgatggcttccatgtcggcagaatgcttaatgaattacaacagtactgcgatgagtggcagggcggggcgtaatttggtacatctcaaataaaacgaaaggctcagtcgaaagactgggcctttcgttttatctgttgtttgtcggtgaacgctctcgttaactagctatactgatttcgtcagactcacagtcaaacatgccggtcagttggcctggtgatggcgggatcgttgtatatttcttgacaccttttcggcaccgccctaaaattctgcgtcctcataatatatgaggcgatttattacgtgtttacgaagcaaaagctaaaaccaggagctatttaatgccggcagctaagaaaaagaaactggatggcagcgtcgacagtcttcgtttcaaacgaatggccaccatgtagaagactgaattcggtaccttgacagctagctcagtcctaggtataatactagtgtttaaaccgtacgtcgacgctagcataaccccttggggcctctaaacgggtcttgaggggttttttggat

SEQ ID NO: 717 - DNA, 223 bp, synthetic construct
  source 1..223: mol_type = other DNA
tcgagtacccatacgatgttccagattacgcttgagaattcggtaccttgacagctagctcagtcctaggtataatactagtgtaatgcgtctcccattgacgccgcaatgatgatctccgagccgttcggccggcatggtcccagcctcctcgctggcgccggctgggcaacatgcttcggcatggcgaatgggaccgtacgtcgacgctagcataacccct

SEQ ID NO: 718 - DNA, 36 bp, synthetic construct
  source 1..36: mol_type = other DNA
atttaatgccggcagctaagaaaaagaaactggatg

SEQ ID NO: 719 - DNA, 5969 bp, synthetic construct
  source 1..5969: mol_type = other DNA
atcataagatgatcttcttgagatcgttttggtctgcgcgtaatctcttgctctgaaaacgaaaaaaccgccttgcagggcggtttttcgaaggttctctgagctaccaactctttgaaccgaggtaactggcttggaggagcgcagtcaccaaaacttgtcctttcagtttagccttaaccggcgcatgacttcaagactaactcctctaaatcaattaccagtggctgctgccagtggtgcttttgcatgtctttccgggttggactcaagacgatagttaccggataaggcgcagcggtcggactgaacggggggttcgtgcatacagtccagcttggagcgaactgcctacccggaactgagtgtcaggcgtggaatgagacaaacgcggccataacagcggaatgacaccggtaaaccgaaaggcaggaacaggagagcgcacgagggagccgccagggggaaacgcctggtatctttatagtcctgtcgggtttcgccaccactgatttgagcgtcagatttcgtgatgcttgtcaggggggcggagcctatggaaaaacggctttgccgcggccctctcacttccctgttaagtatcttcctggcatcttccaggaaatctccgccccgttcgtaagccatttccgctcgccgcagtcgaacgaccgagcgtagcgagtcagtgagcgaggaagcggaatatatcctgtatcacatattctgctgacgcaccggtgcagccttttttctcctgccacatgaagcacttcactgacaccctcatcagtgccaacatagtaagccagtatacactccgctagcgctgatgtccggcggtgcttttgccgttacgcaccaccccgtcagtagctgaacaggagggacagctgatagaaacagaagccactggagcacctcaaaaacaccatcatacactaaatcagtaagttggcagcatcacccgacgcactttgcgccgaataaatacctgtgacggaagatcacttcgcagaataaataaatcctggtgtccctgttgataccgggaagccccgggccaacttttggcgaaaatgagacgttgatcggcacgtaagaggttccaactttcaccataatgaaataagatcactaccgggcgtattttttgagttatcgagattttcaggagctaaggaagctaaaatggagaaaaaaatcactggatataccaccgttgatatatcccaatggcatcgtaaagaacattttgaggcatttcagtcagttgctcaatgtacctataaccagaccgttcagctggatattacggcctttttaaagaccgtaaagaaaaataagcacaagttttatccggcctttattcacattcttgcccgcctgatgaatgctcatccggaattccgtatggcaatgaaagacggtgagctggtgatatgggatagtgttcacccttgttacaccgttttccatgagcaaactgaaacgttttcatcgctctggagtgaataccacgacgatttccggcagtttctacacatatattcgcaagatgtggcgtgttacggtgaaaacctggcctatttccctaaagggtttattgagaatatgtttttcgtctcagccaatccctgggtgagtttcaccagttttgatttaaacgtggccaatatggacaacttcttcgcccccgttttcaccatgggcaaatattatacgcaaggcgacaaggtgctgatgccgctggcgattcaggttcatcatgccgtttgtgatggcttccatgtcggcagaatgcttaatgaattacaacagtactgcgatgagtggcagggcggggcgtaatttggtacatctcaaataaaacgaaaggctcagtcgaaagactgggcctttcgttttatctgttgtttgtcggtgaacgctctcgttaactagctatactgatttcgtcagactcacagtcaaacatgccggtcagttggcctggtgatggcgggatcgttgtatatttcttgacaccttttcggcaccgccctaaaattctgcgtcctcataatatatgaggcgatttattacgtgtttacgaagcaaaagctaaaaccaggagctatttaatgccggcagctaagaaaaagaaactggatggcagcgtcgacatcttcgtggtgctgagcgtgaatcagttcagatgcaaccccaacgccttcagacaagcctccatgaaaaccgacgacgagaagaaggacaccgccatcaagagctacacaagctggctgctgcccaacgacagaaaggagaaggacatggtgcggagcttcctggccctggaccaaggcagcagattctttttcgacctgatgcaagcctggtacggcggcctcacccccgacatcatcaagagcgtgaccaaggagcgggacctggtggacctgtggtgcgccatctactggttcagacccatgaagaaggagctggcctcccaccccatcgacagagtggacctggccaagacctttcagagatactacggcggccccgcctccgacgtggtgcaagagtacctgagcgcctccatcggcgaggactgctgctggaacgactgcagacagaagtaccaagagttctgcaagaacctcggggtggacttcacccccgacctcaagaccctggtgagagagaagctgatcgccgtggccctgaacgacggcagccaagccgccatcagcaacctgttcggcaacggcggcaaggaggacagaaacgtgaaggtgaacatctgcaagaagatcctgattgctctggagaaggccggcaaatccgtgaagtacgtgcgggacgtgcagagcatcatcctgaagtgcgccaacgccaaggacagagaggacttcaacagaatctacgccgacaagaacggcagacccggcaccctgctcctgctcctggacagaaagggcgagaacacctacgacgccgaggtgctgaagagatacctgagaaagaccatcaagagcaagaacgcccccctggtgtggaactacaatcagaagctgttcgagtacatcgagagaggcatccggaatctgctgagaagaaccatcaactacgacgcctgggcctggggcgagatgtggagagtgggccacacccccctgcagaccaaggccacaagaaactaccacttcgcccaagagcagctgaagagacacagcgacatcgccgccgcttcccaaagcagccacgccatcgccgtcgctctgaacgagttcttcgagagccccttcttcgacggcgagaaccccttcaccatctgcccccaccacctgggcaagaacctggaaaagctgttcaaggcctgggccgacgaaaaaaatcagaccgacgaggaggacgccggcgaaaccgccatcaccgactactgcgccgagttcaaggacggcttcgacagagagcccattagaaacctgctgagatacgtgtacgcttccctgagaagcaagtacagcgccaaggagctgatccaagccgccaagtacaatcagcagttcgagagatatcagagacagaaggcccaccccgtgacccccgacaaccaaggctacacctggcccgaggccgtgatcaagcctagcaaggccgagagaaagaacagagagaacagcctggacacaagaatctgggtgagcgtgaagctgctgcaaaaggacggcacctgggagaagcaccacatccccttctacaacctgagattcttcgaagaggtgtacgccgctgcctccatcgccgaggacatgcctagccccaccttcagaaacagcagattcggcttcaagctgcccaagctgctgaacacccacgccaagatcaacaagaaaaagaaggacggcaagaaggacaagaaggccgtgaacgccgccaagagagaggctagaatctacctcgctgccaaggagggcagactgcccgccccctccgtgcccctggacaagctgagcgccgtgatcgctagagtgaacggcaagttccaagtgaccgtgcccgtgaagttcaaggtgaacaagcagcccaagtaccccctgcctcagctggggcagatcatcctgggctacgatcagaacctgaccgccaaccacgcctgggccctgttcgaggtggtgaccgaggacacccccggcgcccacttctgcagaaatcagtacctgagagtgctcaagaccggccaagtgagaagcatcaccaagaccaaggacggccaagagatcgatcagctgagctacgacggcctggagtacaaggagtacggcgagtggagaaagcaagccaagaagttcgcctcccaatggtacatcaccaccaaggtgagaaagggcaaggaaaccaccctgctgagccaacccgccctggagagattcgagagcatcgagaagtacaagcccgccctgtacagattcaacaaggaatacgcccggctgctcctggccgtcatcagaagaaagaccctgaacgagctggaggagatcagacccgagatcttcagactggtggagcaaggcttcggcatctgcagattcggcagcctgagcctgagcagcttcgaggccatcagagccgccaaggccgtgatctacggctacttcagcaccgccctgaagcacgaccacaacacccccatcacagatgacgagagacaagccttcgaccccgagctgttcggcctgctgaacaagctggaaaccctgagacagaacaagggcgaggagaagatcaacagagccgctaacgccctgatcagaatcgccctggagaacaaggccgacttcatcagaggcgagggcgacctgcccaccaccaacaagagcgtcaagaaggggcagaacagcagaagcatggactggctggctagaggcctgttcaacaagatctgtcagctggccgtgatgcacaacatcattcccaccgccgccaacccccacagcacaagccaccaagaccccttcgagcacaacaaggacttcgacgaccctcagcccgccatgaagtgcagatacgctgagttcaagatcgaggacatcggcgacagcgtgctggagagactgggcacctccctgagaaatgccaaggccgggcagaccggcgcctactattacaagggcgcccaagacttcctggcccactacggcctgcaagacatcgaggaagagctgaagaagtgcagaagaggcagaaaggccaacatgccctgctgggagctgcagaagagactgattcagaagctgggcagcaaggacgccgtggtgtacatccccatgagaggcggccggatctacctggctacacacagcgtgaccaccggcgccaagcccatcatcttcaacggcgaagaggtgtgggtgagcaacgccgacgagatcgccgccgtgaacatcggcctgaccatcatccccacaagcaagaaggacgaggagcaccccgacagagagaacgacgacaaggccatcagaaagagcgtcagacggcctagaaagagcggcgagagaagaagcggcgacaagatgcccgccaccgctagaaagaccacaggcggcggccccggcggcggcgccgccgccggcagcggcagccctaagaaaaaacgaaaagttggcagcggaagcaaaaggccggcggccacgaaaaaggccggccaggcaaaaaagaaaaagctcgagtacccatacgatgttccagattacgcttgagaattcggtaccttgacagctagctcagtcctaggtataatactagtgtaatgcgtctcccattgacgccgcaatgatgatctccgagccgttcggccggcatggtcccagcctcctcgctggcgccggctgggcaacatgcttcggcatggcgaatgggaccgtacgtcgacgctagcataaccccttggggcctctaaacgggtcttgaggggttttttggat

SEQ ID NO: 720 - DNA, 28 bp, synthetic construct
  source 1..28: mol_type = other DNA
cagcacaaaaggaaactcaccctaactg

SEQ ID NO: 721 - DNA, 20 bp, synthetic construct
  source 1..20: mol_type = other DNA
tgtggcgcgtggcggggtag

SEQ ID NO: 722 - DNA, 23 bp, synthetic construct
  source 1..23: mol_type = other DNA
catgagcatgcagaggtgagtat

SEQ ID NO: 723 - DNA, 38 bp, synthetic construct
  source 1..38: mol_type = other DNA
cattgacgccatgagcatgcagaggtgagtattttttg

SEQ ID NO: 724 - DNA, 38 bp, synthetic construct
  source 1..38: mol_type = other DNA
gtaccaaaaaatactcacctctgcatgctcatggcgtc

SEQ ID NO: 725 - DNA, 8602 bp, synthetic construct
  source 1..8602: mol_type = other DNA
tggcgaatgggacgcgccctgtagcggcgcattaagcgcggcgggtgtggtggttacgcgcagcgtgaccgctacacttgccagcgccctagcgcccgctcctttcgctttcttcccttcctttctcgccacgttcgccggctttccccgtcaagctctaaatcgggggctccctttagggttccgatttagtgctttacggcacctcgaccccaaaaaacttgattagggtgatggttcacgtagtgggccatcgccctgatagacggtttttcgccctttgacgttggagtccacgttctttaatagtggactcttgttccaaactggaacaacactcaaccctatctcggtctattcttttgatttataagggattttgccgatttcggcctattggttaaaaaatgagctgatttaacaaaaatttaacgcgaattttaacaaaatattaacgtttacaatttcaggtggcacttttcggggaaatgtgcgcggaacccctatttgtttatttttctaaatacattcaaatatgtatccgctcatgaattaattcttagaaaaactcatcgagcatcaaatgaaactgcaatttattcatatcaggattatcaataccatatttttgaaaaagccgtttctgtaatgaaggagaaaactcaccgaggcagttccataggatggcaagatcctggtatcggtctgcgattccgactcgtccaacatcaatacaacctattaatttcccctcgtcaaaaataaggttatcaagtgagaaatcaccatgagtgacgactgaatccggtgagaatggcaaaagtttatgcatttctttccagacttgttcaacaggccagccattacgctcgtcatcaaaatcactcgcatcaaccaaaccgttattcattcgtgattgcgcctgagcgagacgaaatacgcgatcgctgttaaaaggacaattacaaacaggaatcgaatgcaaccggcgcaggaacactgccagcgcatcaacaatattttcacctgaatcaggatattcttctaatacctggaatgctgttttcccggggatcgcagtggtgagtaaccatgcatcatcaggagtacggataaaatgcttgatggtcggaagaggcataaattccgtcagccagtttagtctgaccatctcatctgtaacatcattggcaacgctacctttgccatgtttcagaaacaactctggcgcatcgggcttcccatacaatcgatagattgtcgcacctgattgcccgacattatcgcgagcccatttatacccatataaatcagcatccatgttggaatttaatcgcggcctagagcaagacgtttcccgttgaatatggctcataacaccccttgtattactgtttatgtaagcagacagttttattgttcatgaccaaaatcccttaacgtgagttttcgttccactgagcgtcagaccccgtagaaaagatcaaaggatcttcttgagatcctttttttctgcgcgtaatctgctgcttgcaaacaaaaaaaccaccgctaccagcggtggtttgtttgccggatcaagagctaccaactctttttccgaaggtaactggcttcagcagagcgcagataccaaatactgtccttctagtgtagccgtagttaggccaccacttcaagaactctgtagcaccgcctacatacctcgctctgctaatcctgttaccagtggctgctgccagtggcgataagtcgtgtcttaccgggttggactcaagacgatagttaccggataaggcgcagcggtcgggctgaacggggggttcgtgcacacagcccagcttggagcgaacgacctacaccgaactgagatacctacagcgtgagctatgagaaagcgccacgcttcccgaagggagaaaggcggacaggtatccggtaagcggcagggtcggaacaggagagcgcacgagggagcttccagggggaaacgcctggtatctttatagtcctgtcgggtttcgccacctctgacttgagcgtcgatttttgtgatgctcgtcaggggggcggagcctatggaaaaacgccagcaacgcggcctttttacggttcctggccttttgctggccttttgctcacatgttctttcctgcgttatcccctgattctgtggataaccgtattaccgcctttgagtgagctgataccgctcgccgcagccgaacgaccgagcgcagcgagtcagtgagcgaggaagcggaagagcgcctgatgcggtattttctccttacgcatctgtgcggtatttcacaccgcatatatggtgcactctcagtacaatctgctctgatgccgcatagttaagccagtatacactccgctatcgctacgtgactgggtcatggctgcgccccgacacccgccaacacccgctgacgcgccctgacgggcttgtctgctcccggcatccgcttacagacaagctgtgaccgtctccgggagctgcatgtgtcagaggttttcaccgtcatcaccgaaacgcgcgaggcagctgcggtaaagctcatcagcgtggtcgtgaagcgattcacagatgtctgcctgttcatccgcgtccagctcgttgagtttctccagaagcgttaatgtctggcttctgataaagcgggccatgttaagggcggttttttcctgtttggtcactgatgcctccgtgtaagggggatttctgttcatgggggtaatgataccgatgaaacgagagaggatgctcacgatacgggttactgatgatgaacatgcccggttactggaacgttgtgagggtaaacaactggcggtatggatgcggcgggaccagagaaaaatcactcagggtcaatgccagcgcttcgttaatacagatgtaggtgttccacagggtagccagcagcatcctgcgatgcagatccggaacataatggtgcagggcgctgacttccgcgtttccagactttacgaaacacggaaaccgaagaccattcatgttgttgctcaggtcgcagacgttttgcagcagcagtcgcttcacgttcgctcgcgtatcggtgattcattctgctaaccagtaaggcaaccccgccagcctagccgggtcctcaacgacaggagcacgatcatgcgcacccgtggggccgccatgccggcgataatggcctgcttctcgccgaaacgtttggtggcgggaccagtgacgaaggcttgagcgagggcgtgcaagattccgaataccgcaagcgacaggccgatcatcgtcgcgctccagcgaaagcggtcctcgccgaaaatgacccagagcgctgccggcacctgtcctacgagttgcatgataaagaagacagtcataagtgcggcgacgatagtcatgccccgcgcccaccggaaggagctgactgggttgaaggctctcaagggcatcggtcgagatcccggtgcctaatgagtgagctaacttacattaattgcgttgcgctcactgcccgctttccagtcgggaaacctgtcgtgccagctgcattaatgaatcggccaacgcgcggggagaggcggtttgcgtattgggcgccagggtggtttttcttttcaccagtgagacgggcaacagctgattgcccttcaccgcctggccctgagagagttgcagcaagcggtccacgctggtttgccccagcaggcgaaaatcctgtttgatggtggttaacggcgggatataacatgagctgtcttcggtatcgtcgtatcccactaccgagatatccgcaccaacgcgcagcccggactcggtaatggcgcgcattgcgcccagcgccatctgatcgttggcaaccagcatcgcagtgggaacgatgccctcattcagcatttgcatggtttgttgaaaaccggacatggcactccagtcgccttcccgttccgctatcggctgaatttgattgcgagtgagatatttatgccagccagccagacgcagacgcgccgagacagaacttaatgggcccgctaacagcgcgatttgctggtgacccaatgcgaccagatgctccacgcccagtcgcgtaccgtcttcatgggagaaaataatactgttgatgggtgtctggtcagagacatcaagaaataacgccggaacattagtgcaggcagcttccacagcaatggcatcctggtcatccagcggatagttaatgatcagcccactgacgcgttgcgcgagaagattgtgcaccgccgctttacaggcttcgacgccgcttcgttctaccatcgacaccaccacgctggcacccagttgatcggcgcgagatttaatcgccgcgacaatttgcgacggcgcgtgcagggccagactggaggtggcaacgccaatcagcaacgactgtttgcccgccagttgttgtgccacgcggttgggaatgtaattcagctccgccatcgccgcttccactttttcccgcgttttcgcagaaacgtggctggcctggttcaccacgcgggaaacggtctgataagagacaccggcatactctgcgacatcgtataacgttactggtttcacattcaccaccctgaattgactctcttccgggcgctatcatgccataccgcgaaaggttttgcgccattcgatggtgtccgggatctcgacgctctcccttatgcgactcctgcattaggaagcagcccagtagtaggttgaggccgttgagcaccgccgccgcaaggaatggtgcatgcaaggagatggcgcccaacagtcccccggccacggggcctgccaccatacccacgccgaaacaagcgctcatgagcccgaagtggcgagcccgatcttccccatcggtgatgtcggcgatataggcgccagcaaccgcacctgtggcgccggtgatgccggccacgatgcgtccggcgtagaggatcgagatctcgatcccgcgaaattaatacgactcactataggggaattgtgagcggataacaattcccctctagaaataattttgtttaactttaagaaggagatataccatgggcagcagccatcatcatcatcatcacagcagcggcctggtgccgcgcggcagccatatggctagcatgactggtggacagcaaatgggtcgcggatccatgccggcagctaagaaaaagaaactggatggcagcgtcgacatcttccccacacagagaagaaacaccatgagcggcaacgtggtgagaagctacaagagcgtgctcagacccaacatcagaaagagagagctgctggacgccaccttcaactggttcgacagagcctacaagaagttcttcgacgtgttcgtgtgcctgtacggcggcgtggagcacgacaccgtgcacagcgccctgctgaaggaaaccaccgaccccgacctggtgtgcgccaccatgtggttcagagtggtgcccaagagcagctgcgacggcatcagcgcccaagagatgatcagaagattcggcgtgtacgccggccacgagcctagcgccgtggccatgagctacctgaccggcaacttcgacgacaagaagaaccactggatcgactgcagagagaagttcgtggccctggctagagacatggtggtgaagcccgagagcctgagcatcgacatcaagagcatgatcgagcacaagatcctgcccatctgcagccaagacaactggcaagcctggaacgccatcagccaactgttcggcgagggcaagaaggagaacaaggccgagaaggctcagatcttcgtggacgtggtgagcatgctgagcaacaacagcgtgcagacctgggaggactacaaagaggtgatcagcaaggccaccggctgcagaaccgccggcgagatcaacagcaagttcggcggcagacccggcatcctgagcgtggacttcagcaaggacgacaccggcagcctgcccaaggacttcatcgagagaagaatcaaggacctgagccaaaaggccaaggagaagagcgccgcctacgagctgcccaacagaatgagactgagagagctgatcgctagcgtgatcggcccctacagactggaaacctggagcagcgtggctcagagagcctgcggcgacatcagaagcaagaacagcaacaacctgctgtacgctagcgagagattcaacagaaccaaggagatcgaggagatcctgagcgccaagggcgacgtggctagagcccaaaacatcctagggcagttcagaagcggcgagttcaacgagttcgccgtggagaagagacacctgggcaacctggagagcctgtacaacatctggagcaagagcgacatggacaccggcatcgaggagtacagcagcatccacaaggacgagtacgaccgggaccccatcgtggacctgtacagacacatctacccccacagagaggtgatcagcgccaagaacttcatcgacgccgccgtgctgaacaagctgctgagactgaacgctagcagacacgtgcaccccaccgtgttcggcaagaccgtgatcagcttcagccccaagagcagcgcctacggcagaatcaccccccctagcgagatcgtgagaggcagacccgccggcagccacggcatgatctggctgaccatggagctgttcgacgacggcaagtggatcgagcaccacctgcccttccacaacagcagatactacgaagaggtgtactgctaccaagagggcctgcccgtgaaggacgagcctagaagccccatgttcggctacagagtgggcaacgccatcgccgacacaagcaagatcgacaacagacggagaaaggctagcaagcagttcctgagagctcagcagaacatcacccacaacgtgagcttcgacgagaacaccgccttcagcgtggtgagaaacggcgaggacttcagcatcaccatcagcagcagaatcaaggctagcaatgctaagagcctgatgaccatcggcgacagaatcatgggcatcgatcagaatcagaccgccgccaacacctacagcatctgggaggtggtgggcgacggcgacgccggcagcattcagcacggcaacctgagcctgaagagaatcgaggacggccacatcacaagcatcatcagaggcagaggcggcaacttcgatcagctgaactacggcggcctgagctacgccaagttcagcgagtggagaagcgctagactgggcttcatcagcagcctgaacgccgagctggctagcaagatgaactgggactggtgctgcctgtacgagtggaacgctagatacgctagcgccctgagaaagatcatctacagccacaagggcatcgacatcgagagagtgttcagaagagagatcgaggacttcgtggagggcgtgctgagaatcggcagcctgagcagcgacgccctgcagtgcctgaccaacgccaagagcctgatcagcagctacttcttcctgaacggcaagaaggagcccgaggagcagagaaagttcgaccaaggcctgttcgacctgagcgccaagattgacaagaagagagtgaacaagagacagcaaaagaccaagagaatcatgagcagcatcatgcagatcgctagagacagaggcgtgagcttcatcgtggtggagggcaagctgagcaccgccaccaaggacaacaagagcaaggccaatcagaaggccatcgactggtgcgctagagccgtggtggagaacctggagcacagctgcagcctggtgggcatcaagctggtggccatcgaccccatgaacacaagccacctggaccccttcgtgtacgtgctcaagacaagcctgggcaaggaggctagattcgctagcgtggtgcccgccaagatcaacgctagacacatgaagaacttcaagagctggagcagcctgctggccggcaacggcaagatcaaaaagaccaccgacgccatctacgtgggcgccttccaagacttctgcagagagtacggcttcgtggccgaggacatcagcaagatgagccaaagcgagatccaagacaagctgagcagccatcagttcgtgctggtgcctcagagaggcggcagagtgtacatgagcacccaccccgtgagcagcgaggccaagaagatcgtgtacgccggcagagagagatggtacaacaacgccgacgtggtggccgccgtgaacatcaccctgagaggctgcgagagactgagcgctagcagaaagaccgctagcacaagaacaggcggcggccccggcggcggcgccgccgccggcagcggcagccctaagaaaaaacgaaaagttggcagcggaagcaaaaggccggcggccacgaaaaaggccggccaggcaaaaaagaaaaagctcgagtacccatacgatgttccagattacgcttgactcgagcaccaccaccaccaccactgagatccggctgctaacaaagcccgaaaggaagctgagttggctgctgccaccgctgagcaataactagcataaccccttggggcctctaaacgggtcttgaggggttttttgctgaaaggaggaactatatccggat

SEQ ID NO: 726 - RNA, 60 nt, synthetic construct
  source 1..60: mol_type = other RNA
atcgcaacatctcagaaacccgtcctaagttgacgggtgagcaagggcgaggagctgttc

SEQ ID NO: 727 - RNA, 62 nt, synthetic construct
  source 1..62: mol_type = other RNA
atcgcaacatctcagaaacccgtcctaagttgacggcgcaatgatgatctccgagccgttcc

SEQ ID NO: 728 - protein, 1021 aa, synthetic construct
IFPTQRRNTMSGNVVRSYKSVLRPNIRKRELLDATFNWFDRAYKKFFDVFVCLYGGVEHDTVHSALLKETTDPDLVCATMWFRVVPKSSCDGISAQEMIRRFGVYAGHEPSAVAMSYLTGNFDDKKNHWIDCREKFVALARDMVVKPESLSIDIKSMIEHKILPICSQDNWQAWNAISQLFGEGKKENKAEKAQIFVDVVSMLSNNSVQTWEDYKEVISKATGCRTAGEINSKFGGRPGILSVDFSKDDTGSLPKDFIERRIKDLSQKAKEKSAAYELPNRMRLRELIASVIGPYRLETWSSVAQRACGDIRSKNSNNLLYASERFNRTKEIEEILSAKGDVARAQSILGQFRSGEFNEFAVEKRHLGNLESLYNIWSKSDMDTGIEEYSSIHKDEYDRDPIVDLYRHIYPHREVISAKNFIDAAVLNKLLRLNASRHVHPTVFGKTVISFSPKSSAYGRITPPSEIVRGRPAGSHGMIWLTMELFDDGKWIEHHLPFHNSRYYEEVYCYQEGLPVKDEPRSPMFGYRVGNAIADTSKIDNRRRKASKQFLRAQQNITHNVSFDENTAFSVVRNGEDFSITISSRIKASNAKSLMTIGDRIMGIDQNQTAANTYSIWEVVGDGDAGSIQHGNLSLKRIEDGHITSIIRGRGGNFDQLNYGGLSYAKFSEWRSARLGFISSLNAELASKMNWDWCCLYEWNARYASALRKIIYSHKGIDIERVFRREIEDFVEGVLRIGSLSSDALQCLTNAKSLISSYFFLNGKKEPEEQRKFDQGLFDLSAKIDKKRVNKRQQKTKRIMSSIMQIARDRGVSFIVVEGKLSTATKDNKSKANQKAIDWCARAVVENLEHSCSLVGIKLVAIDPMNTSHLDPFVYVLKTSLGKEARFASVVPAKINARHMKNFKSWSSLLAGNGKIKKTTDAIYVGAFQDFCREYGFVAEDISKMSQSEIQDKLSSHQFVLVPQRGGRVYMSTHPVSSEAKKIVYAGRERWYNNADVVAAVNITLRGCERLSASRKTASTR

SEQ ID NO: 729 - DNA, 5629 bp, synthetic construct
  source 1..5629: mol_type = other DNA
atcataagatgatcttcttgagatcgttttggtctgcgcgtaatctcttgctctgaaaacgaaaaaaccgccttgcagggcggtttttcgaaggttctctgagctaccaactctttgaaccgaggtaactggcttggaggagcgcagtcaccaaaacttgtcctttcagtttagccttaaccggcgcatgacttcaagactaactcctctaaatcaattaccagtggctgctgccagtggtgcttttgcatgtctttccgggttggactcaagacgatagttaccggataaggcgcagcggtcggactgaacggggggttcgtgcatacagtccagcttggagcgaactgcctacccggaactgagtgtcaggcgtggaatgagacaaacgcggccataacagcggaatgacaccggtaaaccgaaaggcaggaacaggagagcgcacgagggagccgccagggggaaacgcctggtatctttatagtcctgtcgggtttcgccaccactgatttgagcgtcagatttcgtgatgcttgtcaggggggcggagcctatggaaaaacggctttgccgcggccctctcacttccctgttaagtatcttcctggcatcttccaggaaatctccgccccgttcgtaagccatttccgctcgccgcagtcgaacgaccgagcgtagcgagtcagtgagcgaggaagcggaatatatcctgtatcacatattctgctgacgcaccggtgcagccttttttctcctgccacatgaagcacttcactgacaccctcatcagtgccaacatagtaagccagtatacactccgctagcgctgatgtccggcggtgcttttgccgttacgcaccaccccgtcagtagctgaacaggagggacagctgatagaaacagaagccactggagcacctcaaaaacaccatcatacactaaatcagtaagttggcagcatcacccgacgcactttgcgccgaataaatacctgtgacggaagatcacttcgcagaataaataaatcctggtgtccctgttgataccgggaagccccgggccaacttttggcgaaaatgagacgttgatcggcacgtaagaggttccaactttcaccataatgaaataagatcactaccgggcgtattttttgagttatcgagattttcaggagctaaggaagctaaaatggagaaaaaaatcactggatataccaccgttgatatatcccaatggcatcgtaaagaacattttgaggcatttcagtcagttgctcaatgtacctataaccagaccgttcagctggatattacggcctttttaaagaccgtaaagaaaaataagcacaagttttatccggcctttattcacattcttgcccgcctgatgaatgctcatccggaattccgtatggcaatgaaagacggtgagctggtgatatgggatagtgttcacccttgttacaccgttttccatgagcaaactgaaacgttttcatcgctctggagtgaataccacgacgatttccggcagtttctacacatatattcgcaagatgtggcgtgttacggtgaaaacctggcctatttccctaaagggtttattgagaatatgtttttcgtctcagccaatccctgggtgagtttcaccagttttgatttaaacgtggccaatatggacaacttcttcgcccccgttttcaccatgggcaaatattatacgcaaggcgacaaggtgctgatgccgctggcgattcaggttcatcatgccgtttgtgatggcttccatgtcggcagaatgcttaatgaattacaacagtactgcgatgagtggcagggcggggcgtaatttggtacatctcaaataaaacgaaaggctcagtcgaaagactgggcctttcgttttatctgttgtttgtcggtgaacgctctcgttaactagctatactgatttcgtcagactcacagtcaaacatgccggtcagttggcctggtgatggcgggatcgttgtatatttcttgacaccttttcggcaccgccctaaaattctgcgtcctcataatatatgaggcgatttattacgtgtttacgaagcaaaagctaaaaccaggagctatttaatgccggcagctaagaaaaagaaactggatggcagcgtcgacatcttccccacacagagaagaaacaccatgagcggcaacgtggtgagaagctacaagagcgtgctcagacccaacatcagaaagagagagctgctggacgccaccttcaactggttcgacagagcctacaagaagttcttcgacgtgttcgtgtgcctgtacggcggcgtggagcacgacaccgtgcacagcgccctgctgaaggaaaccaccgaccccgacctggtgtgcgccaccatgtggttcagagtggtgcccaagagcagctgcgacggcatcagcgcccaagagatgatcagaagattcggcgtgtacgccggccacgagcctagcgccgtggccatgagctacctgaccggcaacttcgacgacaagaagaaccactggatcgactgcagagagaagttcgtggccctggctagagacatggtggtgaagcccgagagcctgagcatcgacatcaagagcatgatcgagcacaagatcctgcccatctgcagccaagacaactggcaagcctggaacgccatcagccaactgttcggcgagggcaagaaggagaacaaggccgagaaggctcagatcttcgtggacgtggtgagcatgctgagcaacaacagcgtgcagacctgggaggactacaaagaggtgatcagcaaggccaccggctgcagaaccgccggcgagatcaacagcaagttcggcggcagacccggcatcctgagcgtggacttcagcaaggacgacaccggcagcctgcccaaggacttcatcgagagaagaatcaaggacctgagccaaaaggccaaggagaagagcgccgcctacgagctgcccaacagaatgagactgagagagctgatcgctagcgtgatcggcccctacagactggaaacctggagcagcgtggctcagagagcctgcggcgacatcagaagcaagaacagcaacaacctgctgtacgctagcgagagattcaacagaaccaaggagatcgaggagatcctgagcgccaagggcgacgtggctagagcccaaagcatcctagggcagttcagaagcggcgagttcaacgagttcgccgtggagaagagacacctgggcaacctggagagcctgtacaacatctggagcaagagcgacatggacaccggcatcgaggagtacagcagcatccacaaggacgagtacgaccgggaccccatcgtggacctgtacagacacatctacccccacagagaggtgatcagcgccaagaacttcatcgacgccgccgtgctgaacaagctgctgagactgaacgctagcagacacgtgcaccccaccgtgttcggcaagaccgtgatcagcttcagccccaagagcagcgcctacggcagaatcaccccccctagcgagatcgtgagaggcagacccgccggcagccacggcatgatctggctgaccatggagctgttcgacgacggcaagtggatcgagcaccacctgcccttccacaacagcagatactacgaagaggtgtactgctaccaagagggcctgcccgtgaaggacgagcctagaagccccatgttcggctacagagtgggcaacgccatcgccgacacaagcaagatcgacaacagacggagaaaggctagcaagcagttcctgagagctcagcagaacatcacccacaacgtgagcttcgacgagaacaccgccttcagcgtggtgagaaacggcgaggacttcagcatcaccatcagcagcagaatcaaggctagcaatgctaagagcctgatgaccatcggcgacagaatcatgggcatcgatcagaatcagaccgccgccaacacctacagcatctgggaggtggtgggcgacggcgacgccggcagcattcagcacggcaacctgagcctgaagagaatcgaggacggccacatcacaagcatcatcagaggcagaggcggcaacttcgatcagctgaactacggcggcctgagctacgccaagttcagcgagtggagaagcgctagactgggcttcatcagcagcctgaacgccgagctggctagcaagatgaactgggactggtgctgcctgtacgagtggaacgctagatacgctagcgccctgagaaagatcatctacagccacaagggcatcgacatcgagagagtgttcagaagagagatcgaggacttcgtggagggcgtgctgagaatcggcagcctgagcagcgacgccctgcagtgcctgaccaacgccaagagcctgatcagcagctacttcttcctgaacggcaagaaggagcccgaggagcagagaaagttcgaccaaggcctgttcgacctgagcgccaagattgacaagaagagagtgaacaagagacagcaaaagaccaagagaatcatgagcagcatcatgcagatcgctagagacagaggcgtgagcttcatcgtggtggagggcaagctgagcaccgccaccaaggacaacaagagcaaggccaatcagaaggccatcgactggtgcgctagagccgtggtggagaacctggagcacagctgcagcctggtgggcatcaagctggtggccatcgaccccatgaacacaagccacctggaccccttcgtgtacgtgctcaagacaagcctgggcaaggaggctagattcgctagcgtggtgcccgccaagatcaacgctagacacatgaagaacttcaagagctggagcagcctgctggccggcaacggcaagatcaaaaagaccaccgacgccatctacgtgggcgccttccaagacttctgcagagagtacggcttcgtggccgaggacatcagcaagatgagccaaagcgagatccaagacaagctgagcagccatcagttcgtgctggtgcctcagagaggcggcagagtgtacatgagcacccaccccgtgagcagcgaggccaagaagatcgtgtacgccggcagagagagatggtacaacaacgccgacgtggtggccgccgtgaacatcaccctgagaggctgcgagagactgagcgctagcagaaagaccgctagcacaagaacaggcggcggccccggcggcggcgccgccgccggcagcggcagccctaagaaaaaacgaaaagttggcagcggaagcaaaaggccggcggccacgaaaaaggccggccaggcaaaaaagaaaaagctcgagtacccatacgatgttccagattacgcttgagaattcggtaccttgacagctagctcagtcctaggtataatactagtatcgcaacatctcagaaacccgtcctaagttgacggcgcaatgatgatctccgagccgttcggccggcatggtcccagcctcctcgctggcgccggctgggcaacatgcttcggcatggcgaatgggaccgtacgtcgacgctagcataaccccttggggcctctaaacgggtcttgaggggttttttggat

SEQ ID NO: 730 - DNA, 8134 bp, synthetic construct
  source 1..8134: mol_type = other DNA
acgcgtgtagtcttatgcaatactcttgtagtcttgcaacatggtaacgatgagttagcaacatgccttacaaggagagaaaaagcaccgtgcatgccgattggtggaagtaaggtggtacgatcgtgccttattaggaaggcaacagacgggtctgacatggattggacgaaccactgaattgccgcattgcagagatattgtatttaagtgcctagctcgatacaataaacgggtctctctggttagaccagatctgagcctgggagctctctggctaactagggaacccactgcttaagcctcaataaagcttgccttgagtgcttcaagtagtgtgtgcccgtctgttgtgtgactctggtaactagagatccctcagacccttttagtcagtgtggaaaatctctagcagtggcgcccgaacagggacctgaaagcgaaagggaaaccagagctctctcgacgcaggactcggcttgctgaagcgcgcacggcaagaggcgaggggcggcgactggtgagtacgccaaaaattttgactagcggaggctagaaggagagagatgggtgcgagagcgtcagtattaagcgggggagaattagatcgcgatgggaaaaaattcggttaaggccagggggaaagaaaaaatataaattaaaacatatagtatgggcaagcagggagctagaacgattcgcagttaatcctggcctgttagaaacatcagaaggctgtagacaaatactgggacagctacaaccatcccttcagacaggatcagaagaacttagatcattatataatacagtagcaaccctctattgtgtgcatcaaaggatagagataaaagacaccaaggaagctttagacaagatagaggaagagcaaaacaaaagtaagaccaccgcacagcaagcggccactgatcttcagacctggaggaggagatatgagggacaattggagaagtgaattatataaatataaagtagtaaaaattgaaccattaggagtagcacccaccaaggcaaagagaagagtggtgcagagagaaaaaagagcagtgggaataggagctttgttccttgggttcttgggagcagcaggaagcactatgggcgcagcctcaatgacgctgacggtacaggccagacaattattgtctggtatagtgcagcagcagaacaatttgctgagggctattgaggcgcaacagcatctgttgcaactcacagtctggggcatcaagcagctccaggcaagaatcctggctgtggaaagatacctaaaggatcaacagctcctggggatttggggttgctctggaaaactcatttgcaccactgctgtgccttggaatgctagttggagtaataaatctctggaacagattggaatcacacgacctggatggagtgggacagagaaattaacaattacacaagcttaatacactccttaattgaagaatcgcaaaaccagcaagaaaagaatgaacaagaattattggaattagataaatgggcaagtttgtggaattggtttaacataacaaattggctgtggtatataaaattattcataatgatagtaggaggcttggtaggtttaagaatagtttttgctgtactttctatagtgaatagagttaggcagggatattcaccattatcgtttcagacccacctcccaaccccgaggggacccgacaggcccgaaggaatagaagaagaaggtggagagagagacagagacagatccattcgattagtgaacggatctcgacggtatcggttaacttttaaaagaaaaggggggattggggggtacagtgcaggggaaagaatagtagacataatagcaacagacatacaaactaaagaattacaaaaacaaattacaaaattcaaaattttatcgatactagtattatgcccagtacatgaccttatgggactttcctacttggcagtacatctacgtattagtcatcgctattaccatggtgatgcggttttggcagtacatcaatgggcgtggatagcggtttgactcacggggatttccaagtctccaccccattgacgtcaatgggagtttgttttggcaccaaaatcaacgggactttccaaaatgtcgtaacaactccgccccattgacgcaaatgggcggtaggcgtgtacggtgggaggtttatataagcagagctcgtttagtgaaccgtcagatcgcctggagacgccatccacgctgttttgacctccatagaagattctagagcgagaaaagccttgtttgccaccatggaacggctcggagatcatcattgcgnaangtgagcaagggcgaggagctgttcaccggggtggtgcccatcctggtcgagctggacggcgacgtaaacggccacaagttcagcgtgtccggcgagggcgagggcgatgccacctacggcaagctgaccctgaagttcatctgcaccaccggcaagctgcccgtgccctggcccaccctcgtgaccaccctgacctacggcgtgcagtgcttcagccgctaccccgaccacatgaagcagcacgacttcttcaagtccgccatgcccgaaggctacgtccaggagcgcaccatcttcttcaaggacgacggcaactacaagacccgcgccgaggtgaagttcgagggcgacaccctggtgaaccgcatcgagctgaagggcatcgacttcaaggaggacggcaacatcctggggcacaagctggagtacaactacaacagccacaacgtctatatcatggccgacaagcagaagaacggcatcaaggtgaacttcaagatccgccacaacatcgaggacggcagcgtgcagctcgccgaccactaccagcagaacacccccatcggcgacggccccgtgctgctgcccgacaaccactacctgagcacccagtccaagctgagcaaagaccccaacgagaagcgcgatcacatggtcctgctggagttcgtgaccgccgccgggatcactctcggcatggacgagctgtacaagtaactcgaggcggccgcgaaggatctgcgatcgctccggtgcccgtcagtgggcagagcgcacatcgcccacagtccccgagaagttggggggaggggtcggcaattgaacgggtgcctagagaaggtggcgcggggtaaactgggaaagtgatgtcgtgtactggctccgcctttttcccgagggtgggggagaaccgtatataagtgcagtagtcgccgtgaacgttctttttcgcaacgggtttgccgccagaacacagctgaagcttcgaggggctcgcatctctccttcacgcgcccgccgccctacctgaggccgccatccacgccggttgagtcgcgttctgccgcctcccgcctgtggtgcctcctgaactgcgtccgccgtctaggtaagtttaaagctcaggtcgagaccgggcctttgtccggcgctcccttggagcctacctagactcagccggctctccacgctttgcctgaccctgcttgctcaactctacgtctttgtttcgttttctgttctgcgccgttacagatccaagctgtgaccggcgcctacgctagatgaccgagtacaagcccacggtgcgcctcgccacccgcgacgacgtccccagggccgtacgcaccctcgccgccgcgttcgccgactaccccgccacgcgccacaccgtcgatccggaccgccacatcgagcgggtcaccgagctgcaagaactcttcctcacgcgcgtcgggctcgacatcggcaaggtgtgggtcgcggacgacggcgccgcggtggcggtctggaccacgccggagagcgtcgaagcgggggcggtgttcgccgagatcggcccgcgcatggccgagttgagcggttcccggctggccgcgcagcaacagatggaaggcctcctggcgccgcaccggcccaaggagcccgcgtggttcctggccaccgtcggcgtctcgcccgaccaccagggcaagggtctgggcagcgccgtcgtgctccccggagtggaggcggccgagcgcgccggggtgcccgccttcctggagacctccgcgccccgcaacctccccttctacgagcggctcggcttcaccgtcaccgccgacgtcgaggtgcccgaaggaccgcgcacctggtgcatgacccgcaagcccggtgcctgagtcgacaatcaacctctggattacaaaatttgtgaaagattgactggtattcttaactatgttgctccttttacgctatgtggatacgctgctttaatgcctttgtatcatgctattgcttcccgtatggctttcattttctcctccttgtataaatcctggttgctgtctctttatgaggagttgtggcccgttgtcaggcaacgtggcgtggtgtgcactgtgtttgctgacgcaacccccactggttggggcattgccaccacctgtcagctcctttccgggactttcgctttccccctccctattgccacggcggaactcatcgccgcctgccttgcccgctgctggacaggggctcggctgttgggcactgacaattccgtggtgttgtcggggaaatcatcgtcctttccttggctgctcgcctgtgttgccacctggattctgcgcgggacgtccttctgctacgtcccttcggccctcaatccagcggaccttccttcccgcggcctgctgccggctctgcggcctcttccgcgtcttcgccttcgccctcagacgagtcggatctccctttgggccgcctccccgcctggtacctttaagaccaatgacttacaaggcagctgtagatcttagccactttttaaaagaaaaggggggactggaagggctaattcactcccaacgaaaataagatctgctttttgcttgtactgggtctctctggttagaccagatctgagcctgggagctctctggctaactagggaacccactgcttaagcctcaataaagcttgccttgagtgcttcaagtagtgtgtgcccgtctgttgtgtgactctggtaactagagatccctcagacccttttagtcagtgtggaaaatctctagcagtagtagttcatgtcatcttattattcagtatttataacttgcaaagaaatgaatatcagagagtgagaggaacttgtttattgcagcttataatggttacaaataaagcaatagcatcacaaatttcacaaataaagcatttttttcactgcattctagttgtggtttgtccaaactcatcaatgtatcttatcatgtctggctctagctatcccgcccctaactccgcccagttccgcccattctccgccccatggctgactaattttttttatttatgcagaggccgaggccgcctcggcctctgagctattccagaagtagtgaggaggcttttttggaggcctagacttttgcagagacggcccaaattcgtaatcatggtcatagctgtttcctgtgtgaaattgttatccgctcacaattccacacaacatacgagccggaagcataaagtgtaaagcctggggtgcctaatgagtgagctaactcacattaattgcgttgcgctcactgcccgctttccagtcgggaaacctgtcgtgccagctgcattaatgaatcggccaacgcgcggggagaggcggtttgcgtattgggcgctcttccgcttcctcgctcactgactcgctgcgctcggtcgttcggctgcggcgagcggtatcagctcactcaaaggcggtaatacggttatccacagaatcaggggataacgcaggaaagaacatgtgagcaaaaggccagcaaaaggccaggaaccgtaaaaaggccgcgttgctggcgtttttccataggctccgcccccctgacgagcatcacaaaaatcgacgctcaagtcagaggtggcgaaacccgacaggactataaagataccaggcgtttccccctggaagctccctcgtgcgctctcctgttccgaccctgccgcttaccggatacctgtccgcctttctcccttcgggaagcgtggcgctttctcatagctcacgctgtaggtatctcagttcggtgtaggtcgttcgctccaagctgggctgtgtgcacgaaccccccgttcagcccgaccgctgcgccttatccggtaactatcgtcttgagtccaacccggtaagacacgacttatcgccactggcagcagccactggtaacaggattagcagagcgaggtatgtaggcggtgctacagagttcttgaagtggtggcctaactacggctacactagaaggacagtatttggtatctgcgctctgctgaagccagttaccttcggaaaaagagttggtagctcttgatccggcaaacaaaccaccgctggtagcggtggtttttttgtttgcaagcagcagattacgcgcagaaaaaaaggatctcaagaagatcctttgatcttttctacggggtctgacgctcagtggaacgaaaactcacgttaagggattttggtcatgagattatcaaaaaggatcttcacctagatccttttaaattaaaaatgaagttttaaatcaatctaaagtatatatgagtaaacttggtctgacagttaccaatgcttaatcagtgaggcacctatctcagcgatctgtctatttcgttcatccatagttgcctgactccccgtcgtgtagataactacgatacgggagggcttaccatctggccccagtgctgcaatgataccgcgagacccacgctcaccggctccagatttatcagcaataaaccagccagccggaagggccgagcgcagaagtggtcctgcaactttatccgcctccatccagtctattaattgttgccgggaagctagagtaagtagttcgccagttaatagtttgcgcaacgttgttgccattgctacaggcatcgtggtgtcacgctcgtcgtttggtatggcttcattcagctccggttcccaacgatcaaggcgagttacatgatcccccatgttgtgcaaaaaagcggttagctccttcggtcctccgatcgttgtcagaagtaagttggccgcagtgttatcactcatggttatggcagcactgcataattctcttactgtcatgccatccgtaagatgcttttctgtgactggtgagtactcaaccaagtcattctgagaatagtgtatgcggcgaccgagttgctcttgcccggcgtcaatacgggataataccgcgccacatagcagaactttaaaagtgctcatcattggaaaacgttcttcggggcgaaaactctcaaggatcttaccgctgttgagatccagttcgatgtaacccactcgtgcacccaactgatcttcagcatcttttactttcaccagcgtttctgggtgagcaaaaacaggaaggcaaaatgccgcaaaaaagggaataagggcgacacggaaatgttgaatactcatactcttcctttttcaatattattgaagcatttatcagggttattgtctcatgagcggatacatatttgaatgtatttagaaaaataaacaaataggggttccgcgcacatttccccgaaaagtgccacctgacgtctaagaaaccattattatcatgacattaacctataaaaataggcgtatcacgaggccctttcgtctcgcgcgtttcggtgatgacggtgaaaacctctgacacatgcagctcccggagacggtcacagcttgtctgtaagcggatgccgggagcagacaagcccgtcagggcgcgtcagcgggtgttggcgggtgtcggggctggcttaactatgcggcatcagagcagattgtactgagagtgcaccatatgcggtgtgaaataccgcacagatgcgtaaggagaaaataccgcatcaggcgccattcgccattcaggctgcgcaactgttgggaagggcgatcggtgcgggcctcttcgctattacgccagctggcgaaagggggatgtgctgcaaggcgattaagttgggtaacgccagggttttcccagtcacgacgttgtaaaacgacggccagtgccaagctg

SEQ ID NO: 731 - DNA, 27 bp, synthetic construct
  source 1..27: mol_type = other DNA
ccaagctggctagcgtttaaacttaag

SEQ ID NO: 732 - DNA, 26 bp, synthetic construct
  source 1..26: mol_type = other DNA
atgatctccgagccgtttttggtacc

SEQ ID NO: 733 - DNA, 31 bp, synthetic construct
  source 1..31: mol_type = other DNA
gctgaagagacacagcagaatcgccgccgct

SEQ ID NO: 734 - DNA, 30 bp, synthetic construct
  source 1..30: mol_type = other DNA
gggaagcggcggcgattctgctgtgtctct

SEQ ID NO: 735 - DNA, 22 bp, synthetic construct
  source 1..22: mol_type = other DNA
ctcacctcgcgacgcaatgatg

SEQ ID NO: 736 - DNA, 26 bp, synthetic construct
  source 1..26: mol_type = other DNA
gcgacgcaatgatgtttttcggtacc

SEQ ID NO: 737 - DNA, 9036 bp, synthetic construct
  source 1..9036: mol_type = other DNA
gacggatcgggagatctcccgatcccctatggtgcactctcagtacaatctgctctgatgccgcatagttaagccagtatctgctccctgcttgtgtgttggaggtcgctgagtagtgcgcgagcaaaatttaagctacaacaaggcaaggcttgaccgacaattgcatgaagaatctgcttagggttaggcgttttgcgctgcttcgcgatgtacgggccagatatacgcgttgacattgattattgactagttattaatagtaatcaattacggggtcattagttcatagcccatatatggagttccgcgttacataacttacggtaaatggcccgcctggctgaccgcccaacgacccccgcccattgacgtcaataatgacgtatgttcccatagtaacgccaatagggactttccattgacgtcaatgggtggagtatttacggtaaactgcccacttggcagtacatcaagtgtatcatatgccaagtacgccccctattgacgtcaatgacggtaaatggcccgcctggcattatgcccagtacatgaccttatgggactttcctacttggcagtacatctacgtattagtcatcgctattaccatggtgatgcggttttggcagtacatcaatgggcgtggatagcggtttgactcacggggatttccaagtctccaccccattgacgtcaatgggagtttgttttggcaccaaaatcaacgggactttccaaaatgtcgtaacaactccgccccattgacgcaaatgggcggtaggcgtgtacggtgggaggtctatataagcagagctctctggctaactagagaacccactgcttactggcttatcgaaattaatacgactcactatagggagacccaagctggctagcgtttaaacttaagcttaccggtgccaccatgccggcagctaagaaaaagaaactggatggcagcgtcgacatcttccccacacagagaagaaacaccatgagcggcaacgtggtgagaagctacaagagcgtgctcagacccaacatcagaaagagagagctgctggacgccaccttcaactggttcgacagagcctacaagaagttcttcgacgtgttcgtgtgcctgtacggcggcgtggagcacgacaccgtgcacagcgccctgctgaaggaaaccaccgaccccgacctggtgtgcgccaccatgtggttcagagtggtgcccaagagcagctgcgacggcatcagcgcccaagagatgatcagaagattcggcgtgtacgccggccacgagcctagcgccgtggccatgagctacctgaccggcaacttcgacgacaagaagaaccactggatcgactgcagagagaagttcgtggccctggctagagacatggtggtgaagcccgagagcctgagcatcgacatcaagagcatgatcgagcacaagatcctgcccatctgcagccaagacaactggcaagcctggaacgccatcagccaactgttcggcgagggcaagaaggagaacaaggccgagaaggctcagatcttcgtggacgtggtgagcatgctgagcaacaacagcgtgcagacctgggaggactacaaagaggtgatcagcaaggccaccggctgcagaaccgccggcgagatcaacagcaagttcggcggcagacccggcatcctgagcgtggacttcagcaaggacgacaccggcagcctgcccaaggacttcatcgagagaagaatcaaggacctgagccaaaaggccaaggagaagagcgccgcctacgagctgcccaacagaatgagactgagagagctgatcgctagcgtgatcggcccctacagactggaaacctggagcagcgtggctcagagagcctgcggcgacatcagaagcaagaacagcaacaacctgctgtacgctagcgagagattcaacagaaccaaggagatcgaggagatcctgagcgccaagggcgacgtggctagagcccaaaacatcctagggcagttcagaagcggcgagttcaacgagttcgccgtggagaagagacacctgggcaacctggagagcctgtacaacatctggagcaagagcgacatggacaccggcatcgaggagtacagcagcatccacaaggacgagtacgaccgggaccccatcgtggacctgtacagacacatctacccccacagagaggtgatcagcgccaagaacttcatcgacgccgccgtgctgaacaagctgctgagactgaacgctagcagacacgtgcaccccaccgtgttcggcaagaccgtgatcagcttcagccccaagagcagcgcctacggcagaatcaccccccctagcgagatcgtgagaggcagacccgccggcagccacggcatgatctggctgaccatggagctgttcgacgacggcaagtggatcgagcaccacctgcccttccacaacagcagatactacgaagaggtgtactgctaccaagagggcctgcccgtgaaggacgagcctagaagccccatgttcggctacagagtgggcaacgccatcgccgacacaagcaagatcgacaacagacggagaaaggctagcaagcagttcctgagagctcagcagaacatcacccacaacgtgagcttcgacgagaacaccgccttcagcgtggtgagaaacggcgaggacttcagcatcaccatcagcagcagaatcaaggctagcaatgctaagagcctgatgaccatcggcgacagaatcatgggcatcgatcagaatcagaccgccgccaacacctacagcatctgggaggtggtgggcgacggcgacgccggcagcattcagcacggcaacctgagcctgaagagaatcgaggacggccacatcacaagcatcatcagaggcagaggcggcaacttcgatcagctgaactacggcggcctgagctacgccaagttcagcgagtggagaagcgctagactgggcttcatcagcagcctgaacgccgagctggctagcaagatgaactgggactggtgctgcctgtacgagtggaacgctagatacgctagcgccctgagaaagatcatctacagccacaagggcatcgacatcgagagagtgttcagaagagagatcgaggacttcgtggagggcgtgctgagaatcggcagcctgagcagcgacgccctgcagtgcctgaccaacgccaagagcctgatcagcagctacttcttcctgaacggcaagaaggagcccgaggagcagagaaagttcgaccaaggcctgttcgacctgagcgccaagattgacaagaagagagtgaacaagagacagcaaaagaccaagagaatcatgagcagcatcatgcagatcgctagagacagaggcgtgagcttcatcgtggtggagggcaagctgagcaccgccaccaaggacaacaagagcaaggccaatcagaaggccatcgactggtgcgctagagccgtggtggagaacctggagcacagctgcagcctggtgggcatcaagctggtggccatcgaccccatgaacacaagccacctggaccccttcgtgtacgtgctcaagacaagcctgggcaaggaggctagattcgctagcgtggtgcccgccaagatcaacgctagacacatgaagaacttcaagagctggagcagcctgctggccggcaacggcaagatcaaaaagaccaccgacgccatctacgtgggcgccttccaagacttctgcagagagtacggcttcgtggccgaggacatcagcaagatgagccaaagcgagatccaagacaagctgagcagccatcagttcgtgctggtgcctcagagaggcggcagagtgtacatgagcacccaccccgtgagcagcgaggccaagaagatcgtgtacgccggcagagagagatggtacaacaacgccgacgtggtggccgccgtgaacatcaccctgagaggctgcgagagactgagcgctagcagaaagaccgctagcacaagaacaggcggcggccccggcggcggcgccgccgccggcagcggcagccctaagaaaaaacgaaaagttggcagcggaagcaaaaggccggcggccacgaaaaaggccggccaggcaaaaaagaaaaagctcgagtacccatacgatgttccagattacgcttgagaattccccttgagcatctgacttctggctaataaaggaaatttattttcattgcaatagtgtgttggaattttttgtgtctctcaggtaccaaaaacggctcggagatcatcattgcgccgtcaacttaggacgggtttctgagatgttgcgatcggtgtttcgtcctttccacaagatatataaagccaagaaatcgaaatactttcaagttacggtaagcatatgatagtccattttaaaacataattttaaaactgcaaactacccaagaaattattactttctacgtcacgtattttgtactaatatctttgtgtttacagtcaaattaattccaattatctctctaacagccttgtatcgtatatgcaaatatgaaggaatcatgggaaataggccctctagagggcccgtttaaacccgctgatcagcctcgactgtgccttctagttgccagccatctgttgtttgcccctcccccgtgccttccttgaccctggaaggtgccactcccactgtcctttcctaataaaatgaggaaattgcatcgcattgtctgagtaggtgtcattctattctggggggtggggtggggcaggacagcaagggggaggattgggaagacaatagcaggcatgctggggatgcggtgggctctatggcttctgaggcggaaagaaccagctggggctctagggggtatccccacgcgccctgtagcggcgcattaagcgcggcgggtgtggtggttacgcgcagcgtgaccgctacacttgccagcgccctagcgcccgctcctttcgctttcttcccttcctttctcgccacgttcgccggctttccccgtcaagctctaaatcgggggctccctttagggttccgatttagtgctttacggcacctcgaccccaaaaaacttgattagggtgatggttcacgtagtgggccatcgccctgatagacggtttttcgccctttgacgttggagtccacgttctttaatagtggactcttgttccaaactggaacaacactcaaccctatctcggtctattcttttgatttataagggattttgccgatttcggcctattggttaaaaaatgagctgatttaacaaaaatttaacgcgaattaattctgtggaatgtgtgtcagttagggtgtggaaagtccccaggctccccagcaggcagaagtatgcaaagcatgcatctcaattagtcagcaaccaggtgtggaaagtccccaggctccccagcaggcagaagtatgcaaagcatgcatctcaattagtcagcaaccatagtcccgcccctaactccgcccatcccgcccctaactccgcccagttccgcccattctccgccccatggctgactaattttttttatttatgcagaggccgaggccgcctctgcctctgagctattccagaagtagtgaggaggcttttttggaggcctaggcttttgcaaaaagctcccgggagcttgtatatccattttcggatctgatcaagagacaggatgaggatcgtttcgcatgattgaacaagatggattgcacgcaggttctccggccgcttgggtggagaggctattcggctatgactgggcacaacagacaatcggctgctctgatgccgccgtgttccggctgtcagcgcaggggcgcccggttctttttgtcaagaccgacctgtccggtgccctgaatgaactgcaggacgaggcagcgcggctatcgtggctggccacgacgggcgttccttgcgcagctgtgctcgacgttgtcactgaagcgggaagggactggctgctattgggcgaagtgccggggcaggatctcctgtcatctcaccttgctcctgccgagaaagtatccatcatggctgatgcaatgcggcggctgcatacgcttgatccggctacctgcccattcgaccaccaagcgaaacatcgcatcgagcgagcacgtactcggatggaagccggtcttgtcgatcaggatgatctggacgaagagcatcaggggctcgcgccagccgaactgttcgccaggctcaaggcgcgcatgcccgacggcgaggatctcgtcgtgacccatggcgatgcctgcttgccgaatatcatggtggaaaatggccgcttttctggattcatcgactgtggccggctgggtgtggcggaccgctatcaggacatagcgttggctacccgtgatattgctgaagagcttggcggcgaatgggctgaccgcttcctcgtgctttacggtatcgccgctcccgattcgcagcgcatcgccttctatcgccttcttgacgagttcttctgagcgggactctggggttcgaaatgaccgaccaagcgacgcccaacctgccatcacgagatttcgattccaccgccgccttctatgaaaggttgggcttcggaatcgttttccgggacgccggctggatgatcctccagcgcggggatctcatgctggagttcttcgcccaccccaacttgtttattgcagcttataatggttacaaataaagcaatagcatcacaaatttcacaaataaagcatttttttcactgcattctagttgtggtttgtccaaactcatcaatgtatcttatcatgtctgtataccgtcgacctctagctagagcttggcgtaatcatggtcatagctgtttcctgtgtgaaattgttatccgctcacaattccacacaacatacgagccggaagcataaagtgtaaagcctggggtgcctaatgagtgagctaactcacattaattgcgttgcgctcactgcccgctttccagtcgggaaacctgtcgtgccagctgcattaatgaatcggccaacgcgcggggagaggcggtttgcgtattgggcgctcttccgcttcctcgctcactgactcgctgcgctcggtcgttcggctgcggcgagcggtatcagctcactcaaaggcggtaatacggttatccacagaatcaggggataacgcaggaaagaacatgtgagcaaaaggccagcaaaaggccaggaaccgtaaaaaggccgcgttgctggcgtttttccataggctccgcccccctgacgagcatcacaaaaatcgacgctcaagtcagaggtggcgaaacccgacaggactataaagataccaggcgtttccccctggaagctccctcgtgcgctctcctgttccgaccctgccgcttaccggatacctgtccgcctttctcccttcgggaagcgtggcgctttctcatagctcacgctgtaggtatctcagttcggtgtaggtcgttcgctccaagctgggctgtgtgcacgaaccccccgttcagcccgaccgctgcgccttatccggtaactatcgtcttgagtccaacccggtaagacacgacttatcgccactggcagcagccactggtaacaggattagcagagcgaggtatgtaggcggtgctacagagttcttgaagtggtggcctaactacggctacactagaagaacagtatttggtatctgcgctctgctgaagccagttaccttcggaaaaagagttggtagctcttgatccggcaaacaaaccaccgctggtagcggtttttttgtttgcaagcagcagattacgcgcagaaaaaaaggatctcaagaagatcctttgatcttttctacggggtctgacgctcagtggaacgaaaactcacgttaagggattttggtcatgagattatcaaaaaggatcttcacctagatccttttaaattaaaaatgaagttttaaatcaatctaaagtatatatgagtaaacttggtctgacagttaccaatgcttaatcagtgaggcacctatctcagcgatctgtctatttcgttcatccatagttgcctgactccccgtcgtgtagataactacgatacgggagggcttaccatctggccccagtgctgcaatgataccgcgagacccacgctcaccggctccagatttatcagcaataaaccagccagccggaagggccgagcgcagaagtggtcctgcaactttatccgcctccatccagtctattaattgttgccgggaagctagagtaagtagttcgccagttaatagtttgcgcaacgttgttgccattgctacaggcatcgtggtgtcacgctcgtcgtttggtatggcttcattcagctccggttcccaacgatcaaggcgagttacatgatcccccatgttgtgcaaaaaagcggttagctccttcggtcctccgatcgttgtcagaagtaagttggccgcagtgttatcactcatggttatggcagcactgcataattctcttactgtcatgccatccgtaagatgcttttctgtgactggtgagtactcaaccaagtcattctgagaatagtgtatgcggcgaccgagttgctcttgcccggcgtcaatacgggataataccgcgccacatagcagaactttaaaagtgctcatcattggaaaacgttcttcggggcgaaaactctcaaggatcttaccgctgttgagatccagttcgatgtaacccactcgtgcacccaactgatcttcagcatcttttactttcaccagcgtttctgggtgagcaaaaacaggaaggcaaaatgccgcaaaaaagggaataagggcgacacggaaatgttgaatactcatactcttcctttttcaatattattgaagcatttatcagggttattgtctcatgagcggatacatatttgaatgtatttagaaaaataaacaaataggggttccgcgcacatttccccgaaaagtgccacctgacgtc

SEQ ID NO: 738 - protein, 7 aa, synthetic construct
PKKKRKV

SEQ ID NO: 739 - protein, 16 aa, synthetic construct
KRPAATKKAGQAKKKK

SEQ ID NO: 740 - protein, 9 aa, synthetic construct
PAAKRVKLD

SEQ ID NO: 741 - protein, 11 aa, synthetic construct
RQRRNELKRSP

SEQ ID NO: 742 - protein, 38 aa, synthetic construct
NQSSNFGPMKGGNFGGRSSGPYGGGGQYFAKPRNQGGY

SEQ ID NO: 743 - protein, 42 aa, synthetic construct
RMRIZFKNKGKDTAELRRRRVEVSVELRKAKKDEQILKRRNV

SEQ ID NO: 744 - protein, 8 aa, synthetic construct
VSRKRPRP

SEQ ID NO: 745 - protein, 8 aa, synthetic construct
PPKKARED

SEQ ID NO: 746 - protein, 8 aa, synthetic construct
PQPKKKPL

SEQ ID NO: 747 - protein, 12 aa, synthetic construct
SALIKKKKKMAP

SEQ ID NO: 748 - protein, 5 aa, synthetic construct
DRLRR

SEQ ID NO: 749 - protein, 7 aa, synthetic construct
PKQKKRK

SEQ ID NO: 750 - protein, 10 aa, synthetic construct
RKLKKKIKKL

SEQ ID NO: 751 - protein, 10 aa, synthetic construct
REKKKFLKRR

SEQ ID NO: 752 - protein, 20 aa, synthetic construct
KRKGDEVDGVDEVAKKKSKK

SEQ ID NO: 753 - protein, 17 aa, synthetic construct
RKCLQAGMNLEARKTKK

SEQ ID NO: 754 - DNA, 38 bp, synthetic construct
  source 1..38: mol_type = other DNA
gtaccgaaaaacatcattgcgtcgcgaggtgaggcgtc

SEQ ID NO: 755 - DNA, 38 bp, synthetic construct
  source 1..38: mol_type = other DNA
cattgacgcctcacctcgcgacgcaatgatgtttttcg

SEQ ID NO: 756 - DNA, 28 bp, synthetic construct
  source 1..28: mol_type = other DNA
gagttcaagagaggcttcgacagagagc

SEQ ID NO: 757 - DNA, 30 bp, synthetic construct
  source 1..30: mol_type = other DNA
tcgaagcctctcttgaactcggcgcagtag

SEQ ID NO: 758 - DNA, 26 bp, synthetic construct
  source 1..26: mol_type = other DNA
aaccaggagacagaacaagggcgagg

SEQ ID NO: 759 - DNA, 34 bp, synthetic construct
  source 1..34: mol_type = other DNA
ccttgttctgtctcctggtttccagcttgttcag

SEQ ID NO: 760 - protein, 1139 aa, synthetic construct
RFVVLSVNQFRCNPNAFRQASMKTDDEKKDTAIKSYTSWLLPNDRKEKDMVRSFLALDQGSRFFFDLMQAWYGGLTPDIIKSVTKERDLVDLWCAIYWFRPMKKELASHPIDRVDLAKTFQRYYGGPASDVVQEYLSASIGEDCCWNDCRQKYQEFCKNLGVDFTPDLKTLVREKLIAVALNDGSRAAISNLFGNGGKEDRNVKVNICKKILIALEKAGKSVKYVRDVQSIILKCANAKDREDFNRIYADKNGRPGTLLLLLDRKGENTYDAEVLKRYLRKTIKSKNAPLVWNYNQKLFEYIERGIRNLLRRTINYDAWAWGEMWRVGHTPLQTKATRNYHFAQEQLKRHSRIAAASQSSHAIAVALNEFFESPFFDGENPFTICPHHLGKNLEKLFKAWADEKNQTDEEDAGETAITDYCAEFKRGFDREPIRNLLRYVYASLRSKYSAKELIQAAKYNQQFERYQRQKAHPVTPDNQGYTWPEAVIKPSKAERKNRENSLDTRIWVSVKLLQKDGTWEKHHIPFYNLRFFEEVYAAASIAEDMPSPTFRNSRFGFKLPKLLNTHAKINKKKKDGKKDKKAVNAAKREARIYLAAKEGRLPAPSVPLDKLSAVIARVNGKFQVTVPVKFKVNKQPKYPLPQLGQIILGYDQNLTANHAWALFEVVTEDTPGAHFCRNQYLRVLKTGQVRSITKTKDGQEIDQLSYDGLEYKEYGEWRKQAKKFASQWYITTKVRKGKETTLLSQPALERFESIEKYKPALYRFNKEYARLLLAVIRRKTLNELEEIRPEIFRLVEQGFGICRFGSLSLSSFEAIRAAKAVIYGYFSTALKHDHNTPITDDERQARDPELFGLLNKLRTRRQNKGEEKINRAANALIRIALENKADFIRGEGDLPTTNKSVKKGQNSRSMDWLARGLFNKICQLAVMHNIIPTAANPHSTSHQDPFEHNKDFDDPQPAMKCRYAEFKIEDIGDSVLERLGTSLRNAKAGQTGAYYYKGAQDFLAHYGLQDIEEELKKCRRGRKANMPCWELQKRLIQKLGSKDAVVYIPMRGGRIYLATHSVTTGAKPIIFNGEEVWVSNADEIAAVNIGLTIIPTSKKDEEHPDRENDDKAIRKSVRRPRKSGERRSGDKMPATARKT

SEQ ID NO: 761 - DNA, 23 bp, synthetic construct
  source 1..23: mol_type = other DNA
tcctataaggtgtgaaagtctgg

SEQ ID NO: 762 - DNA, 20 bp, synthetic construct
  source 1..20: mol_type = other DNA
cagtaagatttggtgtctat

SEQ ID NO: 763 - DNA, 23 bp, synthetic construct
  source 1..23: mol_type = other DNA
tatatcccttctacaaattcctc

SEQ ID NO: 764 - DNA, 24 bp, synthetic construct
  source 1..24: mol_type = other DNA
gtgtctgaggctggccctacggtg

SEQ ID NO: 765 - DNA, 23 bp, synthetic construct
  source 1..23: mol_type = other DNA
agaaaggctgctgatgacacctg

SEQ ID NO: 766 - DNA, 24 bp, synthetic construct
  source 1..24: mol_type = other DNA
gcatctccccattccatgagcatg

SEQ ID NO: 767 - DNA, 22 bp, synthetic construct
  source 1..22: mol_type = other DNA
acagccaacgactccggccccg

SEQ ID NO: 768 - DNA, 23 bp, synthetic construct
  source 1..23: mol_type = other DNA
tagaagggatatacaaagtggaa

SEQ ID NO: 769 - DNA, 24 bp, synthetic construct
  source 1..24: mol_type = other DNA
tagatgctgtccgaggcagtcctg

SEQ ID NO: 770 - DNA, 23 bp, synthetic construct
  source 1..23: mol_type = other DNA
ggtgtctatttccactttgtata

SEQ ID NO: 771 - DNA, 24 bp, synthetic construct
  source 1..24: mol_type = other DNA
ctgaacacatgcacggccacattg

SEQ ID NO: 772 - DNA, 23 bp, synthetic construct
  source 1..23: mol_type = other DNA
cccagaggcaaatggctcccagg

SEQ ID NO: 773 - DNA, 23 bp, synthetic construct
  source 1..23: mol_type = other DNA
ctcctcagttgtgagcccatgca

SEQ ID NO: 774 - DNA, 23 bp, synthetic construct
  source 1..23: mol_type = other DNA
gccagccttgccttgaccaatag

SEQ ID NO: 775 - DNA, 23 bp, synthetic construct
  source 1..23: mol_type = other DNA
accaatagtcttagagtatccag

SEQ ID NO: 776 - DNA, 23 bp, synthetic construct
  source 1..23: mol_type = other DNA
ccttgtcaaggctattggtcaag

SEQ ID NO: 777 - DNA, 23 bp, synthetic construct
  source 1..23: mol_type = other DNA
ccttgaccaatagccttgacaag

SEQ ID NO: 778 - DNA, 23 bp, synthetic construct
  source 1..23: mol_type = other DNA
accaatagccttgacaaggcaaa

SEQ ID NO: 779 - DNA, 23 bp, synthetic construct
  source 1..23: mol_type = other DNA
gtcaaggcaaggctggccaaccc

SEQ ID NO: 780 - DNA, 21 bp, synthetic construct
  source 1..21: mol_type = other DNA
gtcaagtttgcctgtcaaggc

SEQ ID NO: 781 - DNA, 23 bp, synthetic construct
  source 1..23: mol_type = other DNA
tcaaggctattggtcaaggcaag

SEQ ID NO: 782 - DNA, 24 bp, synthetic construct
  source 1..24: mol_type = other DNA
acaaggcaaacttgaccaatagtc

SEQ ID NO: 783 - RNA, 45 nt, synthetic construct
  source 1..45: mol_type = other RNA
gtaatgcgtctcccattgacgccatgagcatgcagaggtgagtat

SEQ ID NO: 784 - RNA, 45 nt, synthetic construct
  source 1..45: mol_type = other RNA
gtaatgcgtctcccattgacgctcctataaggtgtgaaagtctgg

SEQ ID NO: 785 - RNA, 42 nt, synthetic construct
  source 1..42: mol_type = other RNA
gtaatgcgtctcccattgacgccagtaagatttggtgtctat

SEQ ID NO: 786 - RNA, 45 nt, synthetic construct
  source 1..45: mol_type = other RNA
gtaatgcgtctcccattgacgctatatcccttctacaaattcctc

SEQ ID NO: 787 - RNA, 46 nt, synthetic construct
  source 1..46: mol_type = other RNA
gtaatgcgtctcccattgacgcgtgtctgaggctggccctacggtg

SEQ ID NO: 788 - RNA, 45 nt, synthetic construct
  source 1..45: mol_type = other RNA
gtaatgcgtctcccattgacgcagaaaggctgctgatgacacctg

SEQ ID NO: 789 - RNA, 46 nt, synthetic construct
  source 1..46: mol_type = other RNA
gtaatgcgtctcccattgacgcgcatctccccattccatgagcatg

SEQ ID NO: 790 - RNA, 45 nt, synthetic construct
  source 1..45: mol_type = other RNA
gtaatgcgtctcccattgacgcacagccaacgactccggcccccg

SEQ ID NO: 791 - RNA, 45 nt, synthetic construct
  source 1..45: mol_type = other RNA
gtaatgcgtctcccattgacgctagaagggatatacaaagtggaa

SEQ ID NO: 792 - RNA, 46 nt, synthetic construct
  source 1..46: mol_type = other RNA
gtaatgcgtctcccattgacgctagatgctgtccgaggcagtcctg

SEQ ID NO: 793 - RNA, 45 nt, synthetic construct
  source 1..45: mol_type = other RNA
gtaatgcgtctcccattgacgcggtgtctatttccactttgtata

SEQ ID NO: 794 - RNA, 46 nt, synthetic construct
  source 1..46: mol_type = other RNA
gtaatgcgtctcccattgacgcctgaacacatgcacggccacattg

SEQ ID NO: 795 - RNA, 45 nt, synthetic construct
  source 1..45: mol_type = other RNA
gtaatgcgtctcccattgacgccccagaggcaaatggctcccagg

SEQ ID NO: 796 - RNA, 45 nt, synthetic construct
  source 1..45: mol_type = other RNA
gtaatgcgtctcccattgacgcctcctcagttgtgagcccatgca

SEQ ID NO: 797 - RNA, 45 nt, synthetic construct
  source 1..45: mol_type = other RNA
gtaatgcgtctcccattgacgcgccagccttgccttgaccaatag

SEQ ID NO: 798 - RNA, 45 nt, synthetic construct
  source 1..45: mol_type = other RNA
gtaatgcgtctcccattgacgcaccaatagtcttagagtatccag

SEQ ID NO: 799 - RNA, 45 nt, synthetic construct
  source 1..45: mol_type = other RNA
gtaatgcgtctcccattgacgcccttgtcaaggctattggtcaag

SEQ ID NO: 800 - RNA, 45 nt, synthetic construct
  source 1..45: mol_type = other RNA
gtaatgcgtctcccattgacgcccttgaccaatagccttgacaag

SEQ ID NO: 801 - RNA, 45 nt, synthetic construct
  source 1..45: mol_type = other RNA
gtaatgcgtctcccattgacgcaccaatagccttgacaaggcaaa

SEQ ID NO: 802 - RNA, 45 nt, synthetic construct
  source 1..45: mol_type = other RNA
gtaatgcgtctcccattgacgcgtcaaggcaaggctggccaaccc

SEQ ID NO: 803 - RNA, 44 nt, synthetic construct
  source 1..44: mol_type = other RNA
gtaatgcgtctcccattgacgcgtcaagtttgccttgtcaaggc

SEQ ID NO: 804 - RNA, 45 nt, synthetic construct
  source 1..45: mol_type = other RNA
gtaatgcgtctcccattgacgctcaaggctattggtcaaggcaag

SEQ ID NO: 805 - RNA, 46 nt, synthetic construct
  source 1..46: mol_type = other RNA
gtaatgcgtctcccattgacgcacaaggcaaacttgaccaatagtc

SEQ ID NO: 806 - DNA, 25 bp, synthetic construct
  source 1..25: mol_type = other DNA
gaacgaatgttccgatgctctaatc

SEQ ID NO: 807 - DNA, 28 bp, synthetic construct
  source 1..28: mol_type = other DNA
aatgaggtagaatgctcagagttcaagt

SEQ ID NO: 808 - DNA, 26 bp, synthetic construct
  source 1..26: mol_type = other DNA
caactgttctcaggggacctattttc

SEQ ID NO: 809 - DNA, 26 bp, synthetic construct
  source 1..26: mol_type = other DNA
ctctactgtctgcccctaaatgatgc

SEQ ID NO: 810 - DNA, 28 bp, synthetic construct
  source 1..28: mol_type = other DNA
tgccatttaatttcagttaggagttttc

SEQ ID NO: 811 - DNA, 23 bp, synthetic construct
  source 1..23: mol_type = other DNA
cagacctccgagaagccagatgt

SEQ ID NO: 812 - DNA, 27 bp, synthetic construct
  source 1..27: mol_type = other DNA
caagacctgactctgtactcctgctct

SEQ ID NO: 813 - DNA, 25 bp, synthetic construct
  source 1..25: mol_type = other DNA
atttggatctctcctagcgttctgc

SEQ ID NO: 814 - DNA, 23 bp, synthetic construct
  source 1..23: mol_type = other DNA
acggctgacaaaagaagtcctgg

SEQ ID NO: 815 - DNA, 22 bp, synthetic construct
  source 1..22: mol_type = other DNA
catgggtagacaaccaggagcc

SEQ ID NO: 816 - protein, 1139 aa, synthetic construct
RFVVLSVNQFRCNPNAFRQASMKTDDEKKDTAIKSYTSWLLPNDRKEKDMVRSFLALDQGSRFFFDLMQAWYGGLTPDIIKSVTKERDLVDLWCAIYWFRPMKKELASHPIDRVDLAKTFQRYYGGPASDVVQEYLSASIGEDCCWNDCRQKYQEFCKNLGVDFTPDLKTLVREKLIAVALNDGSRAAISNLFGNGGKEDRNVKVNICKKILIALEKAGKSVKYVRDVQSIILKCANAKDREDFNRIYADKNGRPGTLLLLLDRKGENTYDAEVLKRYLRKTIKSKNAPLVWNYNQKLFEYIERGIRNLLRRTINYDAWAWGEMWRVGHTPLQTKATRNYHFAQEQLKRHSRIAAASQSSHAIAVALNEFFESPFFDGENPFTICPHHLGKNLEKLFKAWADEKNQTDEEDAGETAITDYCAEFKRGFDREPIRNLLRYVYASLRSKYSAKELIQAAKYNQQFERYQRQKAHPVTPDNQGYTWPEAVIKPSKAERKNRENSLDTRIWVSVKLLQKDGTWEKHHIPFYNLRFFEEVYAAASIAEDMPSPTFRNSRFGFKLPKLLNTHAKINKKKKDGKKDKKAVNAAKREARIYLAAKEGRLPAPSVPLDKLSAVIARVNGKFQVTVPVKFKVNKQPKYPLPQLGQIILGYAQNLTANHAWALFEVVTEDTPGAHFCRNQYLRVLKTGQVRSITKTKDGQEIDQLSYDGLEYKEYGEWRKQAKKFASQWYITTKVRKGKETTLLSQPALERFESIEKYKPALYRFNKEYARLLLAVIRRKTLNELEEIRPEIFRLVEQGFGICRFGSLSLSSFEAIRAAKAVIYGYFSTALKHDHNTPITDDERQARDPELFGLLNKLRTRRQNKGEEKINRAANALIRIALENKADFIRGAGDLPTTNKSVKKGQNSRSMDWLARGLFNKICQLAVMHNIIPTAANPHSTSHQDPFEHNKDFDDPQPAMKCRYAEFKIEDIGDSVLERLGTSLRNAKAGQTGAYYYKGAQDFLAHYGLQDIEEELKKCRRGRKANMPCWELQKRLIQKLGSKDAVVYIPMRGGRIYLATHSVTTGAKPIIFNGEEVWVSNAAEIAAVNIGLTIIPTSKKDEEHPDRENDDKAIRKSVRRPRKSGERRSGDKMPATARKT

SEQ ID NO: 817 - RNA, 70 nt, synthetic construct
  source 1..70: mol_type = other RNA
atgtgtttttgtcaaaagaccttttgtaatgcgtctcccattgacgccatgagcatgcagaggtgagtat

SEQ ID NO: 818 - RNA, 45 nt, synthetic construct; identical to SEQ ID NO: 783
  source 1..45: mol_type = other RNA

SEQ ID NO: 819 - RNA, 59 nt, synthetic construct
  source 1..59: mol_type = other RNA
gttgcaatcccaaggtaatgcgtctcccattgacgccatgagcatgcagaggtgagtat

SEQ ID NO: 820 - RNA, 45 nt, synthetic construct; identical to SEQ ID NO: 783
  source 1..45: mol_type = other RNA

SEQ ID NO: 821 - RNA, 25 nt, synthetic construct
  source 1..25: mol_type = other RNA
atgtgtttttgtcaaaagacctttt

SEQ ID NO: 822 - RNA, 14 nt, synthetic construct
  source 1..14: mol_type = other RNA
gttgcaatcccaag

SEQ ID NO: 823 - DNA, 29 bp, synthetic construct
  source 1..29: mol_type = other DNA
gcgtaacttaatccagactttcacacctt

SEQ ID NO: 824 - DNA, 26 bp, synthetic construct
  source 1..26: mol_type = other DNA
ggtcattcatcaccttccttaggaca

SEQ ID NO: 825 - RNA, 23 nt, synthetic construct
  source 1..23: mol_type = other RNA
ctggagcctgtgataaaagcaac

SEQ ID NO: 826 - RNA, 23 nt, synthetic construct
  source 1..23: mol_type = other RNA
aagctaacagttgcttttatcac

SEQ ID NO: 827 - RNA, 23 nt, synthetic construct
  source 1..23: mol_type = other RNA
cattgagatagtgtggggaaggg

SEQ ID NO: 828 - RNA, 23 nt, synthetic construct
  source 1..23: mol_type = other RNA
gcattgagatagtgtggggaagg

SEQ ID NO: 829 - RNA, 23 nt, synthetic construct
  source 1..23: mol_type = other RNA
agatagtgtggggaaggggcccc

SEQ ID NO: 830 - RNA, 23 nt, synthetic construct
  source 1..23: mol_type = other RNA
ggggccccttccccacactatct

SEQ ID NO: 831 - RNA, 23 nt, synthetic construct
  source 1..23: mol_type = other RNA
cctcttgggggccccttccccac

SEQ ID NO: 832 - RNA, 23 nt, synthetic construct
  source 1..23: mol_type = other RNA
tcctcttgggggccccttcccca

SEQ ID NO: 833 - RNA, 23 nt, synthetic construct
  source 1..23: mol_type = other RNA
gcagtatcctcttgggggcccct

SEQ ID NO: 834 - RNA, 23 nt, synthetic construct
  source 1..23: mol_type = other RNA
cccacactatctcaatgcaaata

SEQ ID NO: 835 - RNA, 23 nt, synthetic construct
  source 1..23: mol_type = other RNA
cagacagatatttgcattgagat

SEQ ID NO: 836 - RNA, 23 nt, synthetic construct
  source 1..23: mol_type = other RNA
agccagggaccgtttcagacaga

SEQ ID NO: 837 - RNA, 23 nt, synthetic construct
  source 1..23: mol_type = other RNA
acaaggcaaacttgaccaatagt

SEQ ID NO: 838 - RNA, 23 nt, synthetic construct
  source 1..23: mol_type = other RNA
atccctagccagccgccggcccc

SEQ ID NO: 839 - RNA, 23 nt, synthetic construct
  source 1..23: mol_type = other RNA
tagggtaccctcgtgcacccggg

SEQ ID NO: 840 - RNA, 23 nt, synthetic construct
  source 1..23: mol_type = other RNA
cgcggcagccactcgctggtatc

SEQ ID NO: 841 - RNA, 23 nt, synthetic construct
  source 1..23: mol_type = other RNA
gtccttgaggacagacaccactg

SEQ ID NO: 842 - RNA, 23 nt, synthetic construct
  source 1..23: mol_type = other RNA
atccttgttttccagtggtgtct

SEQ ID NO: 843 - RNA, 23 nt, synthetic construct
  source 1..23: mol_type = other RNA
gaagagttgaccatcagttatgg

SEQ ID NO: 844 - RNA, 23 nt, synthetic construct
  source 1..23: mol_type = other RNA
ctctactcctcaagaaaacacca

SEQ ID NO: 845 - RNA, 23 nt, synthetic construct
  source 1..23: mol_type = other RNA
acacagaaccctgccattctaaa

SEQ ID NO: 846 - RNA, 23 nt, synthetic construct
  source 1..23: mol_type = other RNA
agtctgcacaacaaaaacaagca

SEQ ID NO: 847 - RNA, 23 nt, synthetic construct
  source 1..23: mol_type = other RNA
gggtgataggtgcagatggtccg

SEQ ID NO: 848 - RNA, 23 nt, synthetic construct
  source 1..23: mol_type = other RNA
cccaacagttggtataaattgtg

SEQ ID NO: 849 - RNA, 23 nt, synthetic construct
  source 1..23: mol_type = other RNA
cagtctgcacaacaaaaacaagc

SEQ ID NO: 850 - RNA, 23 nt, synthetic construct
  source 1..23: mol_type = other RNA
aggtggtcccttagtttgcaaac

SEQ ID NO: 851 - RNA, 23 nt, synthetic construct
  source 1..23: mol_type = other RNA
ggggtgtacatggaagctacatc

SEQ ID NO: 852 - RNA, 23 nt, synthetic construct
  source 1..23: mol_type = other RNA
cctattaaagtacagtcccggag

SEQ ID NO: 853 - RNA, 23 nt, synthetic construct
  source 1..23: mol_type = other RNA
tagcggtaggtgttcctccggga

SEQ ID NO: 854 - RNA, 23 nt, synthetic construct
  source 1..23: mol_type = other RNA
cgtgctcgggtgcttcggccagg

SEQ ID NO: 855 - RNA, 23 nt, synthetic construct
  source 1..23: mol_type = other RNA
cccctccacggtaccgggcggat

SEQ ID NO: 856 - RNA, 23 nt, synthetic construct
  source 1..23: mol_type = other RNA
atccgcccggtaccgtggagggg

SEQ ID NO: 857 - RNA, 23 nt, synthetic construct
  source 1..23: mol_type = other RNA
gcagttgagcacgcgcaggctgc

SEQ ID NO: 858 - RNA, 23 nt, synthetic construct
  source 1..23: mol_type = other RNA
gccacgccggcatcccggccgct

SEQ ID NO: 859 - RNA, 23 nt, synthetic construct
  source 1..23: mol_type = other RNA
aggacgcggctgtacccacccgc

SEQ ID NO: 860 - RNA, 23 nt, synthetic construct
  source 1..23: mol_type = other RNA
ggccgctgtgtggacctctttgc

SEQ ID NO: 861 - RNA, 23 nt, synthetic construct
  source 1..23: mol_type = other RNA
tctacggcgtaggcccccaggac

SEQ ID NO: 862 - RNA, 23 nt, synthetic construct
  source 1..23: mol_type = other RNA
cccaagtctccaacatgcctaat

SEQ ID NO: 863 - RNA, 23 nt, synthetic construct
  source 1..23: mol_type = other RNA
cccacaccttcactggtccatta

SEQ ID NO: 864 - RNA, 23 nt, synthetic construct
  source 1..23: mol_type = other RNA
atgcttccccacaccttcactgg

SEQ ID NO: 865 - RNA, 23 nt, synthetic construct
  source 1..23: mol_type = other RNA
agcatcttgttacctctcttcat

SEQ ID NO: 866 - RNA, 23 nt, synthetic construct
  source 1..23: mol_type = other RNA
ggcaatgtgactgctgacaaaga

SEQ ID NO: 867 - RNA, 23 nt, synthetic construct
  source 1..23: mol_type = other RNA
agcacgcacacggccttcgtcgc

SEQ ID NO: 868 - RNA, 23 nt, synthetic construct
  source 1..23: mol_type = other RNA
aaggactgactgaaggcctgcat

SEQ ID NO: 869 - RNA, 23 nt, synthetic construct
  source 1..23: mol_type = other RNA
agggggaagccagcaccacaaag

SEQ ID NO: 870 - RNA, 23 nt, synthetic construct
  source 1..23: mol_type = other RNA
cctcttagtacaactatgacaag

SEQ ID NO: 871 - RNA, 23 nt, synthetic construct
  source 1..23: mol_type = other RNA
ccagtcatctcactctacctaat

SEQ ID NO: 872 - RNA, 23 nt, synthetic construct
  source 1..23: mol_type = other RNA
ccctctccccagtgcacgatgag

SEQ ID NO: 873 - RNA, 23 nt, synthetic construct
  source 1..23: mol_type = other RNA
agcagggagatgtcatcagcaaa

SEQ ID NO: 874 - RNA, 23 nt, synthetic construct
  source 1..23: mol_type = other RNA
ggtagagtgagatgactgggaaa

SEQ ID NO: 875 - RNA, 23 nt, synthetic construct
  source 1..23: mol_type = other RNA
cccctcaaccagtctgaagtgct

SEQ ID NO: 876 - RNA, 23 nt, synthetic construct
  source 1..23: mol_type = other RNA
agatcctgtccattgatctccac

SEQ ID NO: 877 - RNA, 23 nt, synthetic construct
  source 1..23: mol_type = other RNA
gcacgcacagtgacgttggggcc

SEQ ID NO: 878 - DNA, 65 bp, synthetic construct
  source 1..65: mol_type = other DNA
ccatggaacggctcggagatcatcattgcgnnnnnnngtgagcaagggcgaggagctgttcaccg

SEQ ID NO: 879 - DNA, 67 bp, synthetic construct
  source 1..67: mol_type = other DNA
ggtaccttgccgagcctctctagtagtaacgcnnnnnnncactcgttcccgctcctcgacaagtggc

SEQ ID NO: 880 - DNA, 24 bp, synthetic construct
  source 1..24: mol_type = other DNA
gtgagcaagggcgaggagctgttc

SEQ ID NO: 881 - DNA, 26 bp, synthetic construct
  source 1..26: mol_type = other DNA
ccttgccgagcctctagtagtaacgc

SEQ ID NO: 882 - DNA, 272 bp, synthetic construct
  source 1..272: mol_type = other DNA
ttattattttaaaaaacagcacaaaaggaaactcaccctaactgtaaagtaattgtgtgttttgagactataaatatgcatgcgagaaaagccttgtttgccaccatggaacggctcggagatcatcattgcgnnnnnnnaccgagtacaagcccacggtgcgcctcgccacccgcgcgacgacgtccccagggccgtacgcaccctcgccgccgcgttcgccgactaccccgccacgcgccacaccgtcgatccggaccgccacatcgagc

SEQ ID NO: 883 - DNA, 269 bp, synthetic construct
  source 1..269: mol_type = other DNA
aataataaaattttttgtcgtgttttcctttgagtgggattgacatttcattaacacacaaaactctgatatttatacgtacgctcttttcggaacaaacggtggtaccttgccgagcctctagtagtaacgcnnnnnntggctcatgttcgggtgccacgcggagcggtgggcgctgctgcaggggtcccggcatgcgtgggagcggcggcgcaagcggctgatggggcggtgcgcggtgtggcagctaggcctggcggtgtagctcg

SEQ ID NO: 884 - protein, 43 aa, synthetic construct
TEYKPTVRLATRDDVPRAVRTLAAAFADYPATRHTVDPDRHIE

SEQ ID NO: 885 - protein, 55 aa, synthetic construct
MERLGDHHCXXXPSTSPRCASPPATTSPGPYAPSPPRSPTTPPRATPSIRTATSS

SEQ ID NO: 886 - DNA, 20 bp, synthetic construct
  source 1..20: mol_type = other DNA
gatggggcggtgcgcggtgt

SEQ ID NO: 887 - DNA, 60 bp, synthetic construct
  source 1..60: mol_type = other DNA
ctccccattccatgagcatgcagaggtgagtatacagaccttcgagggttgttttggttt

SEQ ID NO: 888 - DNA, 60 bp, synthetic construct
  source 1..60: mol_type = other DNA
ctccccagtccatgagcatgcagaggtgagtatacagaccttcgagggttgttttggttt

SEQ ID NO: 889 - DNA, 46 bp, synthetic construct
  source 1..46: mol_type = other DNA
ctccccattccatgagcatgcagaccttcgagggttgttttggttt

SEQ ID NO: 890 - DNA, 55 bp, synthetic construct
  source 1..55: mol_type = other DNA
ctccccattccatgagcatgcagaggtgacagaccttcgagggttgttttggttt

SEQ ID NO: 891 - DNA, 58 bp, synthetic construct
  source 1..58: mol_type = other DNA
ctccccattccatgagcatgcagaggtgagtacagaccttcgagggttgttttggttt

SEQ ID NO: 892 - DNA, 50 bp, synthetic construct
  source 1..50: mol_type = other DNA
ctccccattccatgagcatgcagacagaccttcgagggttgttttggttt

SEQ ID NO: 893 - DNA, 51 bp, synthetic construct
  source 1..51: mol_type = other DNA
ctccccattccatgagcatgcagaggtgaccttcgagggttgttttggttt

SEQ ID NO: 894 - DNA, 54 bp, synthetic construct
  source 1..54: mol_type = other DNA
ctccccattccatgagcatgcagaggtgcagaccttcgagggttgttttggttt

SEQ ID NO: 895 - DNA, 58 bp, synthetic construct
  source 1..58: mol_type = other DNA
ctccccattccatgagcatgcagaggtgagtatagaccttcgagggttgttttggttt

SEQ ID NO: 896 - DNA, 56 bp, synthetic construct
  source 1..56: mol_type = other DNA
ctccccattccatgagcatgcagaggtgagtagaccttcgagggttgttttggttt

SEQ ID NO: 897 - DNA, 53 bp, synthetic construct
  source 1..53: mol_type = other DNA
ctccccattccatgagcatgcagaggtcagaccttcgagggttgttttggttt

SEQ ID NO: 898 - DNA, 52 bp, synthetic construct
  source 1..52: mol_type = other DNA
ctccccattccatgagcatgcagaggcagaccttcgagggttgttttggttt

SEQ ID NO: 899 - DNA, 57 bp, synthetic construct
  source 1..57: mol_type = other DNA
ctccccattccatgagcatgcagaggtgagtcagaccttcgagggttgttttggttt

SEQ ID NO: 900 - DNA, 49 bp, synthetic construct
  source 1..49: mol_type = other DNA
ctccccattccatgagcatgcagaagaccttcgagggttgttttggttt

SEQ ID NO: 901 - DNA, 48 bp, synthetic construct
  source 1..48: mol_type = other DNA
ctccccattccatgagcatgcagagaccttcgagggttgttttggttt

SEQ ID NO: 902 - DNA, 49 bp, synthetic construct
  source 1..49: mol_type = other DNA
ctccccattccatgagcatgcagcagaccttcgagggttgttttggttt

SEQ ID NO: 903 - DNA, 51 bp, synthetic construct
  source 1..51: mol_type = other DNA
ctccccattccatgagcatgcagagcagaccttcgagggttgttttggttt

SEQ ID NO: 904 - DNA, 53 bp, synthetic construct
  source 1..53: mol_type = other DNA
ctccccattccatgagcatgcagaggtgagaccttcgagggttgttttggttt

SEQ ID NO: 905 - DNA, 59 bp, synthetic construct
  source 1..59: mol_type = other DNA
ctccccattccatgagcatgcagaggtgagtatcagaccttcgagggttgttttggttt

SEQ ID NO: 906 - DNA, 54 bp, synthetic construct
  source 1..54: mol_type = other DNA
ctccccattccatgagcatgcagaggtgaagaccttcgagggttgttttggttt

SEQ ID NO: 907 - DNA, 56 bp, synthetic construct
  source 1..56: mol_type = other DNA
ctccccattccatgagcatgcagaggtgagcagaccttcgagggttgttttggttt

SEQ ID NO: 908 - DNA, 52 bp, synthetic construct
  source 1..52: mol_type = other DNA
ctccccattccatgagcatgcagaggtagaccttcgagggttgttttggttt

SEQ ID NO: 909 - DNA, 55 bp, synthetic construct
  source 1..55: mol_type = other DNA
ctccccattccatgagcatgcagaggtatcagaccttcgagggttgttttggttt

SEQ ID NO: 910 - DNA, 47 bp, synthetic construct
  source 1..47: mol_type = other DNA
ctccccattccatgagcatgcagaaccttcgagggttgttttggttt

SEQ ID NO: 911 - DNA, 54 bp, synthetic construct
  source 1..54: mol_type = other DNA
ctccccattccatgagcatgcagaggtacagaccttcgagggttgttttggttt

SEQ ID NO: 912 - DNA, 55 bp, synthetic construct
  source 1..55: mol_type = other DNA
ctccccattccatgagcatgcagaggtgagtgaccttcgagggttgttttggttt

SEQ ID NO: 913 - DNA, 60 bp, synthetic construct
  source 1..60: mol_type = other DNA
ctccccattccatgagcatgcagatgtgagtatacagaccttcgagggttgttttggttt

SEQ ID NO: 914 - DNA, 60 bp, synthetic construct
  source 1..60: mol_type = other DNA
ctccccattccatgatcatgcagaggtgagtatacagaccttcgagggttgttttggttt

SEQ ID NO: 915 - DNA, 60 bp, synthetic construct
  source 1..60: mol_type = other DNA
ctccccattccatgagcatgcagaggtgagtatacagaccttcgagtgttgttttggttt

SEQ ID NO: 916 - DNA, 52 bp, synthetic construct
  source 1..52: mol_type = other DNA
ctccccattccatgagcatgcagatacagaccttcgagggttgttttggttt

SEQ ID NO: 917 - RNA, 23 nt, synthetic construct
  source 1..23: mol_type = other RNA
ccgcagttaccctctgcgtaatg

SEQ ID NO: 918 - RNA, 22 nt, synthetic construct
  source 1..22: mol_type = other RNA
cgcagttaccctctgcgtaatg

SEQ ID NO: 919 - DNA, 300 bp, synthetic construct
  source 1..300: mol_type = other DNA
tataagcagagctcgtttagtgaaccgtcagatcgcctggagacgccatccacgctgttttgacctccatagaagattctagagcgagaaaagccttgtttgccaccatggaacggctcggagatcatcattgcgtcgcgaggtgagcaagggcgaggagctgttcaccggggtggtgcccatcctggtcgagctggacggcgacgtaaacggccacaagttcagcgtgtccggcgagggcgagggcgatgccacctacggcaagctgaccctgaagttcatctgcaccaccggcaagct

SEQ ID NO: 920 - DNA, 303 bp, synthetic construct
  source 1..303: mol_type = other DNA
atattcgtctcgagcaaatcacttggcagtctagcggacctctgcggtaggtgcgacaaaactggaggtatcttctaagatctcgctcttttcggaacaaacggtggtaccttgccgagcctctagtagtaacgcagcgctccactcgttcccgctcctcgacaagtggccccaccaccacgggtaggaccagctcgacctgccgctgcatttgccggtgttcaagtcgcacaggccgctcccgctcccgctacggtggatgccgttcgactgggacttcaagtagacgtggtggccgttcga

SEQ ID NO: 921 - protein, 53 aa, synthetic construct
VSKGEELFTGVVPILVELDGDVNGHKFSVSGEGEGDATYGKLTLKFICTTGKL

SEQ ID NO: 922 - DNA, 300 bp, synthetic construct
  source 1..300: mol_type = other DNA
tataagcagagctcgtttagtgaaccgtcagatcgcctggagacgccatccacgctgttttgacctccatagaagattctagagcgagaaaagccttgtttgccaccatggaacggctcggagatcatcattgcgnaangtgagcaagggcgaggagctgttcaccggggtggtgcccatcctggtcgagctggacggcgacgtaaacggccacaagttcagcgtgtccggcgagggcgagggcgatgccacctacggcaagctgaccctgaagttcatctgcaccaccggcaagctgcc

SEQ ID NO: 923 - DNA, 300 bp, synthetic construct
  source 1..300: mol_type = other DNA
atattcgtctcgagcaaatcacttggcagtctagcggacctctgcggtaggtgcgacaaaactggaggtatcttctaagatctcgctcttttcggaacaaacggtggtaccttgccgagcctctagtagtaacgcnttncactcgttcccgctcctcgacaagtggccccaccacgggtaggaccagctcgacctgccgctgcatttgccggtgttcaagtcgcacaggccgctcccgctcccgctacggtggatgccgttcgactgggacttcaagtagacgtggtggccgttcgacgg

SEQ ID NO: 924 - protein, 54 aa, synthetic construct
VSKGEELFTGVVPILVELDGDVNGHKFSVSGEGEGDATYGKLTLKFICTTGKLP

SEQ ID NO: 925 - DNA, 79 bp, synthetic construct
  source 1..79: mol_type = other DNA
atctccccattccatgagcatgcagaggtgagtatacagaccttcgagggttgttttggttttggtttttgcttttggc

SEQ ID NO: 926 - DNA, 65 bp, synthetic construct
  source 1..65: mol_type = other DNA
atctccccattccatgagcatgcagaccttcgagggttgttttggttttggtttttgcttttggc

SEQ ID NO: 927 - DNA, 58 bp, synthetic construct
  source 1..58: mol_type = other DNA
atctccccattccatgagcatgcagagggttgttttggttttggtttttgcttttggc

SEQ ID NO: 928 - DNA, 69 bp, synthetic construct
  source 1..69: mol_type = other DNA
atctccccattccatgagcatgcagacagaccttcgagggttgttttggttttggtttttgcttttggc

SEQ ID NO: 929 - DNA, 70 bp, synthetic construct
  source 1..70: mol_type = other DNA
atctccccattccatgagcatgcagaggtgaccttcgagggttgttttggttttggtttttgcttttggc

SEQ ID NO: 930 - DNA, 71 bp, synthetic construct
  source 1..71: mol_type = other DNA
atctccccattccatgagcatgcagatacagaccttcgagggttgttttggttttggtttttgcttttggc

SEQ ID NO: 931 - DNA, 73 bp, synthetic construct
  source 1..73: mol_type = other DNA
atctccccattccatgagcatgcagaggtacagaccttcgagggttgttttggttttggtttttgcttttggc

SEQ ID NO: 932 - DNA, 77 bp, synthetic construct
  source 1..77: mol_type = other DNA
atctccccattccatgagcatgcagaggtgagtacagaccttcgagggttgttttggttttggtttttgcttttggc

SEQ ID NO: 933 - DNA, 73 bp, synthetic construct
  source 1..73: mol_type = other DNA
atctccccattccatgagcatgcagaggtgcagaccttcgagggttgttttggttttggtttttgcttttggc

SEQ ID NO: 934 - DNA, 72 bp, synthetic construct
  source 1..72: mol_type = other DNA
atctccccattccatgagcatgcagaggtcagaccttcgagggttgttttggttttggtttttgcttttggc

SEQ ID NO: 935 - DNA, 74 bp, synthetic construct
  source 1..74: mol_type = other DNA
atctccccattccatgagcatgcagaggtgacagaccttcgagggttgttttggttttggtttttgcttttggc

SEQ ID NO: 936 - DNA, 67 bp, synthetic construct
  source 1..67: mol_type = other DNA
atctccccattccatgagcatgcagagaccttcgagggttgttttggttttggtttttgcttttggc

SEQ ID NO: 937 - DNA, 74 bp, synthetic construct
  source 1..74: mol_type = other DNA
atctccccattccatgagcatgcagaggtatcagaccttcgagggttgttttggttttggtttttgcttttggc

SEQ ID NO: 938 - DNA, 70 bp, synthetic construct
  source 1..70: mol_type = other DNA
atctccccattccatgagcatgcagagcagaccttcgagggttgttttggttttggtttttgcttttggc

SEQ ID NO: 939 - DNA, 68 bp, synthetic construct
  source 1..68: mol_type = other DNA
atctccccattccatgagcatgcagcagaccttcgagggttgttttggttttggtttttgcttttggc

SEQ ID NO: 940 - DNA, 70 bp, synthetic construct
  source 1..70: mol_type = other DNA
atctccccattccatgagcatgcagtacagaccttcgagggttgttttggttttggtttttgcttttggc

SEQ ID NO: 941 - DNA, 71 bp, synthetic construct
  source 1..71: mol_type = other DNA
atctccccattccatgagcatgcagaggcagaccttcgagggttgttttggttttggtttttgcttttggc

SEQ ID NO: 942 - DNA, 72 bp, synthetic construct
  source 1..72: mol_type = other DNA
atctccccattccatgagcatgcagagtacagaccttcgagggttgttttggttttggtttttgcttttggc

SEQ ID NO: 943 - DNA, 66 bp, synthetic construct
  source 1..66: mol_type = other DNA
atctccccattccatgagcatgcagaaccttcgagggttgttttggttttggtttttgcttttggc

SEQ ID NO: 944 - DNA, 56 bp, synthetic construct
  source 1..56: mol_type = other DNA
atctccccattccatgaccttcgagggttgttttggttttggtttttgcttttggc

SEQ ID NO: 945 - DNA, 56 bp, synthetic construct
  source 1..56: mol_type = other DNA
atctccccattccatgagcatgcagggttgttttggttttggtttttgcttttggc

SEQ ID NO: 946 - DNA, 74 bp, synthetic construct
  source 1..74: mol_type = other DNA
atctccccattccatgagcatgcagaggttacagaccttcgagggttgttttggttttggtttttgcttttggc

SEQ ID NO: 947 - DNA, 63 bp, synthetic construct
  source 1..63: mol_type = other DNA
atctccccattccatgagcatgcagattcgagggttgttttggttttggtttttgcttttggc

SEQ ID NO: 948 - DNA, 39 bp, synthetic construct
  source 1..39: mol_type = other DNA
ccttcgagggttgttttggttttggtttttgcttttggc

SEQ ID NO: 949 - DNA, 70 bp, synthetic construct
  source 1..70: mol_type = other DNA
atctccccattccatgagcatgcagaacagaccttcgagggttgttttggttttggtttttgcttttggc

SEQ ID NO: 950 - DNA, 38 bp, synthetic construct
  source 1..38: mol_type = other DNA
cttcgagggttgttttggttttggtttttgcttttggc

SEQ ID NO: 951 - DNA, 57 bp, synthetic construct
  source 1..57: mol_type = other DNA
atctccccattccatgagcatgcagaggttgttttggttttggtttttgcttttggc

SEQ ID NO: 952 - DNA, 64 bp, synthetic construct
  source 1..64: mol_type = other DNA
atctccccattccatgagcatgcagacttcgagggttgttttggttttggtttttgcttttggc

SEQ ID NO: 953 - DNA, 69 bp, synthetic construct
  source 1..69: mol_type = other DNA
atctccccattccatgagcatgcagaggtaccttcgagggttgttttggttttggtttttgcttttggc

SEQ ID NO: 954 - DNA, 30 bp, synthetic construct
  source 1..30: mol_type = other DNA
gttgttttggttttggtttttgcttttggc

SEQ ID NO: 955 - DNA, 75 bp, synthetic construct
  source 1..75: mol_type = other DNA
atctccccattccatgagcatgcagaggtgtacagaccttcgagggttgttttggttttggtttttgcttttggc

SEQ ID NO: 956 - DNA, 71 bp, synthetic construct
  source 1..71: mol_type = other DNA
atctccccattccatgagcatgcagaggtagaccttcgagggttgttttggttttggtttttgcttttggc

SEQ ID NO: 957 - DNA, 65 bp, synthetic construct
  source 1..65: mol_type = other DNA
atctccccattccatgagcatgcagaggttcgagggttgttttggttttggtttttgcttttggc

SEQ ID NO: 958 - DNA, 60 bp, synthetic construct
  source 1..60: mol_type = other DNA
atctccccattccatgagcatgcttcgagggttgttttggttttggtttttgcttttggc

SEQ ID NO: 959 - DNA, 49 bp, synthetic construct
  source 1..49: mol_type = other DNA
atctccccattccatgagggttgttttggttttggtttttgcttttggc

SEQ ID NO: 960 - DNA, 68 bp, synthetic construct
  source 1..68: mol_type = other DNA
atctccccattccatgagcatgcagaagaccttcgagggttgttttggttttggtttttgcttttggc

SEQ ID NO: 961 - DNA, 75 bp, synthetic construct
  source 1..75: mol_type = other DNA
atctccccattccatgagcatgcagaggtatacagaccttcgagggttgttttggttttggtttttgcttttggc

SEQ ID NO: 962 - DNA, 76 bp, synthetic construct
  source 1..76: mol_type = other DNA
atctccccattccatgagcatgcagaggtgatacagaccttcgagggttgttttggttttggtttttgcttttggc

SEQ ID NO: 963 - DNA, 68 bp, synthetic construct
  source 1..68: mol_type = other DNA
atctccccattccatgagcatgcagaggaccttcgagggttgttttggttttggtttttgcttttggc

SEQ ID NO: 964 - DNA, 78 bp, synthetic construct
  source 1..78: mol_type = other DNA
atctccccattccatgagcatgcagaggtgagtatcagaccttcgagggttgttttggttttggtttttgcttttggc

SEQ ID NO: 965 - DNA, 24 bp, synthetic construct
  source 1..24: mol_type = other DNA
atctccccattccatgagcatgca

SEQ ID NO: 966 - DNA, 69 bp, synthetic construct
  source 1..69: mol_type = other DNA
atctccccattccatgagcatgcagaggtgccttcgagggttgttttggttttggtttttgcttttggc

SEQ ID NO: 967 - DNA, 77 bp, synthetic construct
  source 1..77: mol_type = other DNA
atctccccattccatgagcatgcagaggtgagtatagaccttcgagggttgttttggttttggtttttgcttttggc

SEQ ID NO: 968 - DNA, 68 bp, synthetic construct
  source 1..68: mol_type = other DNA
atctccccattccatgagcatgcagaggtccttcgagggttgttttggttttggtttttgcttttggc

SEQ ID NO: 969 - DNA, 67 bp, synthetic construct
  source 1..67: mol_type = other DNA
atctccccattccatgagcatgcagaggtcttcgagggttgttttggttttggtttttgcttttggc

SEQ ID NO: 970 - DNA, 67 bp, synthetic construct
  source 1..67: mol_type = other DNA
atctccccattccatgagcatgcacagaccttcgagggttgttttggttttggtttttgcttttggc

SEQ ID NO: 971 - DNA, 62 bp, synthetic construct
  source 1..62: mol_type = other DNA
atctccccattccatgagcatgaccttcgagggttgttttggttttggtttttgcttttggc

SEQ ID NO: 972 - DNA, 68 bp, synthetic construct
  source 1..68: mol_type = other DNA
atctccccattccatgagcatgcagaggtacttcgagggttgttttggttttggtttttgcttttggc

SEQ ID NO: 973 - DNA, 72 bp, synthetic construct
  source 1..72: mol_type = other DNA
atctccccattccatgagcatgcagaggacagaccttcgagggttgttttggttttggtttttgcttttggc

SEQ ID NO: 974 - DNA, 61 bp, synthetic construct
  source 1..61: mol_type = other DNA
atctccccattccatgagcatgccttcgagggttgttttggttttggtttttgcttttggc